European Patent Specification EP 3 580 332 B1, published April 15, 2026. Title: Methods and kits for generating mimetic innate immune cells from pluripotent stem cells. Applicant: Agency for Science, Technology and Research ZENG, Jieming WANG, Shu. The sequence listing filed with the application follows.

SEQUENCE LISTING (15 sequences)

SEQ ID NO: 1 - DNA, 128032 bp, Homo sapiens
atgcggtgggccctagcggtgcttctagctttcctgtctcctggtgagtgcgctgcctacagagaggatcacgggttttgttttgttttgttattttcttcttttgcaaggagcgacatactaagaaatgcctcattatattttgtgttgttcccattgcagccagtcagatatcttccaacttggaagggagaacgaagtcagtcaccaggctgactgggtcatctgctgaaatcacctgtgatcttcctggagcaagtaccttatacatccactggtacctgcaccaggaggggaaggccccacagtgtcttctgtactatgaaccctactactccagggttgtgctggaatcaggaatcactccaggaaagtatgacactggaagcacaaggagcaattggaatttgagactgcaaaatctaattaaaaatgattctgggttctattactgtgccacctgggacaggcacagtgattcagacactgaaaatctgcctgtggttgcttctggtacacaagatagaccagccaactctcatttcctgccctgaatttactgtattctgtacaaagagaaacacagcttaactcctgatctcccctgcaatatcacactcccctggcagcagctgcaccctgttccccaccctcccccaggactttcctgaagaccaagctgccacctccaagcctcagctaagcagcctggctgagagcaagtttctctcagctctcctagaacatggggaaggcccactcactctgcttcctaggacagacaggtacagctagggtccagctgtgaagcaagacattttggacaaaaatgggaagggtattcatactgaatcatacatccaataatggtccagagatcgcagctgagagtggtgcttattccttatgtctataacaatataagcaatactataatgaccactaaaacactaggccaatatatgcagttgaacattctctctctctgccctcccttttattctcgctctcctttcttacttccatgcttgcttttatcattttctctccctccctcccttcctcctttccttccatcaccccaccctccttcctttctttccttccttccttccttgcttttctctctttctctcctttttgtgtacataatcacaatactttttccacaaaatcatttgaaatagtttttctctatttgttcatgccaacattgatatagctgctttaattgttcagtttcatttttatattttggaaatttgtgtattattttgttttgtttcatatttgttttgtatacgtaaaacatttagttggaactgaagtcaaaattataaaagatgacacatttgaagattttagcttccattgtagacttctcattcctcttttctccctgacactataggtaacaatatttttatccgttttcttgaactttttcactctgtcatagcgcagtatgtatcaattctatttcaatgccatatttatatttttgttcctatatttggtttttatacattttaatcaatcttatattttcccgtgtctggattgtgtgtcttacttctaaaggtgcacatacttcataagtatgcataaagacgtccatatcatttatttgaatgtttttatgtgttgattatttaatgatggcatcattgatctatcaggaatttttatacaataattactgtattagtaataataatactggccaggcccggtggctcatgcctgtaatcccagcatttgagtagtacagtcgttaggaatacttaggccgggagattgcgaccagcttagccaacatggtgaaaccctgtctctactaaaaatacaaaaaattagctggctgtggcggtgcacacatgtaatcccagctacttggatgctgaagcaggagaatctcttgagcctagaaggtggagttttcagtgagctaatatcacactactgcagtccagtttgggcaacacagtgagactctgtctcaaaaagactaataataataataatattgatggtaaatatgggtactgacattctggtagttaatgtactaagcacattgcatgcatattgtatttaatctacacagaaacttcattaaggatttaaagtactgttgaatgtaacattagaaattggggggttaattaacattccctaagtcatatactttaatttgataatgattgcaatccaagctctgtggttcagaaaatgagatttgttaattcggtttgcattcccccatcgtaggagtactagcatcattttacaactttacagttcatttatatttcttcttttgagaattgccttgtacactcttttcctattcttctattggaggattagttttttcttattggttcgtaagaattaatatacaccattttagagatactgaccctttatccaatgtgttgaagatatttctcctcatttgttattatttacatttggcaccttttggagaattgaactttgaaaaaaacaaaatctatcaatttttctatggtgtctactttgatgtcaggtttagaaaggccaatctcacctagaatttctatgcaattcatcatcatttaagtctaatgattttctttttattacaactaaatcactatttgtaactggtaaggtagaaatgcagcaatatttgtttccatatggtaagtcaatatccaaaagagaacttatgaaataattgactatttccttgtggatattaacatatcactttatcacatgataaaatattacatacatgcagctttctttctggattttccactgtgttccatgaatcttgtcattctagtgccagtattgccttctcttcagcactgtagctttatagttcttttcacattctgatgaagtttctctcattatctttttgttttaagaattttctgtgcatgctagtgtgatctcaatcctctcccttcccatttttaaaccgtgagacttctgtccagcaagactttttcacgctccaaggcaggcaagcttccctccttcacaaggacctgagaattcagctttcagagctgttcctgtggaagcctcatgtcctgcacatatggtccagaggcagagggagaccaaccggagccccctccctttctcattcccagctgtgatgacagcaaaaactgaactctgtgagctaggccaacaacacaattaagagagacattgttctacatctcattatgcatctttcaaacatgtgtctctatatacttctgacacaggtggtggtaatctgtgtatgccttactgaattttcacaattatattactgtactacttttgtcccctatatttccatctgtgaatccaggtgtactgcagatctcagtcccctttctgagggtagggctgacaaataaaatatacaataccaaacaatttggaagttcagataaacaacaagtttttagtttaagtatgttccaaatattgcatgacatggcaccctgaactacttagaaaaaaaaaacaaaaaaacctcacactcctacttcagtgaacaaaaatcctctaataaagagatcacacccacaggatcacacacacacaaacacacacacacacacacaccccacatacacccatttatcttagagcagagtccaagacccaccaacacacatgatcctcagtcctttcatttttattatttatttatttatttatatttattatactttaagtgctagggtacatatgcacaacgtgcaggtttgttacatatgtatacatgtgccatgttggtttgttgcacccatcaacttgtcatctacattaggtatatctcttaatgctatccctcccccctccccccaccccactacaggccccagtgtgtgatgttcccccactctgtgtccaagtgttctccttgttcaattcccacctacgagtgagaacatgcactgtttggatttctgtccttggaatagtttgctcggaatgatggtttccagcttcatccatgtccttacaaaggacatgaacgcatccctttttatggccgcatagtattccatggtgtatatgtgccacattttcttaatccagtctatcattgatggacatttgggttggttccaagtctctgctatcgtgaatagtgccacaataaacatatgctttgcgtggtgcctccaagtgtcctcgcagatgccaaaaggaaggtggttcagttccctaatcagagacttcctggcaggacaaggtcctggcatcagcattagctgctgcaactctgaagggcagggtgtgagcctgctgtgggactgccccctcctagggctgggcctgctgactccagggtctgcttcccccacctctgcactccctctgctgcaggcctgagctctccttgcccctggctctcttctgcagagggcctgctctcagctgccacaagagggcgccggagaacggacctgagcagagaggcaggggctcctctgcaggtcctcccaggcaccaacccttctgggagggaggaaggcttgggagtcctcttagacagatcctcagtcacttccctctgcttgtgtctcaggaagaccacctcctcctactgtcttctgtgctagggatcacttccttgttgagtggaacctgagttttaagaggatcttctgctcctcttcatctggtccctttccttccaaggccccagagaggaaggcatgcagtgggccctagcggtgcttctagctttcctgtctcctggtgagtgcgctgcctacagagaggatcacgggttttgttttattttcttcttttgcaaggagtaccatactaaggaattcctcattatattttgtgttgttcccattgcagccagtcagaaatcttccaacttggaagggagaacgaagtcagtcatcaggcagactgggtcatctgctgaaatcacttgtgatcttgctgaaggaagtaacggctacatccactggtacctacaccaggaggggaaggccccacagcgtcttcagtactatgactcctacaactccaaggttgtgttggaatcaggagtcagtccagggaagtattatacttacgcaagcacaaggaacaacttgagattgatactgcgaaatctaattgaaaatgactttggggtctattactgtgccacctgggacgggcacagtgattcagatccgccctacaccacactgaaaatctgccttgtggctgcttctggtacacaagatagagccgccccctctcatttcctgccaccaaatttaccgtgtgctgaacaagagaaacattgcttaactcctgatctcccctgcaatattacactcccctggcagcagctgcaccctgttccccaccctcccccaggactttcctgaagaccaagccgccatctcagctaagcctcagagaagcagcctggctgagagcaaggttctcttagctctcctaggacatgggggaggcccactcactctgcttcctaggacaaatgggtacccctagggtccagctgtaaagcaagatattttggacaacaaatgggaagggaatttatactaaattgtgtatcccatcatgatccagaaaccgcagctgagactggtgcttattccttatgtctataacaatataagcaatactataatgaccactgaaacaccaggcctaggtatgcagttgaacattctctccctctgccctcccttttattctctctctcttttttcttaattctttgcttgcttttattatttttctctctcccttcctccctcgctccatcgctccctccgtccttccctccctctctccctctctccttccctcccttcctctcttctttccttccatccattctccttcgttttccttccttccttctttgcttttctcttgctttcctttttgggtacataatcagaatactttttccacaaaatcatttgaaataatttttctctatgtgttcatgtcaacattgatatagctactttaattgttcagttttcttttttacattttggaaatttgttgtattactttgttttgtttcatatctgttttgtatatataaaacatttacatggaagtgaagtcaaaattataaaagatgatgcatttgaagattttagcttccattgtagacttctcattcttcttttctccctgacactataggtaacaatatttttggcagttcacttgagttttttcactgtttgtcatagcggagtatgtattgtttctatttcaatgccatatttatattttctttctgatattcagtttctatatattttaatcaatcttatattttcctgtgtctggactgtgtgtcttacttctaaaggtgcacatacttcataagtatgcataaagacgtccatatcatttatttgaatgtttttatgcattcattatttaatgatggcatcattgatctatcaggaatttttatacaataattactgtattagtaataataatactggccaggcccggtggttcatgcctgtaatcccagcatttgggcagtccagtcgttaggatcacttaggccgggagattgcgaccagcttagccaacatggtgaaaccctgtctctactaaaaatacaaaaaattagctggctatagtggcgcacacatgtaatcccagctacttgaatgctgaagcaggagaatctgtagagcctggtaggtggagttttcagtgagctaatatcacactactgcagtccagtttgggcaacagagtgagactctgtctcaaaaaaatgaataacgataataataatattgatgctacatatgggtactgacattctggtagttaatgtactaagcacattacatgcatattttatttaatctacacagaaatttcattagggtttaaagtactgttgaatgtaacattagaaattgagggggttaattaacattccctgagtcatatactttaacttgataatgattgcaatccaagctctgtgattctgaaaacgagatttgtaaattcagtttgcattccctcatctttgggagtactaacattatttcacaactttataggtcatttatagttcttcttttgtgaattgccttgtcatactctttgcctattcctctcttggaggattaattttttcttattagtttgtaagagttaatatacactattttaaagatactgaccctttatccaatgtgttgaagatatttctcctcatttgttgttatttacatttggcatcttttggtgaattgaactttgaaaaaaaaagcattaaaatctatcagtttttctagggtgtctagtttgatgtcaagcttagaaaggccaatctcacctagaatttctatgcaattcatcattgtttaagtgtaatgattttgtttttattacaactaaatcactatctatatctggtaagaacgaaatgcaataatatttgtttccatatggtaagtcaatacccaaaacagaacttataaaataattgactatttccttgtgggtattaacatatcactttatcacatgataaaatattacatacgtgtggctctctttctggattttccactgtgttccatgaatcttctcattctagtgccagtattgccctctcttcagcactgtagctttatacttcttttcacattttgatgaagtttctctcattatttttttgttttaagaattttctgtgcattctagtgtgatctcaatcctctcccttcccatttttaaaccatgagacttctgtcctgcaagactttttcacgctccaaggcaggcaagcttccctccttcacaaggacccgagaactcagctttcagagctgctcctacagcagcctcatgtcctgcatgtgtgctccagaggcagagggagaccaaccagagccccctccctttctcattcccagctgtgatgacagcagaaactgaactctctgagctagcccaacacaacaactgagagggacactgttctccatctcattatgcatatttcaaacatgtgtctctatatacttcttacagaggtggtgataatctgtgaatgccttactgaattttcacaataatattactgtacttgatttgtccccttattttcatctgtgaagccaggtgcactgcagatattagtctgctttctgagggtagggatgacaaataaaatatacaataccgggggaattggaagttcagataaataacaagtttttagtttaagtatgttccaaatattgcatgacatggcacccagttctactttaaaaacaaacaagcaaacaaacaaattcacactcctactttaatgaacaaaaatcttctaataaggaggtcacacacacaggattacaggcacaacccccacacacaaacacacacacacatttaccttagagcagagtccaggacacaccaacacacatgatcctcagtccttttaatttaaagcacgttcaacccttctcagagtggccttgagtggttgcctccatgagtctgcagatgcgaaaaggaagttggttccgggccctaatcagaggcttcctgtcaggacaaggttctggcatcagcattacctgctgcaactctgaagggcagggtgggagcctgctatgggactgccccctccaaggtgtgagcctgttaattccagggtcagcttacccaacatctgcagtccctcagctggaggcctgagctcttaatgcccctgcctcccttctgccctgggcctgctctcagctgccacaagagggcgccgaagaaagggcctgaggagatgcaggagctcctctgcaggtcctcccaggcaccaccccttctgggaggaaggcttgggagtcccctaagacacatcttcagtcacttctctctgcctgtgtctcaggaaaccagctcctcctactgtcttctgtgctagggatcacttccttgttgagtggggcctgagttttaagaggatcttctgctcctcttcatctggtccgtttccttccaaggcccccgagaggaaggcatgcggtgggccctactggtgcttctagctttcctgtctcctggtgagtacgctgcctacagagaggctcacaggttgggttttgttttgttttcttcttgaaaggggtgccatacaaaggaatacctcattgtattttgtgttgttcccattgcagccagtcagaaatcttccaacttggaagggagaacgaagtcagtcaccaggcagactgggtcatctgctgaaatcacttgcgatcttactgtaacaaataccttctacatccactggtacctacaccaggaggggaaggccccacagcgtcttctgtactatgacgtctccaccgcaagggatgtgttggaatcaggactcagtccaggaaagtattatactcatacacccaggaggtggagctggatattgagactgcaaaatctaattgaaaatgattctggggtctattactgtgccacctgggacaggcacagtgattcagacctgtcctacaccacactgaaaatctgccttgtggctgcctctggtacacaagatagagccgccccctctcatttcctgccaccaaatttcctgtattctgaacaagagaaagacagcttaactcctgatctccctcctaatatcacactgtcctggcagcagctgcatcctgttccccacccctcccccacaactttcctgaagatcaagctgccatctccaggcctcagctaagcagcctggctgagagcaaggttctctcagctctcctaggacatgggggaggcccactcactctgcttcctatgacacacaggtacaactagggtccagctgtgaagcgagatattttggacagcaaatgggaagggtatttatactgaatcatgtatccactcatggtccagagatcacagctgagagtggtgcttattccttatgtctataacaacataagcaatactataatgaccactaaaacactaggcccaggtatgcagttgaacatggtctccctctgccctcccttttattctctctctcttttcttacttctttgcttgtttttatttttctctccctccctaactccctccctccatccatcctttcctcccttcctcccttgtttccttccatccattctccttccttgttttccttccttccttccttgcttttctctctctttctttcctttttgggtacataatcagaatactttttccacaaaatcatttgatataatttttctctatatgttcatgccaacattcatacagctagtttaattgttcagttctctttttcacattttggaattttgttgtattactttgttttgcttcatatctgttttgtatatataaaacatttacatgaaactgaagccaaaattataaaagatgatgcatttgaagattttagcttccattgtagatttctcgttcctcttttctccctgacactataggtaacaatatttttggcagttcacttgagctttttcactgtttgtcatagcggagtatgtattgtttctattttaatgccatatttatattttcgttctgatatttggtttttatacattttaatcaatcttatattttcccgtgtctggactgtgtgtcttacttctaaaggtgcacgtacttcataagtatgcataaagaagtccatatcatttatttgaatgtttttatgcgttgattatttaatgatggcatcatcgatctatcaggaatttttatacaataattactgtattagtaataataatacttgccaggcccggtggctcatgcctgtaatcccagcatttgggcagtccagtcgttaggaacacttaggccgggagattgcgaccagcttagccaacatggtgaaaccctgtctctactaaaaatacaaaaaattagccggctgtagtggcgcacacatgtaatcccagctactttggatgctgaggcaggagaaactcttcaacctggaagttggagttttcagtgagctaagatcacactactgcagtccagtttgggcaacacagcgagactctgtctcaaaaagactaataataataataatattgatggtaaatatgggtactgacattctggtagttaacgtactaagcacattgcatgcacattttatttaatctacacagaaacttcattaaggttttaaagtactgttgaatgtaacattagaaattggggggttaattaacattccctaagtcatatactttatcttgataatgattgcaatgcaagctctgtggttcctaaatgagatttgttaatttggtttgcattcccccatctttaggagtactagcatcattttacaactttacaggtcatttatagttcttcttttgagaattgccttgtcatactcttttcctattctttttttggaagattagttttttcttattagttcgtaagaattaatatacaccattttagagatactgaccctttatccaatgtgttgaagatatttctcctcatttgttattatttacatttggcaccttttggtgaattcaactttgaaaaaaaaacaataaaagctatcaatttttctagggtgtctagtttgatgtcaggcttagaaaggccaatctcacctagaatttctatgcaattcatcatcgtttaagtctaatgattttctatttattacaactaaatcactatttgtaactagtaaggtagaaatgcaacaatatttgtttccatgtggtaagtcaataccaaaaagagaacttatttaataactgactatttccttgtgggtattaacatatcactttatcacatgataaaatattacatacatgcagctctctttctggattttccactgtgttccatgaatcttgtcattctagtgccagtattgccctctcttcagcactgtagctttatagttcttttcacattctgatgaagtttctctcattatttttttgttttaagaattttctgtgcattctagtgtgatctcaatcctctcccttcccatttttaaaccgtgagacttctgtccagcaagactttttcacgctccaaggcaggcaagcttccctccttcacaaggacccgagaactcagctttcagagctgttcctgtggaagcctcatgtcctgcacgtgtgctccagaggcagagggagaccaaccggagccccctccctttctcattcccacctgtcattcccagctgtgaagacagcagaaaccgaactctgtgagctaggccaataccacaactgagaggaatattgttctacatctcattatgcatctttcaaacatgtgtctctatatacttcttacagaggtggtgataatctgtgtatgccttactgaattttcacaattatattactgtacttcctttgtcccctatatttccatctgtgaatccaggtgtactgcagatctcagtcccctttctgagggtagggctgacaaataaaatatacaataccaaacaatttggaagttcaggtaaacaacaagtttttagtttaagtatgttccaaatattgcatgacatggcaccctgaactacttagaaaaaaaaaaacaaaaaaaactcacactcctacttcaatgaacaaaaatcctctaataaagagatcacaaccacaggatcacacacacacaaacacacacacacacacacacccaacacacacacctttatcttagagcagagtccaagaccaaccaacacacatgatcctcagttcttttatttttattatttctttatttatttatatttattatactttaagtgctagggtacatttgcacaacgtgcaggtttgttacatatgtatacatgtgccatgttggtttgttgcacccatcaacttgtcatctacattaggtatatctcctaatgctatccctcccccctgcccccaccccactacaggccccagtgcgtgatgttcccccactctgtgtccaagtgttctcattgttcaattcccacctacgagcgagaacatgcactgtttggatttctgtccttggaatagtttgctcggaatgatggtttccagcttcatccatgtccttacaaaggacatgaacgcatccctttttatggccgcatagtattccatggtgtatatgtgtcacattttcttaatccagtctatcactgatggacatttgggttggttccaagtctctgctatcgtgaatagtgccgcaataaacacacgctttgcgtggtgcctccaagtgtccttgcagatgccaaaaggaaggtggttcagttccctaatcagagacttcctggcaggacaaggtcctggcatcagcattagctgctgcaactctgaagggcagggtgtgagcctgctgtgggactgccccctcctagggctgggcctgctgactccagggtcagcttccgctacatctgcattccctctgctgcaggcctgagctctcctggcccctggctctcttctgcagagggcctgctctcagctgccacaagagggcgccggagaacggacctgagcaagagaggcaggagctcctctgcaggtcctcccaggcaccaatccttctgggagggaggaaggcttgggagtcctcttagacagatcctcagtcacttctctctgcttgtgtctcaggaagaccagctcctcctactgtcttctgtgctagggatcacttccttgttgagtggggcctgagttttaagaggatcttctgctcctcttcatctggtccctttccttccaaggcctcagagaggaaggcatgcagtgggccctagcggtgcttctagctttcctgtctcctggtgagtgcgctgcctacagagaggatcatgggttttgttttctttattttcttcttttgcaaggattgccatactaaggaattcctcattatattttgtgttgttcccattgcagccagtcagaaatcttccaacttggaagggagaacgaagtcagtcatcaggcagactgggtcatctgctgaaatcacttgtgatcttgctgaaggaagtaccggctacatccactggtacctacaccaggaggggaaggccccacagcgtcttctgtactatgactcctacacctccagcgttgtgttggaatcaggaatcagcccagggaagtatgatacttacggaagcacaaggaagaacttgagaatgatactgcgaaatcttattgaaaatgactctggagtctattactgtgccacctgggatgggcacagtgattcagatccgccctacaccacactgaaaacctgccttgtggctgcttctggtacacaagatagagccgccccctctcatttcctgccaccaaatttaccgtgtgctgaacaagagaaacattgcttaactcctgatctcccctgcaatatcacactcccctggcagcagctgcaccctgttccccaccctcccccaggacttccctgaagaccaagccaccatctcagctaaacctcagagaagcagcctggctgagagcaaggttctcttagctctcctaggacatggcggaagcccactcactctgcttcctaggacaaatgggtacctctagggtccagctgtgaagcaagatattttggacaacaaatgagaagggtatttatactaaattgtgtatcccatcatgatccagaaatcgcagctgagactggtgcttattccttatatctataacaatgtaagcaatactataatgaccactgaaacaccaggcctaggtatgcagttgaacattctctccctctgccctcccttttattctctctctctttttttaattctttgcttgcttttattatttttctctctctcccttcctccttccctccgtccttccctccctccttccctccctctctccctccctccttccctcccttcctctcttctttccttccatccattctccttcgttttccttccttccttctttgcttttctcttgctttcctttttgggtacataatcagaatactttttccacaaaatcatttgaaataatttttctctatgtgttcatgtcaacattgatatagctactttaattgttcagttttcttttttacattttggaaatttgttgtattactttgttttgtttcatatctgttttgcatatataaaacatttacatggaagtgaagtcaaaatcataaaagatgatgcatttgaagattttagcttccattgtagacttctcattcttcttttctccctgacactataggtaacaatatttttggcagttcacttgagctgtttcactctgtttttcatagcggagtatgtattctttctatttgaatgccatatttatattttctttctgatattcagtttctatatattttaatcaatcttatattttcctgtgtctggactgtgtgtcttacttctaaaggtgcacatacttcataagcatgcataaagatgtccatatcatttatttgaatgtttttatgcattgattatttaatgatggcatcactgatctatcaggaatttttatacaataattactgtattagtaataataatactggccaggcccggtggctcatgcctgtaatcccagcatttgggcagtccagtcgttaggatcacttaggccgggagattgtgaccagctcagccaacgtggtgaaaccctgtctctagtaaaaatacaaaaaattagctggctgtagtggcacacacatgtaatcccagctacttggatgctgaagcaggagaatctgtagagcctggtaggtggagttttcagtgagctaatatcacactactgcagtccagtttgggcaacagagtgagactctgtctcaaaaaaatgaataacgataataataatattgatggtacatatgggtactgacattctggtagttaatgtactaagcacattacatgcatattttatttaatctacacagaaacttcattaaggtttaaagtactgttgaatgtaacattagaaattgggcggttaattaacattccctaagtcatatgctttaatttgataatgattgcaatccaagctctgtggttccgaaaatgagatttgtaaattcagtttgcattcccccatctttgggagtactagtattatttcacaactttataggttatttatagttcttcttttgtgaattgccatgtcatactctttgcctattcctctcttggaggattaattttttcttattatttcgtaagagttaagatacactattttaaagatactgaccctttatcgaatgtgttgaagatatttcccctcatttgttattatttacatttggcaccttttggtgaattgaactttgaaaaaaaaagcattaaaatctatcaatttttctagggtgtctagtttgatgtcaagcttagaaaggccaatctcacctagaatttctatgcaattcatcattgtttaagtgtaatgattttgtttttattacaactaaatcactatctatatctggtaagaacgaaatgcaataatatttgtttccatatggtaagtcaatacccaaaagagaacttataaaataattgactatttccttgtggatattaacatatcactttatcacatgataaaatattacatgcatgcggctttctttctggattttctactgtgttccatgaatcttctcattctagtgccagtattgccctctcttcagcactgtagctttatagttcttttcacattctgatgaaatttctctcattatttttttgttttaagaattttctgtgcattctagtgtgatctcaatcctctcccttcccatttttaaaccatgagacttctgtccagcaagactttttcatgctccaaggcatggaagctttcctccttcacaaggaccccgagaactcagctttcagagctgctcctacagcagcctcatgtcctgcacgtgtgctccagaggcagagggagaccaaccggagccccctccctttctcattcccagctgtgatgacagcagaaactgaattctctgagctaggacaacacaacaactgagagagacactgttctacatctcattatgcatctttcaaacatgtgtctctatatattcttacagaggtggtgataatctgcctatgccttactgaattttcacaataatattactatactttttttgtcccctatatttccaactgtgaatccaggtgcactgcagatattagtctgctttctgagggtagggatgacaaataaaatatacaataccgggggaattggaagtacagaaaaataacaagtttttagtttaagtatgttccaaatattgcatgacatggcacccagtactactttaaaaacaaacaagcaaacaaacaaattcacactcctactttaatgaacaaaaatcctctaataaggaggtcacacacacaggattacaggcacaacccctgcccccccaacacacacacacacatatttaccttagagcagactccgggacacaccaacacacatgatcctcagtccttttaataaagcacgttcaacccttctcagagtgaccttgagtggttgcctccatgagtctgcagatgcgaaaaggaacttggttcagggccctaatcagaggcttcctgtcaggacaaggttctggcatcagcattacctgctgcaactctgaagggcagggtgggagcctgctatgggactgccccctccaaggtgtgagcctgttaattccagggtcagcttacccaacatctgcagtccctcagctggaggcctgagctcttaatgcccctgcctcccttctgccctgggcctgctctcaactgccacaagatggcgcagaagaaagggcctgaggagatgcgggagctcctctgcaggtcctcccaggcaccaccccttctgggaggaaggcttgggagtcccctaagacacatcttcagtcacttctctctgcctgtgactcaggaagaccagctcctcctactgtcttctgtgctagggatcacttccttgttgagtggggccggagttttaagaggatcttctgctcctcctcatctggtccctttccttccaaggcccccgagaggaaggcatgcggtgggccctactggtgcttctagctttcctgtctcctggtgagtacgctgcctacagagaggctcacaggttgggttttgttttgtttacttcttttgaaaggggtgccatacaaaggaatacctcattaaattttgtgttgttcccattgcagccagtcagaaatcttccaacttggaagggggaacgaagtcagtcacgaggccgactaggtcatctgctgaaatcacttgtgaccttactgtaataaatgccttctacatccactggtacctacaccaggaggggaaggccccacagcgtcttctgtactatgacgtctccaactcaaaggatgtgttggaatcaggactcagtccaggaaagtattatactcatacacccaggaggtggagctggatattgatactacgaaatctaattgaaaatgattctggggtctattactgtgccacctgggacaggcacagtgattcagacctgtcctacaccacactgaaaatctgccttgtggctgcctctggttcacaggatagagccgccccctctcatttcctgtcaccaaatttactgtattctgaacaagagaaagacagcttaactcctgatctccctcctaatatcacactgtcctggcagcagccgcaccctgttccccacccctcccccacaactttcctgaagatcaagctgccatctccaggcctcagctaagcagcctggctgagagcaaggttctctcagctctcctaggacatgggggaggcccactcactctgcttcctatgacacacaggtacaactagggtccagctgtgaagcgagatattttggacagcaaatgggaagggtatttatactgaatcatgtatccagtcatggtccagagatcacagctgagagtggtgcttattccttatgtctataacaacataagcaatactataatgaccactaaaacactaggcccaggtatgcagttgaacatggtctccctctgccctcccttttattctctctctcttttttcttacttctttgcttgtttttatttttctctccctccctaactccctccctccatccatcctttcctcccttcctcccttgtttccttccatccattctccttccttgttttccttccttccttccttgcttttctctctctttctttcctttttgggtacataatcagaatactttttccacaaaatcatttgatataatttttctctatttgttcatgccaacatttatacagctagtttaattgttcagttttcatttttacattttggaaatgtgttgtattactttgttttgcttcatatctgttttgtatatataaaacgtttacatgaaactgaagccaaaattataaaagatgatgcatttgaagattttagcttccattgtagatttttcgttcctcttttctccctgacactataggtaacaatatttttggcagttcacatgagctttttcactgtttgtcatagtgccgtatgtattgtttctatttcaatgccatatttatattttcattctgatattcggtttttatacattttaatcaatcttatattttcccgtgtctggattgtgtgtcttacttctaaaggtgcacatacttcataagtatgcataaagacgtccatatcatttatttgaatgtctttatgcattgattatttaatgatggcatcattgatctatcaggaatttttatacaataattactgtattagtaataataatactggccaggcccggtggctcatgcctgtaatcccagcatttgggtggtccagtcattacgatcacttaggccaggagattgcgaccagcttagccaacatggtgaaaccctgtctctactaaaaatacaaaaaattagccggctgtagtggcgcacacatgtaatcccagctactttggatgctgaggcaggagaatctctagagcctggaaggtgaaggtttcagtgagctaagatcacactactacagtccagtttgggcaatagagtgagactctctctcaaaaaaatgaataatgataataataatattgatggtacatatgggtgctgacattctggtagttaatgtactaagcacattacatgcatattttatttaatctacacagaaacttcattaagggtttaaagtactgttgaatgaaacataagaaaatggggggttaattaacattccctaagccatatattttaatttgattatgatagcaatccaagctctgtggttccaaaaatgagatttgttaattcgatttgcattcccccatctttaggagtactagcaatatttgacaacgttataggtcatttataattcttcttttgagaattgccttgtcgtactctttgcctattctccctttggaggattaattttttcttattggttcgtaagaattaatatgtactattttagagatgatgaccctttatccaatgtgttgaagatattactcctcatttgttattatttacatttggcaccttttagtgaattcaactttgaaaaaaaaacaataaaacccatcaatttttctagggagtctagtttgatgtcagcttagaaaggccaatctcacccagaatctgtatgcaattcatcatcgtttaagtctattgattttcattttattacaactaaatcactatttgtaactggtaaggtagaaatgcgacaatatttgtttccatatggtaagtcaatacctaaaagagaacttattaaataattgactatttccttgtgaatattaatatatcactttatcacatgataaaatattacatacatgcagctctcttactgcattttccactgtgttccatgaatcttctcattctagtgccagtattgccctctcttcagcactgtagctttatagttcttttcacattctgatgaaatttctctcattatttttttgttttaagaattttctgtgcattctagtgtgatctcaatcctctcccttcccatttttaaaccatgagacttctgtccagcaagactttttcacgctccaaggcaggcaagcttccctccttcacaaggacccgagaactcagctttcagagctgctcctacagcagcctcttgtcctgcatgtgtgctccagaggcagagggagaccaaccagagccccctccctttctcattcccagctgtgatgacagcagaaactgaattctctgagctagcccaacacaacaactgagagggacactgttctccatctcattatgcatatttcaaacatgtgtctctatatacttcttacagaggtggtgataatctgtgaatgccttactgaattttcacaataatattactgtacttgatttgtccccttattttcatctgtgaatccaggtgcactgcagatattagtctgctttctgagggtagggatgacaaataaaatatacaatacgcagagaattggaagttcagataaataacaagtttttagtttaagtatgttccaaatgttgcatgacatggcacccagtactactttaaaaacaaacaagcaaacaaacaaactcacattcctacttaatgaacaaaaatcctctaataaggaggtcacacacacaggattacaggcacaactcaccccccccaacacacacacacatttaccttagagcagagtccaagacacaccaacacacatgatcctcagtccttttaatttaaagcacgttcaacccttctcagagtggccttgagtggttgcctccatgtgtctgcagatgcgaaaaggaacttggttcagggccctaatcagaggcttcctgtcaggacaaggtcctggcatcagcattagctgctgcaactctgaagggcagggtaggagcctgttgtgggactgccccctccaaggtctgagcctgttaattccagggtcagcttcccctaaatctgcagtccctctgctggaggcctgaactctcaatgcccctgcctcccttctgccctgggcctgctctcagctgccacaagagggcgccgaagaaagggcctgaggagacacaggagctcctctgcaggtcctcccaggaaccaccccttctgggaggaaggcttgggagtcccctaagacacatcctcagtcacttctctctgcctgtgtctcaggaataccagctcctcctactgtcttctgtgctagggatcacttccttgttgagtgggacctgagttttgagaggatcttctactccttttcatctggtccctttccttccaaggccccagaaaggaaggcatgcggtgagccctagcggtgcttctagctttcctgtatcctggtgagtgtgctgcctacagagaggctcacaggttgggttttgttttgttttcttcttttgaaaggggtgccatacaaaggaatacctcattatattttatgtttttcccattgcagccagtcagaaatcttccaacttggaagggagaatgaagtcagtcaccaggccgactgggtcatctgctgaaatcacttgtgaccttactgtaataaatgccgtctacatccactggtacctacagcaggaggggaagaccccacagcatcttctgcactatgatgtctccaactcaagggatgtgttggaatcaggtctcagtcttggaaagtattatactcatacaccgaggaggtggagctggaatttgagactgcaaaatctaattgaaaatgattctggggtctattactgtgccacctggggcaggcacagtgattcagatctgccctacaccacactgaacatctgccttgtggctgcctctggtacacaagatagagccgccccctctcatttcctgccaccaaatttactgtattctgaacaagagaaagacagcttaactcctgatctccctcctaatatcacactgtcctggcagcagctgcaccctgttccctacccctcccccacaactttcctgaagatcaagctgccatctccgggcctcagttaagcagcctggctgagagtaaggttctctcagctctcctaggacatgggggaggcccactcactctgcttcctatgacagacaggtacaactagggtccagctgcgaatctagatattttggacagcaaataggaaggttatttatactgaatcatttatccagtcatggtccagagatcacagctgagagtggtgcttattccttatgtctataacaatataagcaatagtataatgaccactaaaacactaggcctaggtatgcagttgaacattctctccctctgccctcccttttattctctctctcttttttcttacttctttgcttgtttttatttttctctccctccctaactccctccctccatccatcctttcctcccttcctcccttgtttccttccatccattctccttccttgttttcctccttccttccttgtttttctctctctttctttcctttttgggtacataatgagaatactttttccacaaaatcatttgaaataatttttctctatttgttcatgccaacatttatacagctagtttaactgttcagttttcatttttacattttggaaatttgttgtattactttgttttgtttcaaatctgttttgtatatataaaatatttacatggaactgaagtcaaaatcataaaaggtgatgcatttgaagattttagcttccattgtagatttcttgttcctcttttctccctgacactacaggtaacaatatttttgtcagttcacttgagctgtttcactctgtttgtcatagcagagtatgtattgtttctatttcaatgccatatttatattttcattctgatatttggtttttatacattttaataaatcttatattttcctgtgtctggattgtgtgtcttacttctaaaggtgcacatacttcataagtatgcataaagacgtccatatcatttatttgaatgtttttatgtgttgattatttaatgatggcatcattgatccatcaggaatttttatacaataattactgtattaataacaataatactggccacgcccggtggctcatgcatgtaatcccagcatttggccagtccagtcattaggatcacttaggccgggagatttggacccgctcagccaacatggtgaaaccctgtctctactaaatatacaaaaaattagccggctgttgtggcgcacacatgtaatcccagctactttggatgctgaggcaggagaatttctagagccaggaaggtgaaggtttcagtgagctaatatcacactactacagtccagtttgggcaatagagtgagactctgtctcaaaaaaatgaataatgataataataatattgatggtacatatgggtgctgacattctggtagttaatgtactaagcacattgcatgcacattttatttaatctacacagaaacttcattaagggtttaaagtaccgttgaatgtaacataagaaattggggggttaattaacattccctaagtcatatactttaatttaataatgatggcaatccaagctctgtggttctgaaaatgagatttgttaatttgatttgcattcccccatctttaggagtactagcaatatttgacaacgttataggtcatttatagttcttcttttgagaatcgccttgtgatactctttgcctattctccttttggaggattaattttttcttattggttcgtaagaattaatatatactattttagagatactgaccctttatccaatgtgttgaagatattactcctcatgtgttattatttacatttggcacctatggtgaattgaactttgaaaaataaaataatatctgtccatttttctagggtgtctagtttgatgccaggcttagaaaggccaatctcacctagaacttctatgcaattcatcatcgtttaagtctaatgattttcattttattacaactaaatcactatttgtaactagtaaggtagaaatgcaacaatatttgtttccatacagtaagtcaataccaaaaagagaacttattaaataattgactatttccttgtgaatattaatatatcactttatcacatgataaaatattacatacatgcagctctcttactgcattttccactgtgttccatgaatcttctcattctagtgccagtattgccctctcttcagcactgtagctttatagttcttttcacattctgatgaagtttctctcatttttttgttttaagaattttctgtgcattctagtgtgatctcaatcctctcccttcccagttttaaaccgtgagacttctgtccagcaagactttttcacgctccaaggcaggcaagcttccctccttcacagggacccgagaactcagctttcagagctgttcctgcggaagcctcatgtcctccacgtgtgctccagaggcagagggagaccaactggagccccttccctttctcattcccagctgtgatgacagcagaaactgcaaaatttgagctaggacaacacaacaaccaagagagacattgttctacatctcattatgcatatttcaaacatgtgtctctatatacttcttacagaggtggtggtaatctgtgcatgccctactgaattttcacaattatattactgtacttgttttgtccccttatttccatctgtgaatccaggtgcactgcagatattagtctgctttctgagggtagggatgacaaataaaatatacaatacccagggaatttggaagttcagatatataacaagtttttagttcaagtatgttccaaatatttcatgacatggcacccagtactactttaaaaacaaacaagcaaacaaacaaacttacactcctactttaatgaacaaaaattgtctaataaagagatcacacccacaggattacaggcacccccccccccgccccccgccacacacacacacatttaccttagagcagagtccaaggcccaccaacacacatgatcctcagtccttttaataaagaacattcaaccctcctcagagtggccttgggcagttgcctccaagtgtccttgcagatgtgaaaaggaagttggttcacagccctaatcagaggcttcctggcaggacaaggtcctggcatcagcattagctgctgcaactctgaagggcagggtgtgagcctgctgtgggactgccccctcctagggctgggcctgctgactccaggggtcagctttccccatatctgcactccctctgctggaggcctgaactctccatgcccctggctctcttctgcagagggcctgctctcagctgccacagagggtgctgcagaactggcctgagcagagaggcaggagctcctctgcaggtcctcccaggcaccacccttctggaaggaaggcgtgggagtcccctaagacacatcctcagtcacttctccctgcttgtgactcaggaagaccagccttccccactgccttctgtgctagggatcacttccttgttgagtgggacctgagttttgagaggatcttctgctcctgttcatctgggccctttctttcaagaccccagagacgaaggcatgtggtgggccctagccctgcttctagctttcctgtctcttggtaagtgtgctgcctacagagaggctcacaggttgggttttgttttggatttttcttctttagcaagggacgccatactaaggaatacctcattatattttatgttgttcccattgcagccagtcagatatctactaacttggaagcgaaaataaagtcaggcaccaggcagatggggtcatctgctgtaatcacctgtgatcttcctgtagaaaatgccttctacatccactggtacctacgccaggaggggaaggccccacagcatcttctgtactatgacatctgcaactccagggatatgttggaatcaggagtcagtcaggaaagcatgatacttatggaagtagaaggataagctggaaatttatacctccaaaactaaatgaaaatgcctctggggtctattactgtgccacctaggacaggcagagtgattcagacctgctctacaccacactgaatatctgtcttgtggctgcttctggtacacaagagagagccgtcccctctcatttcctgccctgaatttactgtattctgtacaaagagaaacagcttaactcctgatctcccccctaatattacactctcctgtcagcagctgtaccctgttccccaccctcccccaggactttcctgaagactaagctgccatctcagctaagcctcagctaagcagcctggctgagagcaaggttttctcagctctcctaggacatgggggaggcccactcactctgtttcttagggtccagctgtgaagcgagatattttggacagcaaatgggaagggtatttatactgaatcatgtatccaatcatggtccagagatcgcagctgagagtgctgcttactccttatgtctataacaatataggcaatattataaataccactaaaacactaggcctagatatgcagttaaacactctctccctctgccctcccttttattctctctcctttcttacttccttgcttgcttttattattttttcttccctccctccctccctccctctctccctcccttccttccttccttttttcatttcttccttccttgcttttctctctctttctttcctttttgggtacataatccgaatattttttcaacaaaatcatttgaaataatttttctttacatgttcatgccaacattgatatagctagtttatttgttcagttttcattttaaaattttagacatttgttgtattattttgttttgtttcatatttgttttgcatatgtaaactatttacatggaactaaagtcataattttaacgaagatgcatttggagattttaacttacattctagatttctttttctctctcttttttttttttttttttttttgagacggattctcagtctgtcactcaggctggagtgcagtggagcaatctcggctcactgcaacctccgcctcctgggttcaagagattctcctacctcagcctcccaagtagctgggatttcaggtgcccgccagcacatccagctaatttttgtatttttggtagagacagggtttcctcatgttggcctggctggtctcgaactcctgacctcagatgatccccctgcctcggcctccctaagtgctgggattacaggcatgagcaacctcaccaggccccattctggatttctctttcctcttctctccctgaccctataggtaacaatatttttatcagttcagttgaactttttcactttttcttattcagaacaagtctttcagtattacagaaaagtcttttgtttgtcatagtgcagtatatattgtttctatttgaccgtcatatttatattttcattctgataaggttttatacattttaatcaatcttttatcttccagtgtctagattttgtgtcttgcctctaaaagtgcatacacttcataagtatgaataaagaagtccatatcatttatttgaatgcttttattcatagactatttaatgatggcatctctgatctattgggaattttaatacaataattaccgtagtaataataatatgctaatgataaacacgggtactgacattctggtagttactgtactaatcacattgcatgtaagttttatttaatcttcacagaaaccccattgaggggttaaagtaccattgaatacaccagatgagaaataaagggcttaactaacattccctaagtcatatactttattcgatagcaatttcaatccaagcgctggggttcagaaaatgagatttgttaattcaatttgcattttcttacctgtgtgaatgctagcattacttaacaactttgtaggccatttatacttcttcttttgtcaactgccatttcatactcttcgcctattcttctgttggttatcatttttttcttattggtttgtaagaattaatacacctcattttagagatattgatcctttatcaaatgtattgaaaatatttctcgtggtttgctattattttcagcaccttttggtgaactgaactttgtgtactacttttaataaaacctatcaatttttctaaggggtctattttgatgttaggatcagagaggcaaatctcacttacaatatgtgtgcaattcatcatggttaaagtctaatgattttctgttttcagttttattacaagaaaatctccatttgtagctggcaacatagtaacttaagaagatttgtttctggccgggtgcagtggctcacgcctgtaatcccagcactttgggaggctgaggtgggtgaatcacgagatcaggagatccagactatccggggtaacacggtgaaaccccatctctactaaaaatataaaaaattagctgggcatgttggcaggtgcctgtagtcccagctactgagaaggctgaggcaggagaatggcgtgaacccaggaggcggagcttgcagtgagccgagattgtgccaccgcactccagcctgggggacagagagagactctgtctcaaaaaaaaaaaaaaaaaaaaattgtttccatatggtaagtcaattcccaaaagagaacttattacataatccagtagtttctcaaggatattaacgtacaactttatcatgtgataaaatattacatacacatggctctctttctggactttccagtgtgttccatgaatcttttcattctagtgccagtattgccgtctcttcagcactgtagctgtatagttcttttgacattacagtggagttactttcctttattgcttttttgttttaagggtgttctatgcattgcaatgtaatggcaaatctctcccttctaatttttaaaccgtgagacatcggtcccagcaaggattttccaggcttcaaggcacctgagcttccctccttcacagtgaccccaagaactcagctttcagagctgctcctgcggcagcctcatgtcctccacgtgtgctccagaggcagagggagaccaaccagagcccctccctttctcattcccagctgtgatgacagcagaaactgaattctctgagctaagccaataccacaaccaagagggatgttgttctacatcttattaggaatattttaaacatgaatctaaacatatttgttatagaggaggtgaatatctgtgtatacactactgaatgttcccaattattttattctacttgttttatcacccatatcttcatctatgaatccaggtgcactgcacatattagcctgctttccaaggatagagttgccaaataaaatatgcaatacccaggtaaattggaagttcagataaataacaaataagttttgagttcaagtatgtaccacatattgcatatggcactgcaccctgtacttttttttttctttttttgagacggagtctcactctgttgtccaggctggagtgcaatggcacaatctccgctcactgcaagctccacctcccgggttcacaacattctcctgcctcagcctcctgagtagctgggactacaggtgcccacccccacaaccggctaatttttttgtatttttagtagagacagggtttcatcgtgttagccaggatggtctcaatctcctgacctcgtgatctgcccacctcggcctcccaaagtgctgggaatacaggcgtgagccaatctcacactcctacttgatgtggcctttttacttgagaatgaacagaaatcctctaacaaagaggttacaaacacaaggtcacacacaccccctcctgacccccacacacccatttaccattgaggagagtccatggccgaccaacatacctgattctcactcctgttgagaggaggggccagctgggcttcctgggtcgagtaggggctcagcaagctgtgaaacgcactcatttcctgcatcacgacttacttcggtcctggatgaataatattgaagatatatgcttaaaatattccgaacaccaggatttgtgcatgtgttttcttccccatgaaagctatgaacagcgaaaattttcctgtaagtttccctgtgttctctctccctctcttccttccccctgccccaaaactaaagtaaaataacgttaactgcccgtttttctgtaaccagcagaccttatctatactcccaattccaattccttgtaaacatactttgtaaagtcctgtaagatcctgtctcctttgccatgacgctgcaaggtcataaagtagataaaacctaagttgcaattccggttttcctcaagatctaagacatgttacaaatggttaattgcctttgtttctcgctttggtaacatcttcccgcctcaggtatttcccgccttgaagagtttaaaaggcaatcctataatctaactctggctacccattctggaccccctccatgctttggaagctttgtactttcactctgctcaataaagcctacagctttttctctctctcggtccgtgtttctatcactcgctgcggtcagccgccacaccaattctatggcgtggctaggcaagaaccttaggtgttacactgttaataaagcaggttcaggccttctcagagtggccctgggtattttgcctccaagtgtccttgcgaatgtgaaaaggaaagcagttgaaagaccaaatcaagcttcctgacaggacaaggccctggaagcagcatcaactgctgaaactctgaagggcagggtgtgagcctgctgtggactgccccgtcctatggccctggccagctggcgccagggtcagctttccccacatctgcactccctctgctggaggcctgagctctccatgcccctggctctcttctgcagagggcctgctctctgctgccacaagatggcgctggagaaggggcctgagcagagaggcaggagctcctctgcaggtcctcccagacaccacccctctgggaggaaggctggggagtcccctaagacagatcctccatcacttctccctgcctgtgactcaggaagaccagctcctcctactgccttctgtgctagggaacacttcctgtttgagtgggacctgagttttgaaagcgtcttctgctcctcttcatctggtccctttccttccaagaccccagagaggaaggcatgcggtgggccccagccctgcttctagctttcctgcctcttggtaagtgtgctgcctacagagaggctgatgggttttattttgttctgttttgttttctcattttgcaaggggtgccgttctaaggagttcctcattatattttgtgctgttcccattgcagccagtcagaaatcttccaacttgcaagggagaaggaagtcagtcaccaggccagctgggtcatctgctgtaatcacttgtgatcttactgtaataaataccttctacatccactggtacctgcaccaggcggggaaggccccacagcatcttccatactatgacccctactactccagggttgtgttggaatcaagaatcagtagaggaaagtattttacttatgcaagcatgaggaggagctggaaattgatactgcaaaatctaattgaaaatgattctggatctattactgtgccacctgggacaggcacagtgattcacacctgccctacaccacactgaaaatctgccttgtgactgcttctggtacacaagatagaccagccccctctcatttgttgccaccgaatttactgtattctgtacaaagagaaacacagcataattcctgatctctcccctaatatcacactctcctggcagcagctgcaccttgttccccaccctcccccaggactttcctgaagacaagctgtcatcttcaggcctcagccaagcagcctggctgagagcaagactctctcagctctccgaggacatgggggaggcccactcactctgcttcctcggaccaacaggtacacctagggtccaactgcgaagcgagatattttggacagcaaatgggaaggatatttatactgaatcatatatctagagatcacagctgagagtgttgcttattctttatgtctataacaatataagcaatagtataattaccactataacactaagcctaggtatgcagttgaacattgtctccctctgctttcctttttgtctctctctctactttcttggttacttgctatttttctacacatccctttttctggcctcccctccctccctccctagctccctccctagcttgccttccttccttccttccttccttcctttcttcctccctctctccttcccttccttacttccttcctttctttcttcctccctctctccttcccttccttacttccttcctttcttcctccctccttctcttacttccttctttttttcctttcttccttttctctctctttctttcttttttgggcacacaatcagaatacagaatcattctctatatgttcatgccaactttgatacagctagtttattcgttcagttttcatttttatattttggaaatctgttgtattattttgatttgtatatgtaaaacctttacatggaactgaagtcaaaattataaaacaagatcaatttagagattttagcttccattctagaattctcttttctcttctgtgtctcaccctataggtaacaatatctttattagttcagttgaactttttcactttttcttatttattcagaagtctatcactattacagaaatacctcttttgcttgtcatatatgtgcagtatgcattatttctatttgaatggcatatttatgtttttgttctgatattctgtttttatacatttcaatcaatcttttagtttctggtgtctggattttgtgtcctacttggaaaggtgaacatacttcagaagtatgcctaaagaaattcatatcatttcattaatattttattcatttattacttgatatgatctatctggaatttttatacaataattactatagcaataataataatactgatgataaatatgggtactgactttccggtagttactgtactaagcacattacatgtatattttatttaatcttcacagaaaccttatcaacgggtttaagtaacattgaatatagcagatgagaaagtgaggggttaactaacattccctaagtcatatagtttaatttgatagcaattgcaatccaagctctggggttcagaaaatgagatttgttcattcaatttgcattttcttatctttatgaatactagcattattttacaattttataggccatttatacttcttcttttgtgaattgccttttcatactgtttgcctatccttctgttggggtattaattttttcttatttgtttgtaagaattaatatacaccattttcgagatattgatcctttatcaaacgtgttgaaaatatttctcatcatttgctattatttattttcagcaccttttggtgaactgaactttgtatattacttttaataaaatctatcaatttttctagggtctgtattatgatgtcaggctcagcgagaccaatgtcacctacaattagtgtgcaattcatcatcgtttaagtctgatttccttttttcagttttattacaactaaatctctatttgtaccttttaagttagcaacccaaggatatttgtttccatatggtaagtcaattcccaaaggagaacatagtaaataatcaagtatttccttgtggatattaacatacaactttatgacatgataaaatattacatacacgtggctctctttctggactttccactgtgttccatgaatcttttcagtctagtgccagtattgtcctctctttgttgtatctgaatgagttagagaaaatgccacactttgagacaaattaagattccgtttatttagccggcggccaagagacggctaatgctcaaaattctctcggccccgaagaaagggctagattttcttttatactttggtttggaaaggggaggggtgtctagttaaaacaattttacagaaataaagtaggcaaaaagttaaaaggataaatggttacaggaaagtaaacagttccaggtgcaggggctttaagactattacaaggtcatagacttggggctttgggcgttatcaatcagatggattcctgggaattgcggatatagcttgccacagtatcttatcagttaattgcattcttggatgtgctgggagtcagcttgcacaagttaagtccttgaggaaggggctgccagtgaaagagccaagatggagtctgtctggctctcttagctaagggagagtcaattcaggtggaaacaaggccaggtgattaaaggaaaagggagagtctaaaaacagggttagtaaaaacacggttgggcattacatcttcagcactgtagttttgtagttcattttatattccagtggagattgtttctctcattacttttttgttttaaggattttctgtgcattctaatgtgatggcagttctctcccttctcatttttaaaccatgagagttctgtcccaggcaggattttcctggctccaaggcaggtgagcttccctccttcacaaggaccccaatgactcagctttcagagctcctcccctggcagcctcaagtcctgtacgtgtggtggagaggcagagggagaccaactggagccccctgcctttctcattcccagctgtgatgtcagcaaaaactgaactctctgagctaggccaaaacaacaaccaagagggacattgttctacgttttatgaatatcttaaacatgtgtccaaacttttttttttttttaccgaagtgaaaatctgtgtatgcactactgaattttcacaattattttactatacttgttttatcacctgtatctccatctatgagtccaggtccactgcagacatcagtcagctttctgaggatacggttgctaagtaaaatatgcaatactcaggaaatttggacgttcagataaataacaagtttttagctgaagtatgtcccaaatattgcatgacatggcaccctgtattactttaaaaaaaaaactcacacttctacttgaatgaacggaaatcctctaataaagagatcacacacacaggcatacactcccaacacacacacacacacaaactcacagaggatcacacaaacacccgccccacccccacacacccatttaccttagaggagagtccaagacccaccaacatacctgaccctcgatcctgttaataaagcaggttcaggccctctcagagtgaccctgggtgttgcctctagtgtccttgcagatgtgaaaaggatggtggtttagggccctaatcagaagcttcccggcagaatgagggtcttgcagttgccttacttgctgaaactctgaagtgctgggtgtgaacctgctgtgagactaccccctttaaggtctgagcctgttaactccagggtcagcttcccccacatctgcactccctctgctgcaggcctgagctctctatgcccggagctctcttccttagagggcctgctctcagccgccacagagggcgctggagaactggcctgagcagagaggcagaaactcctctgcaggtcctcctaggcaccacccagagtcccctaagacagatcctcaatcacttatctctgcctgtgaatcaggaagaccagctcctcctactgtcttctgtgttagggatcacttccttgttgagtgggacctgagttttgagagggtcttctgctcctcttcgtctggtcccttacttccaagaccccagagaggaaggcatgctgttggctctagctctgcttctagctttcctgcctcctggtaagagtgctgcctacagagaggctcacaggttttattttgtttcgttttgtttattttcttcttttgcaagggataccatactaagaaatgcctcattacattttgtgttgttcccattgcagccagtcagaaatcttccaacttggaagggagaacaaagtcagtcaccaggccaactgggtcatcagctgtaatcacttgtgatcttcctgtagaaaatgccgtctacacccactggtacctacaccaggaggggaaggccccacagcgtcttctgtactatgactcctacaactccagggttgtgttggaatcaggaatcagtcgagaaaagtatcatacttatgcaagcacagggaagagccttaaatttatactggaaaatctaattgaacgtgactctggggtctattactgtgccacctgggataggcacagtgattcagacctgtgctacaccacactgaaaatctgccttgtgactactcctggtacacaagatagaccagcctcatctcatttcctgcccatgaattcactgtattctgtacaaagagaaacacagcttaactcctcatctctcccctaatatcacactcccctggcggcagctgcaccctgttctccaccccaccctcatgagttacctaaagaccaaactacaatctcccagctgtgtcagccaagcagccttgctgacagcaaagttctttcagctcttctatgggctggtggagacccattccacctgcttcctaagacagacaaattcctcaaggactggtctgtaaagggattcatttaggagactatatgggaagactagcttcactcaagcatttatccaattattgtctataggctaaaatagtgcttattcattgctcaggataaatgttggaataacaactttgcacttcagtaagacatctaacgtgtatcagatctgctatcttttggacacactgacatttttttctacataacaaatcatggtactattggtctgcaggagaatgggtaaaaaagtgatagtcataggtacgccaacttgtgggtcatatcataggttttcaaccatttcaagcatccctgccctaatgcaagtatctgaaggatctgacccttgccctgcagcagaattcattccatgtcccctctggatattagactgataatttggatcaggtctcagcatgggccattgaggaacactacagccctgctgagagataaaaaggattatccactcaaggagttcacacctccgggccgacatggagaacgtgcctagaagcagacttggagggtgctcagtggtgggttgtggaatgtaagcctgaagaagcagagtttaattctacgggggtgctttcataatttagtaccctgacagggctcctggtgttggtccttagacactcctgggatggctccctggaaacatggaggaaaccttggtcgcatgacatgatacggagatgttggagctgcctggacacagttacagagggaggcattaaaaggcttcgagaggtaggcatgctagagtggactttcccactaaacctgagaactcactggataactgtattccctgcgagagcccagagaaccctctgaattaggaaagaagggcatgttctgaaatgggaggaatcagcgttcttgagagtcttggtggaagctgtgccctgtggggcagggttgactataggagacgctgttaaggaattagctcccaagggtcaatggagatgatgtaatttcaaaataagagtccaaatgggcagaattagtgtgagaagacataaagccagaaaagcagccaaggagccctgctctacagaaatctggggtgacagctaataaaccacagtgttcctaggggtaaggaaattgggctaccacagtggtattccacatatgtattccatatatacatatatatctctcccatatatatatatatatatatgagatatatatatgagatatatatgggagagatatatatgatatatatgagatatatatgagatatatatgatatatatatgagatatatatgagatatagatatgtatatctctctcatatatacataatacatatctctctcatatatatatatatatatatatatatatatatatgtaattggaacgtattaagagaagatgaatgaaagaatgatgtcagctcctcctgttctccaactcagagtcctttgaatgaaggggaaggcagattgccttgagggagaaccttgtaatgttctagcaagtatatatggcagtgattctccgagccttttcccccaaaagatcgaagactagttacctgagaaatttgtacacctagggaaggggaataactaggtctttcaaggctgttggagacggcatctgagctaactttgataccaagaaatgcatactgtcaacgtggtcccccattagagtgaggacacatagaagctccccctctaatgctagttttaaaggcccaagtctatctaaaagggcagtcccataggtggatggactgactgtggtctctaccctgtgtctgaggatatcagagtggatatgatgaatggacataaaataaggaggctgcccccctacccccggatagtccaggcagccttcattcctttatttcatttggaacccatatggcttattctctttcactgactggagctcacagtctggctattgtaacctgtcttaaatctttttctctttaaaatatcttgactttgaggcaggtcttagaaaatgactcttcctgtctcaaaatgcagtccttcattctgattgatgaattggaagcacatggctggtgtaaagaataagaaactaattataagccaggaaacagcaggagaagaaagcagagaagcaacgcttaccctgaagaattaatttccgtttagaaaatatcacagctgatgtgtcaaaggccccggtatgcaggaatgagattaaacaaatgtggtcatgaggaagaggtttctgaataatgatagagaagcttgagtctacaagaaatccagagtccagaatactgcaggggagcagtgctgggttcatgtttatctggtctcttgtctattggatcctctttcttccagaaccctaaaccttgaatcagccttatagtcctggctcctagaagagtgtttctcaaagtgtactccacggaccacctggataagaagcacgtgaggcttttaattaaaaaaaaaaaaaaaagtacaggttctgggaagcatccaacacaataagacagaatcttggaatgaagggtgaaaatgtgcattttaaaataacctccagagctgattcttattcaaactgacttttaaaaactgctgcactagtggcaagagatcgaggggctgtcctgagcctgacacagaaaggtgttctagaaagctgctcacaggctccttcgcagcccaccaaatccgcctcactcttatctcccccagcccctcaaagcagctgctttgacagtttctcacatttttgcatgataatcccacaactgcaattccttctggcttcctgtgacctcacgcaagaaaaagttgtgtactaaatgaatctgctttaacttgctctccttcctcggggatcacacctttttaagaaagcctgtcccttaccttgaagcacaaacatattctcatttttattctcccaataccttgaaggttttcttctgcacatgtatttgtttgatctgccttttgtgcgtggggtgggagttaggtaggaatcttaaagtggagagccagtttcttcccaaattactgacctaacccatccttaacccccagttcaaggccacctttgtgatagtgaagcttccacatgctcactcagccccttctgctctctcttcttctctactgtgcatgtcggcttgtacttttgccagtttctctaaagacacaaccagaggtggggtggctgtgtgtgcacaacttcaactttacatgtggggctgagtccctatgttgtatatccttgtgcaaaagcacaatatgttaattgctatagcttttaaaaaaataattaatagtttttcataatcaaattttcttgcttttttgttttttcaaaaaagcatacttttattgaagaataaaccccttatatatgtacacttatttataactatgaaccatgaactaggatagaaatgcattgtgtatattacaaaacataacaaaaataataggggtagggaggtgcagatgttggtcaaaggatataaacctgcagttctatgatgaataagttctggacatctggaatacagcatggtgactatacttagtaatactatattgtacacttgaagcttactgaaagagtaaatctcaagtgttctcaccacacaaacccaaaggtaactatgttctcaccacacaaacccaaagggaactatgtattaattagcttgattgtggtaaccatttcacaatgtatacatttgccaaaacattatgttgtatacctggaatatataattttatttatcaattatacctcaataaagctgaaagaggggattactaattcccacaaaatacagatttaacaaaaacttttattcaacaaacagtgctatgaagttgtaaattggaaacaaaagaaataaaatttcatccacagtcttctcatcaaaacccttcagtggcattcctctttctggtgtcccagtcttgtcaattttgctaataactgtcatcctgggaatacccaatttatcctacatgacaaaatgacaaagtctgattagatgagttctcagattctagcatggccagaagagcactgtcctgggtcggataaatcacgtggaagatgcaggggatgcgtgactttaaaggtccagcccttagtccctggatcttcatgcaggggccgcctcagcctggatctgctcttcctcaccactgcagccctatcccacgctggctgaggtctgcttccacctgggcagtgactggatgacatgggatgagaggacacacctctccctcgcccagcatcgcatttctctttccctggagatctgggatcttggtcagaatccttcaaacgccacccagggcttgagagggcaagccctcctacaccttgactgcgttttgcccaagatttcccccatattattattttaaacgtgtctaatttagacaaatagaacctgtaagtgctacattgagaagagcacagggccaccgaattgggaagacaagtagaggaaaggaaagcaaatgtcaccagacagaatgtatggctgcaggtttacagcagattctattaaaatctatggttgggctgggtgtggtggttcacccctctaatctcagcactttgggaggccaaggcagagagatcacctgaggtcaggagttcaagaccagccaggccaacagagcaaaaccctgtctctaccaaaaatacaaaagttagcaaggcgtggtggcacgcgcctgtaatcccagctactggggaggctgaggcaggagaatctctggaacccaggaggtggaagttgcaatgagcagagatcacaccactgcactccagcctgagctaaagagtgagaccctgtctcaaaaaacaaacaaacaaaaaatctatgattggctgattggctattgctaacaacttttgagtctttaatgatcagtaattgaattaaaacggttaaaacaacaattgagagaaacatagttttgaacactgacaacacaaaataacttatccatgtaaccaaaagctacctattcccccgaaactattgaaataaacaaacaaaaaaattagaaagcggaaactttacaaaaattattctcaccaatgaggttgtccaaatgtcaccaaatttattatagaatagtaataaccaaatttgtgcatgaatcggtgatgacataagtatcttgtaagcattactgaagttttttttttttctattaaatttaccttcaagatatgccttcaggatgaggctttccactgcacttcattatgcaatgccatgttgacttggtatattacctcagatgtgactctaatatggtttgatttgttatgacgagactaaaatgaaacatatcacttttttcatgtgcatattgcaccttataagcacaaggtgcaattaaataaccaatttgaatattgaaaacatatgtagttgttataatttttttctcctctaaaataatattttcttatttctaaaaaaatctagaaaatagagaaagattgaagacaaataatttgcccatttccattgctcactgtctgtattttgcactttctacctgtcatttccctgcgttgaccttttctgaccatagctgtcactttctttcccattaccctagcccacccctgggctaaaggtctatagagtgtataaatgatagccccagaatatccctctgtcaaaacgttctgctagctttgtatttgaccaccttctcaccaactcagcacaaccctaagccctgcatgtgagaatgctgaaaactggaatcatgactttcagtttttgccatcgaagagaagctcaggaactgggtctggtcgtgggagcccagggactcacagcttcccttcccaagccagaccccttttcttgccatgcccacaaccttcccctcatggccatctctttgactactcaggaggtcctgggtgtcattagcaaagctgaaaatgaaccttcatttcagtaggaactcaaggctgggtctatttctccaagcctttggcaggtgtgtccttcgctggcccttcccaatgcacagtcttcaccatttccaaggacgtgccactggcagaggatgagctggtcctgcctccaggccctctctgtctgctggcctgacttagccttcttcctttggagacacacacacactcacacacacgcacgcacacacctggttcttgaaaactgcattagtccctataatttctactttgtgtgaaccccagagatcatttactggaacccatccagtttccaggtgaaacaacaacaccccacatttcttgagcatggtctatgcagctgggattgtgctgcgtgctctgctcacattctcctgtttactgtccatgtggccctatgacacctctctttacagatgaggaaaaagaggtgaaacaacttgcccaagactacacagctatcatgttattttagggcactgaaaatctccttctactaggacctctgggtgacacgctccgatgctggctcagacggttggcatgggtttttttagggattgctgttttgtgtttgtcccttcctctggagcaagcagcacactcattgttctctgagtataagatggttacatgaagcagaaatttgtcaccagcctggcctggcttctctcccaactctgattctctttaggtattacagccttggaaaagctacttaaaataacagccttactccttcatttctaaactgaagataacatttgtcctatagagttattttaggatttaataaagcaatggccctaaaccaattagtgcagtgcaagagttttgctggtgtccaaccaatgattgctattattgctaattataccagcaacactctttaagcctttttcagcactctagccattggtcatccctcccttcaccttgtggtcagatttctgtctctcctctggaacttctttcttcctcccccatttctctcatcagttacctccttgcaccaccagggaaatagcagttcaggccctaagctggtcgctaccataactcaggaaagtgtggctcaggtccatagtttgaaacaggtcactctgggctcctctcccccagtcaggatcagagatatggtgggctgccctgccttcctttgggtcatcctgtttccaggtcagtctcctacctaaggacctgtgtagaggtggcgaggctttgggacatccctacctcactgctctctccctgacagctggctggtggctcatcaggccggagcagctggcccatgtcctggggcactagggaagcttggtcatcctgcagtgcgtggtccgcaccaggatcagctacacccactggtaccagcagaagggccaggtccctgaggcactccaccagctggccatgtccaagttggatgtgcagtgggattccatcctgaaagcagataaaatcatagccaaggatggcagcagctctatcttggcagtactgaagttggagacaggcatcgagggcatgaactactgcacaacctgggccctgcgcagccttgcatgctgccccagccctacacaaaaggactcttcctcccgatccaacaaggccttgggcattttcacttactcttggtcccttgggtttccctgtggcatagaagaaaaaagtcttatcccctgtccctcacctccccatctatcctggaggtcccttccccggtcccactacagatgaggctttcagcttgtgcagactcagtgatctatatctcatcgaaaggggtctgtttaaagatgctccagttcagtgtctctgaagcctttgcaggatgacctgtgctcctgaatgcaggtgccactagccacctgtggctattgagcatgggaaacataccaagtgcaatagtccaagctgagatgggctgtgtgtctaaaatcatattttgaagctttagtgttaaaagtgagataactcttataatgatcaaaagttgaaatgattaggtatcttggactaaagccaatagcattaaaactaattttacctgtttctctttactttttttaatgcagcaactaaaaaaattaaagtgtgtgactcacattggtgactcatttatttctgttggacagtgctgttagagactgatcatttaagaatctgaccatctcccctgaagaatgcacaaataaaatattttggaagagatttcaagggtggaggacttgctgagatttaccacaaaatggttgaaaagctgagactagaagcctactcctgtttccagcttccaagctcttggccctgggactgttatcattttgcaatagagtcagcaattagaagcatgggaaacatgactgcccacttctcagtactttcacccgtgggcgggctgcataggaactgatgtgagtagacagtcgccatggcagggtgatgcagtcctccctggatgagacatttaccttccacttctccttcaacagcaccccagtgtggaacacgtgtgtatcccaagcttctctagacttttgttctcctatctgacaaatgagggggtttagccaaatgtctgctaagttatatgactatgatttttgtattaaagcaaagccatacacataagatcactatgcccactaccttcatataaagcagtcttttttaacatagaataaatgaaagaaaaaaaaagaaagcctgtgttactgatcctccagcaccaaacaggaaacccctctgctgctctatgtgcagaaaaaaaagaaattctttgaagtctaagctgaatttaaatgccttttcaagagaatgcttaatacactgttgatgagaatgtaaattagtacaacttctctagaaaacagtatggaaatttctcaaagaactaaaaatagaactaccattcaatccagcaatcccataactggatatccacccaaagaaaaataaatcattatattagactgcattcatatatttatcacagcactgttcataatagcaaaaatatggaatcaacctaaatgtccattagtggatggctggataaagaaaatgtggtatatatacacagtggagtactattcatccataataaatgtggtatatacacacaatggaatactgcttatccatacaaaagaatgaagtcctgttttttgcagaaacatggaggaagctggaggccattatctaaagtgaaacaactcagaaatagaaagacaaatactggatgttctcacttataagtgggagctaaataatgtgtacaagtggacatagggtgtggaaccagacattggaggcttgtaagggtggtggggggcagaaggaatacagatggaaattaagtaatttcacatcacaatgagtattatccaggtgtggggtatactaaaagccaagactttaccactgtgcattatatgtgtgtaacaaaattgcacttgtactccttaaatttatacaaataaaaaacaaaaggagaatcacttggacccaggaggcaggggttgtggtgagccgagatcgtgccattgcactccagtctgagcaacaagaaataaaaaaaaaaaacgctacgccttgcttctgaaacagcccagcgtctctaacctctactgaaggctcagttcacggctaaggccttccaacttgtgtgagaaggacagaggccatacaggaggaaactttcattctgttttggagttgttccttcatttcatttttctaattgtgctgataaaaccaaatgggcacagagaggagatgcctcctcttctgcctgccccctctctcagtgctttactccaaacaagagtaaatttggtgaaatggtgactatcagggtgtggccaaatggaggcgcaagctccccagtcacctccttatggaacaacatctttcatttcctcaagaggagactctgccactgcagtgaaccttcaccaccacaaacctccaccttcactcctcaccaacacctgctgtactcttcatgaatgctgtgagcttgagcgagttcttaaatttcctagccatcagtttcctcatctccaaaataaagaaaacagcaatgtccaaaatcaatctccctctgaattatactacctggtttcagcctcaacctccagggtgatagaccagcttagagaccaagattttatctttcctaagtgatctcaccttcagaggcatcatcaccagacttttcaagttttgtttcttagaaatggtcccaagttctttccctctcatcgtctcttgctttagggagcctcccagctagtctgtcttagcaagacaagggcatagctggtgcattgctgctggtgagcaggggcaagttcacagaaggcagcatgggagagtataacagaaatcaccatcagtttccaagggcttgctctgtgtcaggcattgccctaaacagtctacctgggcaaacatttattctttgcaacatccagtaaggtaggctgtgattttattctcctttggtagataagaaaacagaggcagagagaactactcaaagagctcaggctttgcagcccgatagaattaatcttaaatctgtcaccaacaagctgttaaaccttgacccattacctgacctgctttgagtagggctttgtgaagattatactaaatttatggtattaaacatcataatggctacaaactgcttgacacattaaggcattcactaagtgtccattgcttggtaactctttaaaaactgtattttaaatggtgatgttttgttaacatcagaacgacaaaaaaatactacaatggccatccattccctcactccaccctttcatctattcaacaaacacctgggaatagagagataaacagcacatgatcttactcccctgggaactcttaactgtcgtttagaatgagagagaaatgggtaaacaggccaagacttgggtaggaggtgctaggagagaggaaggcactaggtggcgtgaagagaaagcaatttgaagcatctccatcctggacttactgggtgaggtaagcttcctggggaagactgcctggggctgagcccagaaggataaacaggaattagccagggaatgtggagtagaatgcagtccaaacacaaaaaaattcaagtcaatccatagaagtgggtcgtggaattccaggcagaaagtgactaaatgaagatggaaggacagggagggggtggccacatcacagagaacctcttatcctaagaactctggacttcatcttcagaggcaaggtagagagagcaaggactttagagcaggaaaaggaccaggtcagtctagtggccatggggaaggtgggtgggaggggccgagatgggatgtatggaggtgcgtgaggtggaggcagtggtgagccaggaaatgtttaggacgtagaatcctcaggaattagagtgcggtgaattagaggggagaattgaggctgatgctcaagctcctggcttgggcaatgtgggtagttatgtcatacagggaactcggaagaagatatggtttgggggaagggaatgagttcactctggctatgagcagactttgtttgagatcccatgtcagacgtacttgaaaatgtccaagagttagctggatatgggtacagacagctttcgatttaactgaggtccgacttaagatttttttttactttatgatggtgcaaaagtgacacgcatttggtagaaaacataatttgacctttgctgtttccccaggacagtgatataaggttatgatactctcttgcgatgctgggcagtggcagtgagctgcagctcccagtgggtaaattaagcatggaaatctggaacacagcagcttttaagggatgcactggggagagcagtttgtaaaaataccttgggacggattaaatgtcttggcttagagaaagaacaacagacaataggaaactgtcattgaggagaagccgggattcaggagatgtacattattcaggtagctgagggaggggacaggaacctgaatcttcaacagaagcaaacaaactgggatggagggcccagcctcatgaaggtgaccagaaggacccggtgctgcaggctgtgtgggtagctgagcagagctaagcggcttgacggaccaacatctctccagctggttgaagacaagctctcagaagacaatgctgcatgtcacagccccagcaaccaacaacaccagcctgacaacttgctggggtggccgccttgtggtctgaggtggccgtctaaactatgtggtctgatctcaggctgcagaccttgcaggactgtcttcacacagactggaagtgctaacaggtggtgaggacaccgctttacaacgatgcagggggccccatgtcaccctcacccatgggaagtttgacttggtggactcagccaagccacagaggtctaacgcttctctgcggtgatttcaggctgccctggcagaaagcacagtgcctgcagacatgctgtcactgctccacacatcaacgctggcagtccttggggctcgtaagtagttttgctcccccaatcactttggactgatattctctattgttatatatttttataaattccaaattcttggtttatttactccctcccatttttttccccagtgtgtgtatatggtgcaggtcacctagagcaacctcaaatttccagtactaaaacgctgtcaaaaacagcccgcctggaatgtgtggtgtctggaataacaatttctgcaacatctgtatattggtatcgagagagacctggtgaagtcatacagttcctggtgtccatttcatatgacggcactgtcagaaaggaatccggcattccgtcaggcaaatttgaggtggataggatacctgaaacgtctacatccactctcaccattcacaatgtagagaaacaggacatagctacctactactgtgccttgtgggaggtgcacagcagcagacagtttgagccatcccattcaataaatgtttattgagtctttgtttataattacgaattgggaagccacagttaccaccagtgtgcttgtaaacagtttttaagataaacattcatgtggtgactctacttggagttgccaaattccacatattttctcaaagcagaagctttgcataagtctatacaagtgaccagcctcctctttttcagggttgtactctctcaccaacagcttttctaggtcacccatgcttatttttctggttcaacctctcctactcattatatattttttttctggtataatatatacacatttttagtgtgattcttttgtactagtcaatatgcattacataagttttctctgaccttcctatttctctcgattaaaaaatggatatgacattaaatggtattcatttttctggaggttaacatgtaacaaacgcagcatgatctaaccacgagcagggcagactgcaatgacaaatctatcacatgcatgccttgagtggtgatgtttgattttgtacaaaatccgtaaacacttccactaatcgaatctaagtcaaagtccactttggattggggtttgagaaaaaattcatttgctgcaacctctgcctcccgggttcaagcgattcttctacctcagtttcccaagtagctgagactacaggtgcgtgccaccacgcccatctaatttttttgtatttttaatagagacggggtttcgccatgttggccaggatggtctctatctcctcctgacctcgtgatctgcccacctcagccttccaaagtgctgggattacaggcgtgagccaccgtgcctggtcatccaaccatgagcttttgatagactactctgagccaggcattatgcacagcagaaattacaaggcccatacgctctgcaaaggcccgaggttgcttctgttgaaccacattctgctactgggctgccattcaccactaaaatggcagtcctcaacttgaatataactcatgattgtaagtctcttatgaattttcgttacttctagttcaactcaggctttgcaatttattattgttgatggtgttgttttaatttatgtttttgccatgaaaccctttcttgaaatgtgatcttacaaatataaaatagagaaaagtagatttccactgggaaagagttcagagatgaatgatccttagtctcatcttctcaaatttctctgatactttgatttttcaacagctcaataattatctgagtatacatataatgtacaaagtggtcaagacctgggcctgtcatgtcagaaggacataggtccaaatggggctctacttaccacggataagctgtgtggcaaggccttgagcttctctagccccatttcctcacctgtgaggcaatggtcctgtggttatcatatgggtggctgtgagaactcctgacatgatgcatttcaaggatttggcctagtgcttggcatattgtgacagcccagcgttatctgacaagagacaaaactagatacaacaaaaaaataacagcaagcacacatatatagtcatgtgtcccttaacgacaggaaaacatcctgagaaatgcatcctttggcaatgtccttgttgtgcagatattgtagagtgcccttaacacacacctacatggtacagcctactacatacctaggatatatggtatagcttattgctcctaagctgcaaacctgcatagcatgttgctgtactgaatgctatatgcgattgtaacactgataaatatttgtgtatttaaacatagcatagaaaaggtacagtaaaaatagaatataaaaaaaatgctacacatgtgtagggcagtttcattataatttgtccatctttgactgaaacattattattcagcgtatgactatatatacaagaaaacatacacacacacacacacacacatacacacatctggtttttttttttttgagatggagtttcactcttgttgcccaagctggagtgcaatggcgcgatctcggctcactgcaacctctgcctcccaggttcaagcgattctcttgcctcagcctccaagtagctgggattacaggcacgcactaccatgcccggctaattttttgtatctttagtagagatggggtttcgccatgttggccaggctggtctcgaactcctgagctcgtgatcaccccacctcggcctcccaaagtgctgggattacaggcatgagccaacacgcctggcccatatacacatctttatatatccagggcttagtgctacgtctatcatagtgtggctattacattttatagagagaatagctaagtatgaagaaactcttacaagaggttatcccagattaatttaattctaagcttttggtcatggttccctaagacctttgactcacacacagctggacaggacagtggccttgtgcatagtgcagatgaccattataggggaaaaacaagtcgaaattcatagtcctttactcctcctgcccttctccttttgcttaaggtgagcttcaccaggaacattttcgccacaccaaaggaaaactagccagaggcaaaccagctctaagttaatatttgccaattaaatggtttaagttttggattcacagaaacactgacagcatcttattagaatatactgtactgcatatagtaggggctcaatgaatatctgttgaattgagattgatactttcattattattgatgggttcattttacctaatgggtcaacgcgttgtatggatggatgccctgaatattctgatgatttgggttcgacttcttttcttttctacctgaggtgggtgagctacaatgactctgaataatagaatcaacattatattatctagttaatataaaatctgaataaaatctaaggaaatcttggaaagcaatattttcataaaccatatcatctgttgccgaactccccacacatacaagtactatggaaaaagtaatgtctactgcccaggagtcatcttatagaaaccacaattctagaagttgctgtacccacctggaaatccatgctgactgttttgtctcgggtgctttttgctttcagtcctgtgaaggggttcacaagaggcagactggggtagacaaaaaaagggcacagactttgaaatgcttatctccagacattgcgctcatgagtatttttatctgtgtcatttctgtacttttgaaatggtctaatagaaaacacattactttttaattttattttaaaattgacttaaaaaaagaattcctgttttataatattaaacatatccctgcacattattgagcacctagagacaatatgtaaaatgtgttggttagaaggacctggaaggggctctgcttgactactttttctttcctcttctctaacaacgtttgcttcttgtaaaaagcaaaatcttaccttttctcctgtttcctactgatcactgtgctgagctaaagaaaatgttagtgatttgaatgctcaaggcagcttattgggcttgtatgtcttcctggaacactaggatttttcaagcctgtagatcaaaggtcttgggaaaaaagaaacaacttttttcagtgagctaactgaaatagaagagaatggcgactcctacccacacctcttggatcctggacatcagctctggctgtggggcaaatggcactgcatattggccaatgtggggaggatgcagccaacttaaggccccttttcagggagggaacgctgaccccacgctcctatttcccagctgcctgctgatgtttccattttctacccccaaacaacacctgcaggatagggaagaccatccatgcagcccagggcggtcagacttttaaggcagagttatgtggaaaatggacttggatgagccaaggaggaaatcctgcagatggcccaataagtggattatgtttgacttcagataagtaggacaagctagggagccagaaggttttattagttttgtttcactttccacaaaaccaccaaggtcccatctccaacagaacaggatgtgtgactgttccttgagtaaaaaaacaggaaactggacaaatcttgagagatcatcattaattagtacttctttagttgatttcttaatatggaggagcatgtagattattaataatgcttttgttcttgagttaagtgaaggagtcttaggtatttgttgactcattaaataaatcaccaacatgtagtagactcaaataagaaacataaaagtgatacacatttagataaatgattatagtgctttatgcttgtagtgcttcatgaatcgatagtatgattaatccaattgtgctcgtagtgttctttacaacaactaagtttaaaatagagaaacaatctcaactctcattagatgattgaggatagagaaatgcctgtcacgttcatgtcaagtagaatttatcccctcacccctgttgctataattgatgtgtctcttctgtagatccctaatttaatttcttgtcacttttaagtcaacttttaactagcaaattagcaaagtgctaagggattcagagagattgaatcacgtgctatactttactgtagtcccgttctctttatattttacttataaactaaagttacagagtaattatcaaaactccatatttgtgttctgaaattggcagaatttgaatttgcagtccataggtcagcagatttctctgactttccttattttctttgcttagccacagaaaaacagaaaaatcagtgagtttacatgcacagaattaaatgtacagactattctctgaaagagctcagttctatgtgaaaatgaataatgtaataaatattcttatgagtgtagtaatagtagctattgtttattgagtacttcttatgtgcatggcactttatactgcatgctttatgtcatttgagcctaacaaaatactatcattattattatctcatttttatagatattttctttttttaataaactcttttatttgcacgtttgtgtcttgggttattcgtggggtgagaaacctccacacttccaatcccagccatctggtacaatctggtgttgtggtccagctgtcggcaaagggtagaggtgggtgcagggctggccccccagtctgcaccaacctcttcagagcagggagctcagaccatggttgtacttgcactgcttcagggcctcgctgaagccttcacacagggacaggtcactctgcgtggtcgaacagtccaggaactgccggatctcgtaggcgcaggaccccatctgcaggggctggggggcagcgcgtgtgggggtctgctgggcagcaggctggacgggctccgagctcccccatctgaaggctcaggtcagggcgctgcccatgacgtgtcccacagccgagcccacggctacccctgcggccatggacgccatctaagccatgaggctcggctggccggaaggggcggagatggggcggctgccggaggcggtggctgtgtgggggcaggtgggcagagggcgcggcgggagggggctgggtggtcggaccgccgcgctgcggcttcccagagacatggtggcggcggagggacccgggcgatcttaaatgacagcgatggcggcagcggttctgtcgcggggacaaatgccctttatagatattttctaagtacagatttgagactttgataaattaagatacttgatagtaagcagcgaggctgggatctgaatccaggtctgtctgactacaaaatctattgccttgatctcctacagtgatgagaaaaacaaaaccaaacacgaacttttaaatagagacatttcagggggaaataaaaaaatttataattcgttttatgagttttttttttttcatttgcggccttaagctcctttccccagggtcacatgaagttagttaaattgatgctaacggtgtttacttacagacaatctgcagagaattctctacagagaattttcttatgcaatcaagtttttctgacttctgggttctaagatttttttctttttttaacaagaaaaaaaagcgtaaccaaaactgtgtttattgagcaacagaaaagcagcgagatggaacacagagatattccccctgattatcacctttccgctgcactcccttaccctcagtccgctggggagcacagaaatgttatccaaaggtggatgggaaagggtggaaaggctgagacccaactgcagcctggcctgagatggccacatcatgttctgcttcctgcctggctgcccagggagggcctggatgggcagagggccaagtcagtgtcaggctgggaactttacatgcttttctcacttaaatattgtcatctcctttctcagaggaggaaccagagattcagagagactctgtagcctccaagatcacgcaggcatcactagtagcagagaagggatgtagagcaagtgtgacggtccataagacttactctcttcccaccacaccacactcacccagcaagaactggaataaatgacaagggagggaagaggggctcagacttctctgtatattcacaaggatgtggaatgtgttcctgtaagcgtacccaagttgggaatttggtcctttaaagaaaaaggttgaagcaggaagacttccagtttgctggatgaaacataatgcagcaatcaaacagcccgactcttttgagtgaatatcaataggaataccactataccattcacttgttcttcaaaggaaaaaatgaaactaatgagtccttgattccatgacatagataaatgttctgagaaggaagaagttaatggatcactgggaaggcttcatagagccagaagattcaagtaaaagtcttgccaaacaagaaaaggagaaagttcatttttgtcacagtctggttgcaacagtaaaaactagcttttgtcatcatcacattttctaatatcgaaaggacatattttaggaaaaagcatcccaaatttataggtatgttgttatttatagaacttcatttttttaaatcaaactcttcagtgaattaatttttaccacctcctcaggtacaggataaatgggacatttgcagccagtttcctccttgcccatgtttgctgcgaggtggggcgtggatgtggggaacctctctgggggaagaggatgggtgcagcagcccgacgactggtcgtgaggccccaccacaaaaagcctccacttaaagggcaatgctgagagccccaccacacctcatgatggggaattcctctgtctagagatgttatttattgtcattcaagtcaaggaactaaaatcctaagaaaaagagcataccccaaagccaaactaggcctcctaacagtagctctgtgctcatcctgcttcaacaaggaggcagagtagagaggaaggaggtgaaagatatggaacccactgagctcccactttattccaggcgtattatgcacctatctaagccaatgctggtagatagggatttcaatttcattttcatagttgagggcactgggtgtcagatagcaacaagtcaagctaacagcaggctgaactggaattaaaagcaggactgaatgattgcatgctcgcctgtatagcacactacgtggatttgcttggcattgaagaaataggttttagttccagctctaccatttactagctgagaggccttacattaccccctcttccccatggggaatcccttcctgcctcaaaatattgtttggattaaataagccaatgtttgtaaaagagttttggaaattgtagacaccataacaaagtaaagagttatagttttttttaaacacattttcattcattctaatatgatttctcatatgaattatctcctaaggatagtcaatatttatggagctcccactatagggaaggcatccttcttgatgaaataaggggctttaacaatccctacaacttatgactttgacttaacaaaaacgaaatctagcatgtgttatatgaaagtagcaggtaacaagtggtctagcaaagctgcagtgctatatgctgagtgatagaggtatttgttgtaacatccactccaattcctcaagaaaatagatggtggcaaagaagattaagtgatattgctcattaaatgatgagaatttttacatactggatattcagtgggagtttcattttgtcccaatctccgctgacactctaagctcaggagaatggtagtaatacaaaagaaggggacaaaaccagagattcacagtggagggcaagcccctctccagcagacattggtaatgtctgagacattttttactgtcacaaacagagtgagaatgctactggtatctagtgagtagaggccagaagtgttactaaacatcctacaatgcacaggacagccccacaacaaagaattatccagcccaaaatgtcaataatgcagaggctgagaaaccctggggtagttggccatatttctcaaagacttgctaagaggtagacaaaactgatgactccaacctttggctcatgagctatatccaggctaattacagtaagagctttcctggggactctaattttgcaaagactttctctgaaaagcactgttgggatttccctggaaaccccctcctctcccagtgaggaggtgatgaggtagctcttctacttccacaccaaataggactctcaggtcctacatccaccatgggtccagagcagagccctgtgtgtgggtcatggaagtgttgggtctgtgccgtgagcgtttggtggccagataaaccagtgaggactctcacctggaaaagtggacaggtggcttcaggtcatagcccacgtggtaacttggaccaactctcccctgaaatcagttagataatcatgatgaaataataataatgaaaaagaatctttctaaaagtttctaagagttagcaagataacaaggtgaataacttttaccctggcaaatggactgattatcatggtgtcatacagctatgggtaaagttcccatgtgatcctgaccaatcagcaacctcagaaatgactgatctgggcgcagggcctaaggacacccattttctctgtgaacactctttgaggttccccttcctcatcctggtgcagcttctcctgctccaggttccctatttcctcagccttgtctcaggcactcagcctgagcagacgggacgtcacagctacagatatgcacctgttcttcactctgggaatgtgaacttgttctcctacttctcagattggctgagggatttttttgaaaatgaatgtctcatttcttgataactttggtttcattgaaaatgctattttgtttctaattgaaattgggtaaaaacaattgaagcaagtaaaaatctttatttcattagcagaaatgaagcatatattttcactgtagggtatttagatagaacttttcatacacactcaggtactgaccaacaccaaatcaggcttttgaggatttgatatttacttggaaaaaaaccctgttccaggtcaattacaggcaaagagctgcaaccatatataaaattctgtatataaattctctatataaaattctgtctacttccctttagttcttaatataaaattcctagaaaaatagaaagacatgatgacccaatataatggcccccaggaaactagcatgacattggagctgaggtaatgggcacttgccccattatcatgtctgcgaccacatccttcccaatgtggaagagcctcgtccagccctctgccccagctaggcctcagcctcagcttgcagcacttcctgtgttcctcagatgatgcctctgtgatcacaggaaaccagaaagggagtctgatgactatcaatttcaccccacaaatgccagtacctatacccccaagtgtctgatttgacatcatttcctattgacttaggttcctatttagagactatgtttgttgaaactgcatgattatttcagagagaaagcaaggtccattatatcatttcttagaaacttctagtcatggtgaattgctcagggtgaagatgccagcaaggaacaagatggaattcatatccactcagttcccactggctgccagaaaatgggatagatgttctacatattcagaatttcaggtgattgtcataagaacctggtaaataaacttattcatgaaagaaataactgatgtttagacaggggcagttatctgtccaaacaaatagttcatgctctttcaagtgcactattgggccactttgaataccctttgggtttattaacttaatggaaatagggccaggggcagtggctcaggcttataattccagcgctttcagaggctgaggcaggcagatcatttgtcctcaggaattcaagaccagcctgggcaacatggtgaaactccatctctacaaaaacacaaaaattaaccaggtgtggtggagcttgcctgtagtctcagctattccggaagctgaggtgggaggatcacttgagcccaggaggcagaggttgcagagagacaagattgcagcactgcactccagcctgggatacagagcaagactctgtctcaaaaacaaacaaacaaaactttataggaatgaactgtggcatttgtgggtaattatgcgctggcccggacttactgcctagtcctgcagagctaggtcaagacagaatgggcagtgactcaagacagaatgggcagtgactcaagaagccatggctaaagggtcatgctgaacacacatttggaagagttcccaccccccaccccacccccaccctgctccccaccggcattctgccttaggacccttcttctcactggaggggaaaaggctaagaaaacagaaaaccctctctgttcttgtgaacttgctttagcagataatatcatgggtgggatacctggagagggatcaaaacctcacagcccagacttaagtaaatgatcaaaatgtgtaatgaggatcatgttttggaaatgtggccaacatatttttattctctaaaataaatcatgtcaccttttgtcctttctttattgtagctaatccatgatatttactacccatagaaagagatggtagttgcccagaacaaactcacttttttttttttttttttttttttttgagatgaagtgttactctgtcgcccaggctagagtgcagcgcacaggcgcccgccaccacgcctggctaatttttttttgtttgtttgtttttagcagagacggggtttcaccgtgttagccaggatggtctcaatctcctgacctcgtgatacgcccgcctcagcctcctaaagtgctgggattacaggcgtaagccaccacagcctgccacaaactcactttttgaattaattgtgagatgttgggcttgaaaatcaggttcaatttttttttaaagagttttctatagttgtgattctctcattcataggtcaaaaggccacactggcaaagtaacaacacagaattttattacagctgctagatatgaagactcagcatatgatatcggtgacgttaataccttcccagggagaagcgctgttccttctggctgggaagtgcgagccggtggggggagagagaggagtagagcattatgtggaggtacttcccggttcccttgcgtctgagggtcttatgccagaggggatagaaagcccaacagaaactcaagatagaagaaggagaatctgcgagtgtctgtctcctgtcaagcttccctaatacagccctggtagaacttcatcaacagtggaaggcatttgcaaaggtgagcccaaaccagcacccctttccacacaggctgtccatgtagaaggcccagatgcttctcagggtctctgagaggatacaaagctactgagggggccagagggcacagcacctgggatttggatgagaagctgcaggaagggaactttgcaccccaagggcatggtgtggagtcaatagtggcaagttcagtctggttttttacatcagccggttcagaggaagagtgaaatccccaagatcagcagggcaaaatgctggaagttgtcgaggatgcagagagtagcaggaagacacctctgagaactcactcacacaccctgcccctgtgtagagatgtcatcctggggatgagaaggaggaagacagagaaacgcagaaaagcctaagcaggcaccacaaagagaccgagcccgtctgaaagaggctgctctaacctggtggaaactattttaagttggtaagtttagtgcctccccacaatatcagaacgagcaagagacgacaggtataggttgtgtacatttcccctctgcgttgaatgatagcgtgtgcgtgttccaccactgtgccctgctcaaagttagctgggtggctgtgccctgctcaaagtcacttgggtgaggggcgcccgtgggagccaaaaatcccatcttacacccaccccctgcacactctggagttgggctgtgacatgctggagaaaggtgtctttgtctaattattctgcctaagggcatgccttttgttaattagtaaaaggaagccttatttgtgctctgcagagtgggggtgctgtttaggaggtaattcgtgatagaaccacacagacaagatagattcaatttaaataaattgaatctatgaagcttcctaaccccatggaaacacaaaattagtttacacaaaaataatcattaaagaactaatgaaaataatgtttgaattcagccaccagacattacattccagagccttgagaaaaactgatgaaaaaaaagtcatgaaaaaaagtcattcgcacaagtgacaccatggtgtgaagtcaaggagcacagactctggagtcagagggcttgagtcaacctgagcatcttcagctttgactgtgaagacacagctttgactctctgtgttgcagagatggtagtgcccactccagtgacgcttgtgaggattagttgagataataaatacaaaatgctgagcatcaaacctagagtagagaaaggtctcaagtaagtactcattaccagtatttgttatttaatttcacttttgtctacattcccttgtgtgaaatggtttggataattaattaaggaaaactttccctcagggacattgctgatattgcaatcttcactagatacacttatctctacctccgcctccacctccaccttcacctccatctcttctctgtctctatctctatcttcctgttgtttatctatctaattatttataaatgaactggtgggtttgttgttgttgcagcctggctaatgttatccagacatatctgaaacctcatgagtggcatggaatggcagtccctgcttgaaccatttacctcctttcctaacaccaacaatcacacacacctgacactgacctgaagcctctggcctgtcctcggaggcaaagactgggtagacaagatgcctggttaccagcaatcttctgcaatttcctctgagctattgagattgcttttctctttgctcaaattatgtgagaaacttttaaaaaagaatttaatgtgctcttttgatatttcaggtgttcattcaaaagcctatgttattctctgtctctctgtctcttttcctagttgggtaatcaaaatggcacaatcagaaatatttatatctgcaacagaaaagaagaataaatttattcatgcacaagtacattatgtacatatatatgtttgtgtatacatatatctgtataattgatatatttgggagaaataaaaggtttcattaagcacacaagttctagagttagaccctctgtcgcaaattactgtcctgtcacttaactcctgccagaacaaagtgcatacttgaacaaaatgcctgctctgtaaaaatgccttgatcttgaataaaatgcctgctaggtcaaagcttctattttcccacctagaaaatgggaacaataataagaatcctcacttaatagataatggaaaaagttgcttgcagcacagagcctgctacagacaatgccttcaattaatgcaaactattaatattatgaaaagtgagtatctgttttctgacaatgttttcaataatataaattctgcctttgttcactttatttgtttgaaaaaacaaataaaaaaccaaacaaaaaagtgtcttaaaagtgtccatttgtctttcttcttgactcctagtaacgctttcctgtgtttagggaattttcacctcatgggttttggtgagtgaatgaattcatctccctctacagaaaagaagaatgcctgatgcattttctcagcctttattccaggtagtcaggtagactatggactccagcaattagatacactcctcacaacccctccattacacacacacacacacacacacacacacacacacacacacacacacacggctgctggagttgcagggtctggaaggaactgtctggcagggatggagtgtgcagggtgcctagtgagttccagcgtggccgtggctgccctggctgtggcagcaccagggctctaagccgggccctgcagactggctcaatctgcagcatgggcgctctctcttacttcccattcccaggacacatcctgtgcaggggaagagtgagtccttctagttgtagccacaggcccattggtctgctgacctccacctcctcaatattcgactccccagcattgagtgtctcaaaaacagtatttttcagaaaagagggtgaacagggcaactgctttaggaggagccatccgagccagctgcttcctctcctgtctcctagggaggacccaagctgtcggagttcatacctgtcccacaaaacacgagccagagctggacaaaagtgacagggacaaccactgtccaaggttaagtgagccctgaggcaccagaagatctccaagaaagccacatggaaatcataaaatggagctgaatggaggaaaagagaagttctgtaatgtggaaaaatgaagtactaacaatatttgactgttttcccttgatttagccaggttactacttcaaaacagtcagcaaagcattttaacaatgaaagctgttggggaaattaaatggctggaagtggagggaaactgtgcattgtggtgcatgcctgttgtcctagctactcaagaggctgaggcaggagggtggcttgagcccaggaattcaaggctgcagtgagccatgatcacaccactgcactccagcctggccaacatagcaagaccctatctctacaaaaataaaaataagaagtggaggggagataaaaatgtagtggtaggagtagtagtaataatatctaataattactgaaaatttactatatgtcaggaactatactaggtgtacttagctatttagtctgcataaaattttaataccagtgttattattgtatccattttcagatgagagatttgaggcacaaagagattaagaagtttgcacagggtcagacagcccctatgtgataaagatgaacagttagacattaaaacatgttttggttgggtgcagtggctcacgcctgtaatcccagcactttgggaagctgaggtgggtggactgcttgagctcagaagtcggaggccagcctgggcaacatggtgaaaccccgtctctacaaaaaatacaaaattagccaggcatggtggtgtgcacctgtattcccagttactcaagaggctggggatgaaaggattgcttgagcctcagaggttgaggctgcagtgagccatgagtgtgccactgcactccagggtgggtgacagaacaagatcttgtctcaaaaaatatatgtaaagaaaaaattctccaatgacatgggaagttgctcagaatataagctgaactgaaagaatacagaacactatacatgtaaatatatctatagtccataaaatcatattaatattcatgtatccaaaatgaaaatatctacaagtgagcatatgataatgtgaatagtagtgggcctttgtgatatgaccgtagatgtttttattgttatctttccccattgctctgagtttcttcaatgagcactgttaccagcatgttctacctatcagctgtgtgacttctgtggagttgatgactctgtgcctcattccctcatccaaaaaatgaaaattccaagtacccatattaagtgatcattgtgaagattagaaggtgaaaaacgtttagaaaaaaaaaaggctagcaaatagaaaatgctcaataagtatttgctattataaaagttaatgtttattaaatatgcaacaatttaaaatattatgctgaggaaaagtgttcacgaacaactcctaggcaattagaaatccttctcatttccacagaaattaagcaacccccatggccccctcacattcgtgcagagaacaccatcgagattgctagcctgatttgagataagcagggtgagcaggaggggggctcagtgctgagcctgcaggaggcactgaagggcccaaaaaaccattttctttctctccccagttcaggccacaccctccagaacctgaccagagtcgtctagccaccaggtccgcactttcctgccttctccttgggtacaccgccccgaagacaggatgtcactgctggaagcatttgccttctcctcctgggctcctgagttgctgtccgaacatttcagtctagctgcgtgaccaaaatcattcttcaatgtttccctcttctactgtcagatgttcattggaaattctcctcttttacttacagttggacttggattatcaaaagtggagcagttccagctatccatttccacggaagtcaagaaaagtattgacataccttgcaagatatcgagcacaaggtttgaaacagatgtcattcactggtaccggcagaaaccaaatcaggctttggagcacctgatctatattgtctcaacaaaatccgcagctcgacgcagcatgggtaagacaagcaacaaagtggaggcaagaaagaattctcaaactctcacttcaatccttaccatcaagtccgtagagaaagaagacatggccgtttactactgtgctgcgtgggattacaccatactagaactgttgaaacaacatgcacaaaatcccctcccagggtctgtgcccaccacatccttcccaacaggggcaaccacagccagtccccagctgggctcccagactcaggctcgccttctctgaggctcttccggggctttccaggaagctgttatgggttataccttcgttcccacctgatcccaggacttgtgctccagaatctttatttgacactgtttcttaatgcattaaagacttgtctggggactgagagaacataggtcgtgccactgtccatcatatcaccacctagagacttccagtaagtagcaaggtgcagttgagacagggatccttattacgtacagtcaagacaacccccctgcaatataactatcactggcccagtttacaatgaaagaaatgaaagcttagagaactgaggttgcatgatctgccagacaagtcatgtctttgagctggtctatgagaccacaccgaacagtttaaggattgcaattctctaagtaaatgctaggatatctgggataaattcgggaaggagtaagtgcccttttttctgggaggggtagggaggagaatttgcctgcatgagatcgtcagaatagagctccaagtcatcccaggggccattggatgagacccttcatgttggaataacctttggtcttacctgtaaaggaagagagaattgtatcgtgtgtgtgtgtgtgtgtgtgtgtgtgtgtgtgtaagttctctacagtgttctcaattctttgcatatattagctcctttaacccacactacctatagtgtctgctctgttgttctcatcaaacatatctaactcctgaaataagtggagtattagttcatgcacttgtccaaatcacagagctgataggtggcaggacagcctagggagggacccaggtaatctggttcctcttgaatatgacactaaactgcttctgaatcacaggagtataaaagaaaagacacattgttcctgtccccatggaggagacagaactgaccatcatggaacagtaactgacacacattactaccgtgtgctgaaacttgtgcccagggttccagtgattaggtgtattcagagaacaagtaaaatgccaataaagtaccaaatgacttttctttctttttttttttttttgagactgagtctcgctctgtcgcccaggctggagtgcagtggcgccatctccactcactgcaagctccgcctcccgggttgaccccattctcctgcctcagcctcccgagtagctgggactactggcgcccgccaccacgcccagctaattttttgtatttttagtagagacggggtttcactgtgttagccaggattgtctcgatctcttgacttcgtgatccgccagccttggcctcccaaagtgctgggattacaggcgtgagccactgcacccggccaccgattgacttttcaatataaaaacataagaaatttgggttttccatatctaggtacgtgacaggtactgttatctatacttcatgttcattatcattattatgtgatcatgtaaatttcttaagtctctggaagccatttaggcacttatagatgtagaactgagacctaaagatttcaaataactcagctgatgttagatagggtaagtagtctagaagggtgcatattgtcataggtcattaatagtaatattcagatgagcttttgaaggacctgatatatttttaaatataaaattaaaagatcagaatataaaactgtaaatgtaaaacccattaaaaaacgtttaatcatggctgggtgcagtggttcacgcctgaaatcccagcactttgggaggccagggtgggcggatcacgaggtaaggagtttgaaaccagcctggccaatatagtaaaacacgtttctactaaaaatacaaaaattagccgggtgtggtggtgcacgcctgtggtcccagctactcaggaggctgaggcaggagaattgcttgaatccgggaagtggaggttgctgtgagccgagatcgtgccactgtactccagtctgggtgacagagcaagactctgtctaaaagaaaaaaaaaatttaatcctgtgatcctgtgtaatgatccaaacaaatatattactatctacaaatgtgtagagaacatgcttaaaagtaaattctgattgctcttattttctttattttaattaactaattaatgttctactagagtcttctcaaaatattttcatcattttgcaacatttggtcaggttttcttcagtgaggattgggtagttatccaagctcccatgtttaccaactttgtgatctgggacgtcatgcgtgccacactgttcttgtctatcagagagagataataataccactgcctctcaacgctggtgagaagtgtgaaggaagtaatggaagaaaacgtttagaacaatgttagcaagtctacaatagatgtttgatataacgttaattttaaaggcttatgattacacataaaaatgaactttatttaaaaacacccctctctgtgacatagtgttcatgagatagttctgaagtccaaggtgagttcccacagactgccctgtcggtccctccagcaatttcaatcaagtttcctcttgaggtgcaccctctttataagtgaaattggatttctctgagttataatctgcattgtgacatcccaattaattataaaccaaatactttactgtatttcaaacagaaatgactatagctttttaaatgaggtatgaataatgctagtgtaaaatttcagtttgccttttttaaaattgtaaaatactgtccatgttttatactcctgagtcctgcatccccaaaacattaacagagggatcaatttttacgtgaggtaaagaaagttatatgcttatatatctggaaaaatattgtacagtctgaaaatcaaggagagaacagctaagtttgaagcagaattagttcaactccagagctgctcccatccctttccacagacacattcttgtcaggtaatgcaccctacaccccgtcagtggtcagtgtaatgctcctgggaactgctcagctcttcagtaggccatgaagtccccagagggcacctgacccaccacatttttctctctcaccaagtcatgccatgctgtctccccactgactggggccagccagcaaccagggtccttctcctggggatatggctcagcagacagcaggatgtccctgctgagaatattcatatttttctccctctgcagcggtgagttgctcctcaattatttcaacatagatgagagatgaaagtgattctttttttcttttattttaagacagtctcgttctttcacccaggctggagtgcagtggtgtgatctcagctcacttcaacctctgcctcctgggttcaagcaattctctcttgtgcttcagcctccaaagtagctaagattacaggcatgcgccactgtgcctagcttatttttttatttttagtagaggcagggttttgccatgttggtcaggctggtctcgatctcctggcctcatgtgatctgccctccttggcctcccaaagtactgtgattacagtcatgagccaccacacctggccagatgaaagtgtttcattatcatttcctctttctatgtcccaggttcatggggatttctcttttttgtttgcagttgaacttggtaagttaaatttaaagcaataaaaaatgtcaactacatttttgtcaacagagcaacagataaaagtgtctaggtatcttgtgtggtgtccactgaagactttgtaaatatagttatacactggtaccagcagaaactgaatctaaattatgagccatctgacaaatatcacttcaataacaagccccagttcgagtttgcttaggtgagaaaaacaagaaacttgaggcaagaacaaattttcaaatgtctacttcagtctttaccataaacttcataggaaaggaagatgaggccatttactactgcactgcttaggacccacagcatcagtgccacactgtcccacacaacaacctctgttgggtctctgcccaaccacatccttcccatgggagcaaactctatggactcctagctgggctcccaccctcagccttgccttctctgcggcacttctggatctttctgggaagccatcttgggttaatgctttaagcaggaagcatgcctgatcatgacgttcccagatattcattgaacactacttcctaatgaattaaggtttggcctgggaatgagtggacacaggctaaggtcccattcctgtcagcatccagataattctattaactgcaaacggcttaggccaagggagagaatcgttgtgtataggaatcccatatataattatttcaacacctctgcaacagaactattatttgcccattttaataaagaaattaaagcttacaagttcaaaatgactggtcgaagttgagaagtgcatgttttttgttttttaaaactggatcatgaggccaccttgaatatctaaaagtcacagttgtacaacagactctttgaggtgactttggggtggagcaagtgtcttttttctgtagagaagaagatggttcctcacttcacactaaggggtgtgacagtgtgatatcatcagaaaagagccccaggcatcggactgttaaatgagccatactttgcatttattaactcctttaacctctggcaacctctgaggtctgttctgttatgaacagaagtgcattttactcaggtaagtgagatctatttgtcctagccactcatccaggtcacacagctggttcatggcagtgtaggattggacccagctagtctggctccagagtctgtactcctcagtcacagaagggtaaagagaagtacattgttcctactcccatggagaagacaatactgacaacttctgtaaaacatttactggcacaattattattttgaactgaatcaggtgaccagaatttgagcaattaggaatccttgttgaataagtgaaataccaataaattatccattttttcaaaatataaagtgatacaaattcgattattttatgatgccatctctaaaataattgagaaagaaatgaagaatacctttaatccatgtacttttcctatagcagtacatactaggcacccccatggaaaaatatagataccaccttgcattcgtgccacgtgttgtcttacttattcgataatttccaaggtcaggacaacatattcatcctcatcatccccttttccaaggagccaggaaggctactgaaggaaataaagggggttccaggaaaggctgacctggggctggaatcagacaatccgtcatcctttatcctcccaccccgatgcactcagccttttgtgatccacatcctgtctgtgtaattcctgaccatcatattccctcagggtgggccacacttggtttcttgaacctatatgggcctttacttgttaactttaatattagctaaagtagacagtaagatctgaggaaaaacacagcgaatctgagaggataagctgttttcagacagggatgcatagacaggcttgcggaaatacttgtgtcaccctcttctcgtggttgtctcatctactactcaaaacagcctcagagagcagcaatgaggtatccactgccagatccctgtgtccagatcatagagcagagctctcctgcagcctttcaggcatcagactaaatggtgagaaacagagaaagagatactagattcatagtgcattcaaatgacagaatactatgcagcctgtgaaaatgatattgtatgcatttattaataaaattcaaacatcttcacaatacaatgtaaagaaaagttcttgaagtgtacaaaacctcttaaaaatataaatgtctgtgttgatagaataattttttaaaaacagaaagaaattatccaaaattttagaataattattcccgagggaataattatttaaattattctatgtacttttactaatttttatatattttcttaagtgagatactaaggctttgttgtaagatatacttaacaaagtaattttctcttgtttggtagtaatactaagacacgataacgtcattaaggactcatgctgtgccaggtactgatatctgagtattttatgcattaccattgtgtaacacgataatataagccccttagtacctctagaagatatatatgtaggcaaggtacacatgtagaaactgaggcccaagagcttaaataactcagcccacattctatagggttaagtggtataggagtgtttaattgtattcggtcactaaaaataatgtgcacatagactcaagacctgcagtattgctcatgataataaagtaaccaaaataagagagtataaagccaaatatgtaaatcccaccgaaatatatacatatatcatatgtataaataataccaagccattctatttcttttttaaaaatttttaacttttaagttctgaggtacatgtgcaggatgtgcatgtttgttacataggtaaacgtgtgctgtgtggtttgttgcacctatcaacccatcacctaggtactgagcccagcatgcattagctatttttcctaatgctatccttccccacaccctgcccgccaataggccccagtgtgtgttgtttctctccctgtgtccatgtgttctcatcattaagctcccacttataaatgcggacatgcagtgtttggctttctgttcctgcattagtttgctgaggataatggctttcagctcatccgttttcctgtgaaggacatgatctccttccattttatggctgcatagtactccatggtatatatgtaccataatttctttatccaatctatcattgatgggcatttgggttaataccatgtctttgctaccgtgaatagtgctgcaatgaacaataccaagctattctatttccaaccataaatatgttgagaaaaattcaaaggaaaagtaaatgatgggtgccttttgttgtcaatttttatatctcattttactcagattttccttaacggatgactgctactcacctgagttcttatgtttaccagctctgtgtttttgaatgagtcactcaaactctgtttgccgttgtcctcatttgacacatggagataatcataaaacttactgcacaggactgttgagaggatcaagtaaaataatataagaaaacatctagacaagtagcaagttgtaaatggatattagatgcttgtcaagtttcttactgcagttctgaattaacagctaattacagaaagatagtcattgggacagaacactgcaggtttatcttcacattttcaaagccatatttctgcaatatggtactgctggggaatgggagagtgggcaagagaacatccctgccccacccctagaggtacacattcatactaggtatttctttccagatagttaacccacttacccgatctgcccagcactcatgggatgcaggaaaccctggaactgctcataactgtagcagctcatgaagaaccctaaggaaccacctcatctagtacttctgagagacctcaacagccccgccttctgccactgacttgagacctccagtgaacagggttaccttctccctggggaaccagactggcagaaagcatgccactggtagtagctgttatcttcttctccctctgggtttgtgagttgccccctaatcatttcagtctacagaagagattgaagtcattctgtattattacctcttcacgtatcgttggcttatgggaatttctcttcacttgcaattgcacttgggcagttggaacaacctgaaatatctatttccagaccagcaaataagagtgcccacatatcttggaaggcatccatccaaggctttagcagtaaaatcatacactggtactggcagaaaccaaacaaaggcttagaatatttattacatgtcttcttgacaatctctgctcaagattgctcaggtgggaagactaagaaacttgaggtaagtaaaaatgctcacacttccacttccactttgaaaataaagttcttagagaaagaagatgaggtggtgtaccactgtgcctgctggattaggcaccacagtgttagagttgtcaagataacctacacagaaactatctccgagtctgtgcctgtccacatccttctccatgtgggcaaccacagcggtttgctcagctgggtgcccagccggagcctgccctccctgcagctcttctggaatgttgcaggaagacatcttagattctgctcccttggtgtgcagaatcacattggtgattcatggtgtccaaacgggaaaagttttcttgttccctctcagggcgtgcgataaggatgtggctcccttcttggtgcccctctcctcaaacctctagggggagcatgcacacgtgcaggttgtggggctccgaccccacagcagtgtctaggggtgaatgcttataactcctgaggccccagtgggcctgtgttacaaggtgtccttttagtttggctgtccataggtgacttgctttagccagctcaattagaccccctgccttattgcaaggacggagggctttctgtatccctgggtttcttgccttggtgtactgaaagaattggataacatgtgggcttggagaatgagtgcaagttttttatttttgtttttgttttgagacggagtctcgctttgtcgcctgggctggagtgcagtggcgcaatctcggctcacgcaagctccgcctcccgggttcacgccattctcctgggcagtctcccgagtagctgggactacaggcgccccccaccatgcctggctaattttttgtatttttagtagagacggggtttcaccgtgttagccaggattgtctcgaactcctgacctcgtgatctgcccacctcggcctcccaaagtgctgggattacaggtgtgagccaccgcgcctggccgagtgcaaggttttattgagtggaagtagctcttagcagatgggggagccagacgggagatggagtgggaaggtggttttcccctggagttgactgctcagcggccaggctttcctccaaccaccccgccaaactctgctttgttctgccagtcgatggcctgcagcccgccagtctcgccaaactctgctttgttctgccagtcgatggcctgcagcccgccagtctctgtaggtgtgcttttccacattagtgttcctctcgatgtccagccacttgtgtgtgtgcccactagggtctcaggggttttataggcacaagatggaggcgtggcgggccagggtggtcttgggaaatgcaacatttgggcgtggaggcaggagtgcctgtcctcacctaggtccgtgggcacaggcctgggagtggggccctcgacagggaccacgtccttcctttccctgcacttccctcccccaatcccatatcagtgtcagcaattaggatccaaattagggacattttgacactatttcctacaacattaggatatctgggaactctgaaaatacagagtgggtggcttagagcaaaattcatctgtctagtaattcgctacgtagagatttctagtaactggttcagaatgaaagtaggaagcagtatatattttacatagatattccctgctgttatcattattttcccatttggttcatgagcattggaggttttcaaagttagagtgatctgtcaaacatagtaactgtgtgctttttattcgcacctgaggccatcctgaagaaatctagggacaagtaagtagatctgtaagtaaacaatcacctgtttggggtatatgagagatgaaagtataaatcctgtgtcctagaggaagagcatgcagctcacttcacactcagggctcagtgctgggacaaaacaagcactgtgcagtggaacccagctcctaggcacagtgggggatctcaggatgggggctatgctttggagatcttgtctttcagggttctgcaaagaaaactaaaaatcctgagtaaaataggattagatagttaagaagaaagataatacatgcttcctgcatcggtaaaggaaataaccataataatacccctcagaaattaataaataagaaataatgattgacaattattttatgtttattccatgattaatcattgggtggttgggaactttcaaaaaataatgaaacaaaatataaaactgtaaaactgtaaaagtcctctctcacttctttgaaactttcaaacaacaaattaatgatgaaaaatccggagtttcaaagattttctcctatttatacctttagtactatggatatctgacagcatattgccatacatgcagtctacttacagtccttgaagtaattgcaacgtattttttctccattctcccttctgagaatcagcttgtaccatcctgataggataagaggagaaatgctattgaaagcccaatgagggaataccaggagcctccatggcaggtcagcccctttccaggtgcagactcagaatctggagtcccgcatcctgtccgccatgattcctgaccatggtggtccacagggagaatgacctgagcgcctgagtgagtcctcaacagacctcacctctcacctgatgcatacataaaagcaaagggaagaagattgttaaggaaatacagagcctgagaacatgaacttttcaagaaataggtgaatgaaaagatggaattcagcttttcacaatgtcagtgttaagtattttacatggattattttatttaatcctcaaaagagcagtgtagagtgactgtagtggccacacaaggtcaggtcttagaagatgcagtcactttgactttttaagagactcctgggagatttatggggaagaaaacttagagacacactagagtgaggaagaggaaggaaagagacaccgtatctgtgtgaatttaaagtaatgaaatactatgtagcaattaagcagtgtttttgaagaactataagtaaaattgaaaatattcaccatgtatttagcaggaggatattgaacacagaactgatttaaatagtaagctctcatgtacatacatgtatatattgaagaacgagcaaaaggaaaaaaattctccaaagtttaaagagtgggtgtctctgaaaggatgggtgattttaacatcttcttggtacttgcacagattttacacattgtaacaaaaagctgctactacttttaaagatgtatgccataatggcttcaatattttattgattcatgcatttaataatgaaactgtttatataacaacataaaatataactatatatggcacacttaaaattatttttatgtttttccacttaatcatatcactactctatagctctcagaaaaaaaaaaacaaaaataccaaccttcatgttaatactggttactattgagcagaaggtcagcaaactatgtctatgaccagcagtctccagttttgtaaataaagttttattgaaatacaaccatgcctatttatttatatattgtttatggctgcttttgctagctgcttttgcacttgaatggtagagtacattcagtcagtcttcactatctgtgcattaaatacctgcgaattcaaccaacagtggatcaaaaatatttgaaaaaaataaaaaattacaatacagcaataaaaataatacaaataaaaacaatataatatagcaactacatacatagtatttacattgtattaggtattatacataattagagatgatttgaagtgtagaggaggatgtgcatttgttatatgcaggtactatgccattttatatcagggacttgagcatacatggattttggtatctgtcggggatcctggaacaaatcccctgaagattctgagagatgactgtagctataacagagacccacaaagcccaaaatatttattatttgggtctttacagaaaatgattttcagtcactgtcctagagtgatagactcatgagtgacatttattcatatttagtgtttcccaatttctcaatttttctttaatgaccctttgttacacatccaccctccccatattagctgtgtgacttcagataaattagttagcatatatttgattcattttcctaattgtaaaatggagaacataataatgattactcaaataaactgttgagaaaagtaacttaaataatacaaataaagttcttgcaagtgcttggggcatgcctaatgctcaacaaattgaagcactacattaatcatatgagttattattgcatattagaaaataaaattatttagactaatactctaagtccttggtactcaaagtttgatttgtgaaccagcagcattggcttcacttaggagcttcttttaaatccagtcagtcaagcctcagcccaggcctactgcgtcagaagctcttttcagaaggtccctcctacatactatggtgtggggagtgggagtctaagggccaaactgttcaagatataagctccacagtctggtacaagtgcaagccaatcccatttccataggatggttgtgtctagtgtcctctctaatttctggagagcaatattgaactgatatttggcctctctggggctgaaatagatggcatcctcccaattaattaaacaaatatactcaattgtccacgtatatgtacttttattttcatttataaaatttgttataaaatcagcacaaattttcagtattttatatagtgagaaatacaggtgttttataaccttgagttttagatccacattcaacccacaggaagagtaatttttgctttgagtacaaaatacatatcactgtatcctcatatccacatatcacatatcctcatatcactagggctactgaaaaacgaaataggaggcaacagggaaggggagagaaattgaagttaattgccactgtcaccactcacccacacctcacccttcataggaagagttctcctctaaccatcaccatattgccagatctcctgggcactggagtatttagagggccagccatttcagatctgacaacgctgcactctacagaaagggttgtcagggaatcactgtgacccactacttctttccctgacacctgctcagaccaagctacccttgccacacactaaacattctaggcacaggcatcctcactttcctgcttcttcttgggaacacagcctggcagaccagagcatgtcagcaccaggagcatgtagggattcaccttggggtttgctccagtcatttcactttgtatatcaggtgaagaaattctttatcacttcatctttacatatcaggtgttcatgagaattaattttctttgcttacagttattctcagggcgttaaagttggcacaaatttaaaatacccagggcaaaagataaggatgcttttataccttgtaaaatatccagccaagactaaaaatgaagtcaaatactggtgtcagctgaaacctaagtcggcattggatgtgtgttgacaatcgcacctgctcagggtccattaggtgttgtggcttacaatgatgctcatccttccacttcaaccttgaaagtaaatttcacaaacatgaagatgaggtcatttactgctgtgattattgagcccactgggcatcaagcacacacttccctgccttctccttgggacacagcaggatgtcgttgctggaagcatcatcttttcctctctctggactcttacgggttccccatcattttgactcttgaggagagagcaagtaaattatttaatggtgcatctttatacctcaggtcttcatatggatttctcttctttgcttacagcttgttttggatacaagaaattggagcaacctgaaatattaatttccagagaaaaatattaaaagtccaaatactatctggggtggtatctagccgcttatactggctgagacataacttgatgcattttcctcaacaacatgaccctctcaattcacttaggggctgtagctgaaaatgatgttcctagatctgttttgacctacaagataaattctcaggaaaaaggaaatggagatagttatgtgcttgctggaatcacagatgagagatgtcaggacacccgcacagaatccctctttaggtctgtgtgtaccagcccccttccaacaggagcataggcttagcagggttgtcagggttggactgcacctcccaggacttccccttcaacctctggaaacttgattatgttcacacattaggacatacagaaatcagtgtactctgtgctcaaggtccagggattacctgaaagtttatatgatccagactcaaagagggaatcactgagtggcaggaaacgtgctgggtatcttacacatcttatataaccattgcaatactttcgcaatgtcatcttcatttttttccactttaatatgaaataatttgaaagataaaataccttcttaaaccccaaatgcccatgtttcctcagctgtgtcctgtgaccttgaagaagttagcattcatttgctccactcatgttgggggtgagtgtgaaatgaagctcctgccctctcctcaggctcattccactctgagggatcctcctacagtccagccagcacacttcctttgcacaggtctcagatcctcctagggaagggagggggcattagatgatccaccgacaaggtggatccccaccaggatggatcctcttcccggcttctgcctgtgattgcagcagccgtttattcagggtactctgctccctcttgggcactgctctaaatcctttacatgtaactcatctcatccttgggacatcttttcacattggtctgttgtgattctcatcttacgggggaggaaacagaggcagagcgatgtgatttactttgtggtcagagttcttaactggggggggggaggggctggggttctggcttcagcgtctgtcctcgtaaccacgctgtgtcctgactctgagagaggaggtaaaaatagcatctaatatgtggtctctacggctagaaagaaaactgataggaaattaaactagacattttagtgaaattataaaggctgaatgcagactagtgggagagtgtgagccgctgggggccaaaattttagggaatttcccaccatcttttagactttttctccaggaaccctatgcaggctcttgcagggaagagcatggagaatccagagaaagctcccctttttggtactggcttagaaggggaacagtagccactgtctaaattcacccagacctaccccacctcttctccactgtagaaggacttaatctgcaagagaaggtttctatggaatttcattttagttgagggagggaaaaggaagccaccatcaactctgcccaatactttatccctatctccacagagtaatgagttttaatgtgcagaagggtgggtgtcaaaatcatagcccaaggacactggtgggtgcctcctatgactggaaatgtgccacctctggaataagagcagcaacagttgtgaagttacattctcaagtcccggtttgaccctgcctgtttaagacagaagctgaatgaaaatagcagagaatggctcccttcctcacctcaccaccatactaccttgagcaaaagcaacagtagaatgcagtgaagagagcttcaaaagacagactgtctctggggagcagaacaaagggatggctcaaagccaagaacaagggatgattagagaaatctaaagtctctaatgtcctatgaagaacaaactccaatccagacaacttagtagcaacaacaaacttctaacccagtctaactcctaactagattaacacaaactcccacactaaaggtctggcagaaagaaagatgcaggcattttttttttcttttttcttttttctttttttttttttttttgaggcggagtcttgctctgtcacccaggctagagtgcagtggctgatctcagctcactgcaacctctacctcccgggttcgagtgatttacctgcctcagcctcccgagtagctgggactataggcatgcgtcaccatgcctggctaatctttctatttttagtagagacggggtttttaccatattggccaggatggtctcaatctcttgacctcgtgatctgcccaccttggcctcccaaagtgctgggattacaggcatgaaccagcgtgcctggccaatgtaggcatttttaagcatcaaatatagttatctcagtatctactgtgttatacaacatcgtcccctttcaataaaaaaatctaagtaccttaccccaaaacaagaaggaacacagtcttgaagccacaaagcaatcatacgcatcggactctgatatgactcagatgtttgagctgtcaggcagggagtttaaaataactgatgagtatgttaaaggctctaatggaaaaggtagacaacatgcaaggtcagacagagaatttcagcaaagagacagcaattacataaaaaaattcaaatgaaaatgcaagacataaaaaaaaaacacagtaacagaaatcaagaatgcctttgaagggctcaccagtagaccctatggagataaggaaagatttggttaacataaagataggccactagatatgacccaaactgcaatgcaaggagatgagaaagaaagaacaggagagaaagcatatcttcatggaagaacagaactgtggacaatatcatattttcaaacatatttgtaactagaatccctgaaacaaaagagacaaagagcagaacaaatatttgaaaaaataatggctgagagtattccaaatgtagtgatagataccaaaccacagaacaaaaaagctaggaaaacaccaaccaggataaatattaaaaacagaacaaaatacctagacatattagatttaaactgttgaaaaccaaaaataaagagaaactcttgaaggtagctagagggaaaaaagcagattttccatctgaaaccacgcaagcaagaagacattggagtgaaatctacaaagtgttaaatgaaaaaactgtcacttggcataaagacagcttcagacaaaataaaaactgagagaattcattgccagcagttgcacttcacaagaaatgtctgaagttattcaggcaaaaaaaaaaaaaatgatatgggtcaaaaacttgaattcacacaaggaaatgataagaactggaaataaaataaatgaaggtaaaacatagtcctttaaaccttaattgctctaaaacaggagttggcaaactatttttgcaaaggacccaatagtaaatatattctacgttggtggacaacatagtctctgttgtaactacacaaatgggctattgcaacacaaaagtccttgctactcttaagtctggagggacatggaactgttataacaaccgggagggtatctgtattgaaagggacacagccaaccggtcttagtttgagttcccccaggaagtgagcctcaggctttgaggacagctagtttgtttgggagacacaggaagactagtaggagagtgaggagatgatgttaagaaaaggaaggcagataattaaattactttcattaattagatactaaatgagcaacaggaacctcatagaagttcaaaacctaacagatcaattaaatcataatttcttgtttttctgttcctttaattcgtgggactggccatgtaaaataaataaaatctgcagacccctatgtgatctgatggttagtgtggtagtgaaccagggaatcttgctaagtgtcagaacgtgataagaaagtaaccacagagcagaaaaatattcctggtgttaccttaagttataaagacagagcttaaaatcgagcacacatattatatctatgtgaagcaaatgaaaaagatgagcagatattagcctgtaagggaatacaccaaactgttaatagtagttgtctctggttggtggggacaaaaagtgactgttttctctgcatttctttctgacccatctacccatgttgtcttcccatagctatttactgccctttgtttctacagcttcctaactgttctgaaatcccttactaatcagagcagtttccctggtatgcccatcacacatatgggcatgtgggacatagagattagctttttttctgactagattagtaaattcttataatagaaggacctgctgaaccaaggctggaatttcctactcttcactctgaaagctggaaccaatcccaaggggctggccacacacttggttcaaattgggtagtcctggcctgctttctgccttcttagagtgacctaggacttgttcatgtccaaggccttaccagccacacctagaaaatagcaagaacaatagtagcaaccatatctataccattacatttagctcagtacctctctttttggatgtctgacaagtagccaaaaaaattattgattccaattccactcccttcccccaatctccaagcatgtattattttcctccccagactttcctattgcagtaaatggcaacagtatattgtatcatctgatggaatggcaagggtgttttctcaagcagatagtgttttgttgacttctgtgttttttgtttctcctagtaatgagagaagagtgcagagacccaactattactgagtttcctgtgatatgagatctgaagggagtttacaggagctcttgaagctatggtttcacctgcgagaaagacacccacaaaccaggcccaaccctgtgtggtccaatctgagactggagtaggctgtctcaacagagcccctgaccgaaacactacagacccaatgcagggaagacccagtcttctctctaacttactgcaggtttagaaactctttgtgttccccctgacatgtgcagggcaataggccagccatgacggcaatgattgtcattctgaagtgcatggcccaaatggccccatggatgtataatctcctggtgtcactgaaagacaaataaaaagaaagtaaattgtgagatataatttgatattcagattcaactagccccgctcctcacagattattttgctaggtgttgtcactgactactcaatgctttttagaatatgcaaatcaaccatttcatctgctttttatttcgtttaatatgttctgtgattcctagaaagcaatacccagcatcctctatatggccatttgagatacagattctctatattatacagacctagactatacttgggaactgcgttccttccacacatatctctccaactgtgaagtaattgatgaacagggtttgggatctggaaaacttgaactgaaatcctggctcagtttgaactccctaattctgtttcctcacatgacttttaatggtaataaccatttatagggtaaagcagaaagagataaatgcatagttagtgcctgactcatggtagacactatatttatgagttttcttctctttcactatcagaaagcacaggcccatggattgtcatcctgcagcagggggaaggtaagtgaaaaggagatttggggcttagagtagcatatcaatttctcaagacatttttccagacacgagtcttttatgcaaacatttcttgtttgccaaaaagaaacaagtgtttcaccaggcatgtttgcctgtgggagcagtatcagttgaaaagtatctataaatctacaatatgcatagtggcatgttaagtaccccaagtgcaaaagaaaccctaaaagactaaatcttcaggttaagaatgaagacaggtggcacaattgctaaaagggagaatctgattgaaagtgcagtgacccggcctctcccaaacactgccctggtgtttttagaaacaagtgaagatccactggactatattgtaacatatctgatattatctaagtgatgacatatgtgaaatcaaattatgctaatttatgaaagttagtggtccacagattgtcagtatgtgatttttttatctcttgtacatgtcagataatgtgtttttttttgcttcagagggtggtctctctcagaagtgtcttaacttactgctgtacctgatttaattaagatccactacaatttctgaaagataaaccaatgtgaaaaaaatgtgcaaattattattttggttcatgttggcaaccaaaccctgaaatgaaatgtgagatatattttcgtatcttttgatggtctaacaaatttggttgaagctgttctctatgaaaattattatcatcagacttgaaaaagtgatgcaaaacttcaagcaatgcagtatcaacttgtgctttacctcacttgacttacttgttatttatatatttgttcattcataacccatcttcttggaagcaggatttaagttgcctcagtttgttaactcaagacatgacaaatgtggcggggaggatgtatgtgttccaaaacacagggttagaggcgaaactgcttatctttatacacattcatttgggtttcattttacgcctttagtaaaactgaacatcatggtcttcacatagttctttttttttgtaaacttaataaaatatgttataattcattacttactttttacattgtattacttaaatctttcatggctgttgaaatgtagacagcttctaagacttctgatacttccccacatggttctggaataaggaaaagcagaggacaaagagggattgaatgggcatcatcccatctatgacaggtgcaaagggtaattgacagtacgaagtaacaataacttattattttcagataaaaagacacagaaataagatctttccattctaccttatgaagtgaagtctctctgtctgaattattacataaatgataagagaaaattaaacagtttttagcccctactgtgtcccatgctcgattataaatatcgtacaaaagtcctgggaaataggtctaattctctccatttaaaagatgaggaaacccaggctctgagaagtgtgtgtgcccaagggcacatcaccaggagtggaagaactggaatctgaacctgggttttccaattttaaagtgtctttttcttcattcccaacttcctgagataataatttatttcataagaatcctttaaaagctcgagtaaacttgttaatgtttattgctgcagccactctgtccatctccaccatcactgcaacaattcaggtcctggttgcctcttattggattatggcgaccacctataaaaccatctgcttcagccaaattgctgtcctggggagcgccccttcctttctgcttgcacatctatctttctccagtgcaaatgtgatcatgtcactttcctctctaaattttttagcaagtcctcattgtctattctttcaaaaacatttatttgaaaatactataaaaatagaaaattttccacatgcttacttcctaaaaattaatgtgttaagtttctcctaccccatttccatcccatgcccctttactcaatggatacaataaatctccaatatgttccttctggccacgtgttgctttgtaattttaattttaatctatttggaccctgtgttatctgggatgaggtagagtggtatttttattttctaaggtaattattttcctaatgcccgtttccaaacaatccatcatttcctttcaatttaaaaatgctgcagcgtgttttaaatatgcacacatatttgacacattttctggagaatttctgttttatttgtctgtttcattattcttacatcattatcatattatctcagtagctttgtgataaaaattaagatctactatgccaaatgtctattcactgtaccatttttcagaaaatctttttcaatcatctcatatttattcactcctgtagaatttaaaatcaacttatctagcccaacattaaacctcacagcctagaacaacaacaacatgtcgtagtaattctgactggaattgctggaaatttatagatgaatttaggatgtattggcctctttatgataggagctttttattcatcaatgtatgtttctccatttatttaggttttattttatgcccttaggaaaactaaacactgtgttcttcatatcattcttgtatttttttggtaaatttaataaaagattttataattcattacttttccacattttattagttaaatccttcatggctcttgaaatattgacagctgctaagacttctgatgcttcgcctcatggtcctgaaataaggaaggccagaggacaagaagagattgagcgggcgtcattccatctatcacaggtgtaaagggtcattgacagcgccacataataattttgaattttctattaagaagaaaccctttccaaacataattttcacccagccccattgtcctctccattgaattgggggctgtgagctgctgtgtatggacaggtaccctctgtgacctcattcatatcttcctgaatgaggactcaggggacttaggctggagcagggtggatctggagtggacatggaggttgtcaaggcttgtcctcctcagcccttgcaagtgaacacctcatctgtactcaggagatcacacagctgaccccggcttaagatggcagatttttcaacatattagataactggatttgttttttttggtcatgcctcagtataattaaagaatgtattatttcatgggagatagaattctacaaatttcttctattattccaggagaaataataagtcattgcagaacacattttttcatttggcattgccttggtaaagcatcatgttgccaaatgataaaagtggctttttgaaagtggagaccgttgttcaaatttctcaagtatatctgcattgacacatttgcattttcagttactaaagagcttcctcctttcagaagtatcttcccaaattgctagcagagaggctctggtgtttgtgggaacagaagggcttttcctttgatgtaatctcaaagcagtttcaacacaattgaacccctggaaaaaaaaaagacaattctctgaatacttttcctggtaatttagaaaagcagtgggttgacccattaaacctgctgttttctcttcctgcttttttttttccatttcccttttctgttggtgcttttcaagaattactgccttagaagaaaacaggcaatttatgaggaaaaattacaaactatcacatgtcacaaaacctatattcaaggacttccaaaaaagccagaagatgaaattgctagttcaaagttgttggattgctagtcgtgtcccgaggatcagaaggctgagatttttgtagaagcttagaccggtgtgataccactggttggttcaagatatttgctgaagggactaagctcatagtaacttcacctggtaagtaacttttctttctgtttttattccagtaatgaaaaactgatagatgatttttagaaaaaaatgatcaaccttatctgaatatgtcacattcctggcctcagtatacgaacagcaattttgcagattagctgaatatggaaacaaaacgattttgtacatgatatcttcccttccctgtctgtaagcggattaaaattctactttaagaatacacacacacacacacacacacacacacacacaaaagatagactctggcaagaaattaaaatgttttgaggcccatgtctatacaccattagtgtaagtccttggtccaagttacttttttgttggtcttttaagtgagagacataaaaatggagttttattaattacttcttctctgtattttgagatataacatagtgctcccttcttctgctagcctgccaaacccatgttattgattttgatctcatcctgagaaatagtatagaaaaaaattacttcttatagtaaattactatagaaggtcaatacatcccacttattagtgttctagtttctttgagggaggctgaagtcagtcaaaatttatgcaattgggactcttgttatatcacctggaaatggcccggtttaatagaatttgtaagttcaaccagccatgtcagctccaaggtcaatgaaaagagtcttcatcattttacatcttcatttgttcattcatcctctcagcaaatatttatcaaaaacagtttttgttctggatgctagagataaaagggcaaagaagacacagtctcaacactcaaaagctgccagtctggcagataagtattctagattctggcttggttgggccctgtccacgttctttggcctgtggctgccggagaagcagaaggtcttgggttcatgagctcattttctttcttaatttgtgtagcagttattgcttataagatctatgtattgcgtttggtgggaggatttgataaaatgacccaatattgtccttttaaggagaaaattaatattagcaaagtttattgagagccagacaccatgctaaatagtttcaatgctttatctccttcctcatcagacctatgcaggagatcctcttagtcccatttcacagatgaggaaactgaggcctagagaagctcagttactttcttaaagtcacatgactagtcactgtggaaaagtctgggatctatctaagcttgtctactccaaagtgcctggtctggacccttatgtgatatttagaaatattaagtcatatttttatactttgaatatttcttcttctgtagcttgaccctatgaatggactctttagttgactatttttctagtaacaactcccaatttgtattactatttgtgtattaatacaattcttctacttctaattatggcactgaaatgacctctctcctccaaaaagtcatatgggatatacatttattaaatactcaaaatataatttttagggtatttctgtagaatgagtcattttgacgtcattccactcagctgtctttctgtattggcatcaaatttgctagatatgttgaaactgatgtaggagctatcgcagctatgctatattgcagtgctaagtcgcataactcagagctgcctcagattctctgttgagtagcacacgatttaatttgatgaaactgtatagatattttcaagtcaaaagtagcagtctttcagcaatgaatcatcattaagaattcatattttctaacaactcatcagtattctatcagtgagaactggattctaaaaagaacttactttatttttattttttattttttgagatggagtctcactctgtcgcccagctggaatgcagtggcatcatctctgctcactgcaacctccgcttcccagtttcaagagattcttctgcttcggcctcctgagtagctaggattacaggctcctgccactacgcccaactaatgttttgggttttttttgtatttttagtagagatggggtttcaccatgttgaccaggctggttttcaactcctgagctcaagtgatccgcttgcctcagcctcccaaagtgctaggattacagggatgagccactgtgcctggccaaaaagaagttattttagaatcaatctagatacccatccctccatacatatgaatcccaaaatacctataaatcatattgaatatctatttattaaatgtcaaacataggaatcctattattgtctctctttgaaaattaaggaaatattaactctaaattacacttaagacaaagtgtatacaagaaaactttttagggaagatttagaagattcaggcaaaatcatgagaaaaggtaaaatcagactctctaatgtatgggatacaaggagagaatgtacatagcccaaagtgcccagggcaaggtgaggtcagttcttaaattcctgattacattcagatccagtgtgattttgtttgacctttgtcttgacttaacgtcagcagggccaatttttatgtatttatgtaaatattgaaaaaaatgttggcacaattttaagacaaacacaaagggagattcttataaaggcttctcaggtggtgggcaagagttgggcaaaaaaatcaaggtatttggtcccggaacaaagcttatcattacaggtaagttttctttaaattttgcaatgtaaagaagggatgggaggctggcaggcaggagctggctcagaattctaggattccctccttggtcactaatcatggtgaaatctccagagaggtcaggtgacttggttcatgccttaggagtcagaacttttcctgccctagcatgggagacattactaaggagcttagaccaactgcaaatctctaaaggatggaggccttatgttgttccattggtatctctctgttgaaagttttgtgaacaagtttagttttgagattttatttcttcagttctaaaaataaccaatggaaaaaattaaaaaaaaaaaaagtaaaatcagctaccctccttatttggtcaccaaaagatgaaatatttgataatttgaccaaagaatggttaatatcaaatgttaaaatatttctcggtgtgaccatatttagaagtaacataagctgcatttattgttatttaaattggtccaatgagtttgtttattatttgttagcttaagtttaaagatgtaattttgcctggatgagagaaaacatctcataaagatactcttagtctgttagatccactgaaatgaaagttttcagagaattttcacaaagttgataaagcatcggaaaaaatgaaagcagttttacatttttaattccttagtggttgagatcttatgataaaatgaacttataagttaaaaagtgaccttccgattctcttttatccaattgacttaatgagaattgtagcaatcaaattcataatttgtaattttctgagaagtgatttttcaggaaagtgcggtgcaagaaaaggtatggactttgtttctcgactcctggagctagcactttctatgtaactcccttttaggaagtgtattttgatttaccagttgttcaaattataaaaatgctggttcattatagaaaaattggaaaacacaaaaataaacaaaaaattataatttgatattgaccctcatcacattatcattttgttatatttttatttaaacatttttctctgctttttgtttgtttgttttacaaagttggaatcatactagatacacaataatagatctggctttttcacttcacactgcttcataaacattcttttcaaatgtccttaatatttttcaataccagaacaaagttgaaacttctgttttcacgttgatctgtacaaagaagataatggagattatttatctaaagtggatgttataaagattaaatgaaattaaatatggaaattacctaccagaatgcctggcacttggtaggtgatagaaatattatttcctcttctagaattcaagttactacccacgaaaggtctttatacactcaggaatacagataaatgtatcgactcccatctattcagcagctcacttcagaacaaatatcactatttgtaaaatgctttctatgtctaaaagactaattgtacctgcttctaaaagtaattagaatgttttacgtattatctcaaatatgatctacctgaatacaaggtgatttttcattttcaagagaaaatttatgtttaagaaaatatgtattttcccctcccccaactcgaatatgtaaatttatagggctacaggtaaaacagtcaaatgtctacctataacatttaatttcttacctggttcatactttcaaagttaaaaattatatcaatatcaatatcagttgagaaatattgccttttttgcccttatatttcattaaaacttttgttttgatgcttcacatgcatgtaaagcatctatctcagaacagctttctaaggcatctcaggtcaaagcgtccactttggaatcctcttatgatggtgtctctgaatattttattctaagacacaattattcactcacaaaataaaaggatatatttttttccaatttattctgttattctacagttgtatgaagtaaaaactacagagacattaccccaagtaataatgaccaaatccgtgataaatttctttgcctttttttttccttttaccagtgctattccccaaactagcatcattgagttcatttcatgtcgatatctcctccagttagtccttctggatcaaagcagagtattagaagaacattttttaatatgagaagttacacaaagactgtaccatacataaggcacctccccatgttgtgagagaaaattttggggaaaaaaagcttcattttaagttctggcactttctatctaaatttagtatgtaggtgtccctatcacagagctaggatttgcaaacatagtctccattccttgtgtcttatttgagcttgaccttacaaaaccatcaactcctgggggcaaaggagaaacatgctaaatgcacaaactctttgttatttatttaagctatctctttccaaaatctatttgagaagacctaaattaaaatatacaagcacagtcagaccattaaatatatacagatgatctaaagccctaaggaaaggagaaggaaaaaggcctgtgattacctagtgaggagcacagtttaaaattttatgctcaaaagaaggagaaaaaggtaggggaatacatacatcttactaattgataaaaagaagcacaccaaattttcaaatatcatatttttttctattactagattggaaaaagacttcaatgcatgagtcctttagaaggaaatggaagagtgggcagtgccttcaacttccattttggaaaatgaaaggaatggtcatgaaaaacccactgcatattaccactgcatcagtgctatgggcatcctgacatttaatgaaatgcgcagatggtgatgctcagcagacatggtcaggcagataacatgtagtgatctaaagtgacaacagagagatggatttgaggaccaggcctcttgccttttctctacccattctgccttgaagggtaaagccaggtgtttcaagctggactttggcatgaactagacagaagtcagtttcaggctgaagtttctggtgaaacttggaaggcaaataagttgtgctgctgattagaaaaaggctcacttgttttgaaaaacacaagtgaagaattcccatacactgactgcatatattagactttagccaatgttccctttgactttcttaacacggtaggtaaggcaaaggataacctattaaagattgggcgtgtgaaagccatgtttcttgtgatgatggggacgatggctttgagaatcccagagcaaagtggaatgcaaacagaggaactgagaaattattcctcctgcttaattgctatggatttaactgccactccaaaatgctgaattttttttagtaagggcaatgcttggtcctatagggttaaaatgtcatgtcaaggcacacaatcatagcaaacagattgctaatcataacaatgacatcatcatcatcataatctcttatatttccatagcatttatttttgaggcagggtcttcccctgttgcccaggcaggagtgcagtggtgtgatcaattctcactgcagcctcgaactcctaggctcaagtgaccctcctgcctcagcttctcgagtagctgggcctacagtcgtgcacatcatgctcagctaatgctttttgtatttttagtgaatatggggtctcactgtgttgcccaggctggcctcaaaattctgagctcaagcaatcctcccacctcagcctcccaaagtgctggaattataggcacaaaccactgcactgggacctataacattttaatcaaattgcttttttatatcttgtttcattttggtctcacttcagtgctggtagcgatgttgaactgattttgaaacatcactgtttttagacaaataaaacaccaaaagctttaagttatttgatttgtggagcaacagaacttgttatgagcaaaatgaaccaggactggaaccctggtcttttgagaatcccagaccaccagaatttgaagaactcagggaaactgaattagagtttttgatatggactgaatcactgtggaattattataagaaactctttggcagtggaacaacacttgttgtcacaggtaagtatcggaagaatacaacatttccaaggtaatagagggaaagcaggaaattattaaactggaataatgtaataatgtttagaaaaaagaggaattggatggggatttgatgtagaaaacttaggagagactttaaaacaaacgctcatactaaaagagaacatagataacattgcacagatatcataataagatttggctttgtgcatatacggacttccataaagggctcatatgtaatgtatgaaatgatctcattaaaatgtctggccctgagaccaaatgtattatgacaggtaagtttgtgatagactctacagagtggacacatattcatctctgatggtcaaagacatgtttactcttgttgtgaaggagcccgggtgttggagtcaggtccacctggaactctggctccaccactcactgcttagtgaaattgagtgattattctctggcctcagttttctaatccataaaatgggataacagtatgaattcagcagggttgtataagaattgcacaacatagtgtgaattaagtacttggcacattgtccaacccaaaataggtgcccaacaaatgttttctggattcacatgtaaagagacaatgggatctactatggagagttgctctcagtccatctaatttacagagcagcaattctccagaggattcagctgtacttctaactgctcaaatggaaggttatcaacatcagctcacacacgcaaaaattgaacttatggattcgtttcttgttagcaggctttttaatcacgtggcaaaaacattgtattaagatgtctgttttttatttttgttgttctatgtgctttacttaatcctttatcttaattgatatcatttctaacaccaacatattggtcctaagatttatagccaattagtttagggttctgttcatatgtctcaggaaaaaaaggttaaaatcttaccaaaaatggtcaagatatcaaatcaattaaatccagttggaaacatcataaatctgaaatacatatttaaacataaaatggctataactatttagctaatgaaaaaataagaaatagagaacacttaaataaatatccatatgtagatttaatatatcataccgtctctaaaaactgtagttgatatttggtaaatttacaatgctgcattttaataaactacaaacaacttaggcaatttaactcaaatatactatttgattttgcaaataaatgtacataaatgaatccaacaataaaataaattttatttattattttaaataaaatatgtaaattctatttgttattgaagtaagtaaaaatgtaccatacttggccataaaaaactcttaatatgtacattttaaaagtagtattttaaaaatcatgtgagaggatgatccacaatatcggcccttaccatgtgtaatcaagtatgctatttaatgattcgttaactactacgttgagaaagttttggaagttccagattcattttgtcctgaaaagaatgaaacttaaagaatctagctaaagaaaggggacaagaggcaatgaatgctgtggtaccgtacagaaaatgtccaagtttatcatttgatttttaatttctttagtacaatgaattagaagtatttcaatgaagagacactagttcttaggatgaaaattagattggaaaatatattgactagagactacaattatataaatataatgtacaattgaaaaattactcatattttataacatgcttttaaaattagaagcaaactatatggtggagaaatatacactgtctcacaagtataacaagtaaaatactatttgcactaaaagcaaagagtatgaaattaagatgagcacattatgcctaattaaatttatagcatgctcacaaattaatatttctgtatatgtttactaattttgtatgaaaatcagaagctttgctacacagacagaaattatcaagactgttttcttttcttctgaaatgagaaatttaattcttattttcttagaaattgttcaattattaaattcacttcaaaccagccaaagcattggagtttcaattggaaatcaaaatagaaagaattgtaacatttataatttcagttattagattaaaaatacgtgtataacccattaacattccagattcaagtgatatgcctttgtaaacatatgatgctttgttatgtatcttgaccctatccctataagaagctctgaaatcatgacttttaatagagcaattatatgtacattttattcagcaggctaagatgaagagaataatggagctttaaaacagttaagcagcatataggacagatacaaattctgggagagacataaagagtcaaaatatagatacactgatttacacagaccttctcattaatggggtaaatttatataaaacccagtataaaaaatacacccctggtgcattcttagtcattcttaaacttcaaatgaaattccaaaataaaatgtgcttttggtgaatattttctgaagcaaaatgaaattttgataagtgcgttactgcagaagattaacacaagagtatttctgaaaataatcaagaaaaaatttaaataagagttttggaaagttgccattttgtttctaaattcaggagatggtgaataatctggaggtacagctgtaaatactgctgcatcccaaaacttggagggtgcagatgtgaaattgagatgttatataaagttagatattaactagggggactgctcatggtatacacattgaagctacatggtcaacttgatagacagtatgtacatgcggaagtagattctctttaaaacaagtgactgtgtatgttaaaaataaaagtgaacaaaatggctaggcatggtggctcacacctataatcccaggatttgggaggctgaggcaggcagatcacttgagcgcaggagttttaaaccagcctggtcaatatggtgaaacatgttcctagaaaaaaaatattagccaggcatggtgatgcatacctgtagtcccagctacttgggaggctgaggtgggaggatcacttgagcctgggaagtcgagactgcagtgagctatgatcttgccgctgcattccaacctggacgacagagcaagccccagtctcaacaacaacaaaaattttgacattgattcatatgggaaataagataaataataagataaatatggtgcatcgcagaatcagttaaatgaagagtgggagtacacgaaattgcagaacatgagaatgtgtcatatttggccaaagaacataagttacaaaggatggaaaagggaagtgggaaaaggaccaaagagtctcatctgtagagagatcattaaggttttctgaccttccactttcccctgccatccaccttgaaaacctgcttcactatgatgaaacaaaagagattaaaaaataaaataaatatgctcatgaactttggaagccctggtaggaggcagttaaaaatcacactcatcacagcatgtgcagaataaacaaaggccaggttttcgtccagcatctgacatttgagagctgtgacttttggcaagttatttaatgtcttgattctcttttcaacatctgtaaaataagcacaataataagtactgtgcagcctatcctggatgaaaggccgcagtggacaccagctcaatggcatcttctctttttatggttatgtactaggccactccaaactgtgcaatgtgtgtgtttctctaatgattcttttaaactcatatttcatttctccccatagataaacaacttgatgcagatgtttcccccaagcccactatttttcttccttcaattgctgaaacaaagctccagaaggctggaacatacctttgtcttcttgagaaatttttccctgatgttattaagatacattggcaagaaaagaagagcaacacgattctgggatcccaggaggggaacaccatgaagactaacgacacatacatgaaatttagctggttaacggtgccagaaaagtcactggacaaagaacacagatgtatcgtcagacatgagaataataaaaacggagttgatcaagaaattatctttcctccaataaagacaggtatgtgtttacgcatatcatctgtcagaacacttctttgaaagtgaatgctgcattttttcctttcagtattaatgaaaaacaaacataaatctttcttaaatattgttacatttaatggtagcataaatgccctgctacttttctatagaattaaaatggtataggttttggagaaaacaaaattgaaaaagttactgaaggtttgtcagcctcagctccattatccaaaataagaaagtcacgtgctggtttttagggttgttagatggattaaagaaacaacatacacagaagcatctagcaacgtgacacgtggtaaacgctcaaaaagtgttctcccttcttttgatgactttacttgatcaggaaataacatatatatgtctttcaggaatgttctgcccaagcaggagagtcactcacctcaatcttgctacccacaaagtttaacctaaaaacaacgggttcattgttgacaaaatgatgtttatctgttgttgacagaatgatgtttatctaaaaacagttccaattttctatttcctttgctgagacacaaaggggaggcaaatgtgcaaagcttgagggtagtcttaccactgtgcttaagtgttctgatttttctagtgatcagggcaaaataaaaagtatagtaagttccaaggcagtgaatattatacaggagagaagttacagttttataatgtgttttcctttacactaaattctaaaagtaaaaagtctttttttttttttgacagagtttcactcttgttgcccaagcaggtgtgctatggtatgatctcagctcactgcaacctccacctcccgggttcaagtgattctcttacttcagcctcccgacaggctgggattgcaggcgcctgccaccacacctggctaatttttgtgtttttagtagagatggggtttcaccatgttggccaggctggtctcaaattcctgacctcaagtgatccatccacctcggcctccaagtgctgggattatgggcgtcagccactgtgcccagcctaaaagtaaaatgtctttcatgagcttcccaaggcagctacgttaaggaggacacttctcttaatgtcattctacagtagatttctaatgctctttcttggaagtttgtttttctgagaaaagctaaaaatataacatggaagtgatcatattatataatcaatgaagtgcttttcaaggagataaaactaatctggtccacacttgcaaccaaccttgattgagagagagagagaactcaggatacacttgaagattttattatggggaacagttactttattctttttacctcaatcaatgcatggaaataagtgatagtcattttcatttatcttttaataaatgaagtcaccatgaggaaaataaaaagacattgaaaacccattaaagtcagcccttaaagatatttggacatgcagacttgataactaacgtttgcattcttgagacttacccaaaacccatacctcaagtccaagtttttagaattcatgaaataaagatctcagtgagtgcataaaattgcgcaccagaatcatatccgtatagacaagaacacatctactagaaaaataataaaccaacacaccaatgcaactgtgttttcttctgttttaaagtatgttgtctttgtatgcatgtttgcttcttcctttttttttttaacatcacagataaattcaactctcacctcaggttttattgagagaactgtcaatgtgacttggcctctgtctttctagtcccagaaagaattgcactgaaatctgagctcctgtaataaaaacaaccatttgctgagagtaattaacatactgaaagagattttcttagagtacacaatggtgacattatattgcctctttataaataactttctatctatttctgtggattattcctacaaagtacttttcatatgtccaatttcttttcttcccctacaactactgtctgaatactggctctgctatttgctgatatgattctcggcaagttgcctgcactttttaaactttatttcctcattcagaacatggggccatacataatacaactcacttcagtgttattggggaattaaacaaaaaatgcatgggaagcatttaacatagtgcctgacacaataatgagtactcagtagatgttagcttttattaatattgttgttgttatgtccagaaacactatacctccagaaaatcatgggtacttgctggggacattggggatatgcatgatttggaaaagaatgactgctttttttgcttagatgagaaatttttctaagccagactccttcaaatatgtaagattctgttgtggattcaaggactgaaagaattcttggccgagtgtggtggcttatccctgtaatcccagcattttgtgaggacaaggcaggaagattgcttgagtccaggagtttgaaaccagcctgcgcaacatggcgaaaccctgtctctacaaaaaatacaaacattagctcggagtgagtgctgacatgtgcctgtactcccagctactcagaaggctgagatgggaggatctcatgagcctggggagtttgaggcttcagtgagccgtgatgacaccgtactatactccactccagcctgggtgacagtgagaccctgcctcaaaaaacaaacaaacaaacaaacaaaacaaaattaatctttttgctgatgtcatgtcagcagtgtgtgttgaaggctgtaaagcagccatttgttcagtttatttttccattgaacaagtatttatcaaaaacatactttgtggcagtcactatgctaggagctatgaatacagaaggaaaagtaaatgctcttggatactacactccagttgtgataaaaaagaaaaaatgtattcttcaccaacttcaacatcttgatgtgcaaaaacataatacatgaattagatctacctaattacacagaattagaccaattgtttctggaattgtgggctcatatttttaataactgtcctcctgcctctctgtcgacaggttttataaatattcatttaattacacacacacacacgaacaattgactagtacttgctctcattcttctagatgtcatcacaatggatcccaaagacaattgttcaaaagatgcaaatggtaagcttttgtgtttttcccttcctcctgatcattttgttttgaacttctctggcttgaaaaatcagggaatggattttgctaggttggatgctgcagaatggacctagtgatattttaaattagtccctcattttctaggagttgtattaacaaacctaactactgctttggggtatgagatgactgtaaattagagagggtacagtggtatagtgatatgcttttaattatttcaaaaaaaagattttattcattcatgtgtcttttttctttttcttttcttttttttttttttttggacagagtcttgctctgtcacccaggctggagtgcggtggcagtatctcagctcaccacaacctccgcctcccggcttcaagtgattctcctgcctcagcttctcgagtagctgggactacaggcgcgtgccaccatgcccggctaatttttgtatttttagtagagttggggtttcaccatgttggccaggatggcctcgaatttgtgacctcgtgatctgccccctcgccctcccgaactgttgggattacaggcgtgagtcactgtgcccggcctcctgtcctgtcttttgtttaatgactgggaaaaacatgataccatgttgcttctcgagttgttttgttttagtctttggtctttgctagtagctaataacacgaactagtgtttatcaagtgctttttacacagaagggcttgggctgtgttctgcattttcttgtttaaccctcttaaaactcctataaaatggtacatatttttctcccaatttacagtccctttaaagcaaataattataaaaatccctatacatgtcacacagctagatctgggatttcaaatcaggccatcaaacaaagagtttatgtacttagtaagttttctgttctttttctacaatagagtcagatagcaagaaattaccaagccaggaacctgaaacaaaacggacatcatgtggggctgggtgggtgcatgggctttgcagactggactttcactccagctcttttaatgattaggtgtaagtgacctacattttgtgagcaacagttttctcatcagccaacaaagaataattacaccagattcacagttattgaagagataaaggcatgaatgtgagatgtctggcatagggcatctcatttagcagacacagaatgagtacttgtttctggctttttctctctacatatgcacaaagaatgcgactagaagcatgggctctagccctgctcaactttcctctatttccaataccaaggggctctgacttaggctgccacaccaggcaaggagggcagtaccacctcacttgaccaagggcagggagtcacggacacatcacttcttgagatccttttccacaccaaggactgatgtttctggaattctcactttatgaagacaaaacatataaatggaaattttctcaggtagagactcactcttgtagctcattgagtaggcactagtggtccacccccactgtctttacttattccttgacatcacatatctcttgcaaaacctcaaataatattaaatgcaatcacccaataatagcatagccataattagaggcatttaggaaagacaggtgagtgtgccacaactacctaacacatcagcaaatctggattaaccactttctttgattttccacaatgcaaccttactttttaatagttgggaatgttctaagtgaatttagcagaggttgttaatcaacttgaaagctgaattctgacttgtctgactcttggtggtgctggtagcagtagatgtttacttttaggttttggtggtggtggaatatcacttcaacgtaaatcatcagaaataagtatttgtgaacccctctcgcattaatgtatcttattctgtaaaaagaacatgtgcaatttctcttagatacactactgctgcagctcacaaacacctctgcatattacatgtacctcctcctgctcctcaagagtgtggtctattttgccatcatcacctgctgtctgcttagaagaacggctttctgctgcaatggagagaaatcataacagacggtggcacaaggaggccatcttttcctcatcggttattgtccctagaagcgtcttctgaggatctagttgggctttctttctgggtttgggccatttcagttctcatgtgtgtactattctatcattattgtataacggttttcaaaccagtgggcacacagagaacctcactctgtaataacaatgaggaatagccacggcgatctccagcaccaatctctccatgttttccacagctcctccagccaacccaaatagcgcctgctatagtgtagacatcctgcggcttctagccttgtccctctcttagtgttctttaatcagataactgcctggaagcctttcattttacacgccctgaagcagtcttctttgctagttgaattatgtggtgtgtttttccgtaataagcaaaataaatttaaaaaaatgaaaagttgacttttgtccatggtattttaattggatgacatcaaattgaacatccaaggtaagaaacagcatggcaattgggctgtggaattctgtattggttgtaagaatggtccaacaccccatttctaattctttccctgagatcgtggttatcacaccttctaagaagaactacaaccaaatgaaggagctcatgtgacttctgtttgaaaggtcaccagagtcagattcattcggtttaggacattccagtggctataggacactatctactgtgacgcgtaccgtgtgagctcagctctagagtgtttcacagacactgtgtttcctgatcctcacgatacccccatgagagctgccctaaaagcagagaggcagcgtgatggagaggttcagcacatgctctctgatcccaggaatcctgggtatggtgtttcgtatctgtgtgacctcaggtgagttccaggaactctatgtgccataatctcctcatgtaaaatgaagttataatgccccgtttcctggagttatgtggattagatgagttaatgacacctggcacatgcaagtcctccacagtgtcggcacgcactgttggtagctctactctagagacagtaataaaccaaaaagtatctgacacaggcctcaatcaacttagaagtttattttgcctatgttaagggcatgcccaacttcctgagataataatttatttcataagaatattttaaaaactcgagtaaacttgttaatgtttattgctgcagccactctgtccatctccaccatcactgcaacaacgcaggtccttgttgcctcttattggcttatggtgaccacctataaaaccatctgcttcacccaaattgctgtcctggggagtgccccttcctttctgcttgcacatttatcttcctcaagtgcaaatgtgatcatgtgactttcctccctaaatcttttagcaagtcctcattgtctattcttctttcaaaaacatttatttgaaaatactattaaaatagaaaattttccacattcttacttcttaaaaattaatgtgttttaagtttctcctactccatttccatcccatgcctctttactcaatggatgcaattattcttctacatgttccttctggccatgtgtagctttgtcattttaattttaatctatttggaccctgtgttatctgggatgaggtagagtgatatttttattttctcaggtaattatttgcctaatgcctgtttccaaataatccaccatttccttacaatttaaaaatgctccagcatgtttttaatagctacacatatttgacacattttctggagaatttctgttttatttgtctatttcattattcttgtatcattatcatattatctcagtagctttgtggcaagtattaagatctactatgccaaatgtctattcactgtaccatttttcagaaaattctttttcaatcatctcatatttattcactcctgtagaatttaaaatcaacttatctagcctaacattaaacctcacaccctagaacaacaacatgtcgtagtaattctgactaaaattgctggaaatttatagatgaatttagggtgtattggcctctttatgatagaagctttttattcatcaatgtatgtttctccatttatttaggttttattttatgcccttaggaaaactaaatactgtgttcttcatatcattcttgtatttttttggtaaatttaataaaagattttataattcattacttcttcacattttattagttaaatccttcatggctcttgaaatattgacagctgctaagacttctgatgcttcccctcatggtcctgaaataaggaaggccagaggacaaaaagagattgagtgggcgtcattccatctatcacaggtgtaaagggtcattgacagcgccacataataattttgaattttctattaagaagaaaccctttccaaacataattttcacccagccccattgtcttctccattgttgtgggggctgtggcctgccgtgtatggataggtgccctctgtgacctcactcataccttcctgaatgaagactcaggagacttaggctggagcagggtggatctggagtggacatggaggttgtcaaggcttgtcctcctcagtccttgcaactgaacacctcatctgtacacaggagatcacacagccgacaccagcttaagatggcagatttttcaacatatcagataactaaatttttttttttggttatgccatagtttaaataaagaatgtattacttcatgggacatagaattctacaaatttcttctgctattccaggaaaaatgataagtcattgtggaaaacatttcctcatttggcattgccttggtaaagcatcgtgttgccaaatgatacaagtggctttttgaaagtggagacctttgttcaaatttctcaagtatatctgtgttgacacatttgcattttcagttactaaagagcttcctcctttcagaagtatcttcccaaattactaacaggccctggtgtttgtgggaacagaagggcttttcctttgatgtaatctcaaagcagtttcaacacaattgaacccctggaaattaaaaaagaaaaaaaacgacaattctctgaatacttttcctggtaatttagaaaagtagtgcattgacccactgagcctgctcttttttctctctatcgcccaggctggagtgcaatggcacgatctcggctcactgcaacctctgcctccctggttcaagcaattctcctgcctcagcctcccgagtagctgtgactacaggcacacgccaccacgcccggataatatttttttgtatgttagtagagacggggtttcactgtgttgccaaagctggtcttgaactcctgagttcaggcaatccacctgactcagcctctgaaagtgctaggattacaggcgtgacccactgcgcccggcctttctttttttgttgttgttggttttttatcttaacatttcttttttctgttgatgcttttcaagaattactgccttagaagaaagcaggcaatttatgaggaaaaattacaaactatcacatgtcacaaaacctatattcaaggacttccaaaaaagccagaagatgaaattgctagttcaaagttgttggattgctagtcatgtcatgaggatcagaaggttgagatttttgtagaagcttagaccagtgtgatagtagtgattggatcaagacgtttgcaaaagggactaggctcatagtaacttcgcctggtaagtaattttttttctgtttttattccagtaatgaaaaactgatagatgttttttagaaaaaaatgatcaaccttacctgaatatgtcacattcctggcctcagtatacgaacagcaatttttcagggtagctgaatgcctggcacttggtaggtgatagaaatattatttcctcttccagaattcaagttactacccaagagaggtctttatacactcaggaatacagataaatgtatcaatccccatctattcaacagctcacttcagaagaaatgtcactattcataaaatgctttttatttctaaaagcctaattgtacctgcttctaaaagcaattagaatgttttacgtattatctcaaatatgatctgcctgaatacaaggtgatttttcattttccagagaaaatttatacaagtttaagaaaatatgtattttcccctcccccaacttgaatatgtaaatttatagggatacaagtaaaaaagtgaaatgtctaattataacattcaatttcttaactggatcatacctcaaagttaaagattatatcaataccaatatcagttgagaaatattgccttttttgcccttatatttcattaaaatttttgttttatgcttcacatgcatgtaaagcatctatctcagagcaactttctaaggcatctcaggtctcagtgtccattttggattcctcaaatgatgatgtccctgaatattttactctaagaaacaatgatccactcacaaaataaaaggaaattattttttccgatttattctgttattctacacttgtatgaagtaagtaagaactacagggactttagctccaagtaataatgaccaaatccatgataaatttctttgctttttttccttttaccagtgctatccccaaaactagcattcattgagttcatttcatgtcggtatctcctccagttagtccttctggatcaaagcagagtattagaagaacattttttaatatgagagtttacacaaagactgtaccatacataaggcacctccccatgttgtgagagaaaaattttggaaaaaaagcctcattttaggttctggcactttctatctaaatttagtatgtaggtgtccctatcacagagctaggatttgcaaacatattctccattccttgtgtcttatttgagcttgaccttacaaaaccatcaactcctggggacaaaagagaaacatgctaaatgcacaaactctttgttatttatttaagctatctgtttctaaaatctatttgagaagacctaaattaaaatacacaagcacagtcagaccattaaatatatacagatgatctaaagccctaaggaaaggagaaggaaaaaggcctgtgattacctagtgaggagcacagtttaaaattttatgctcaaaagaaggagaaaaaggtaggggaatacatacatcttactaattgataaaaagaagcacaccaaattttcaaatatcatattttttctattactaaattggaaaaagacttcaatgcatgagtcctttagaaggaaatggaagagtgggcagtgccttcaacttccattttggaaaatgaaaggaatggtcatgaaaaacccactgcatattaccactgcatcagtgctatgggcatcctgacatttaatgaaatgcgcagatggtgatgctcagcagacatggtcaggcagataacatgtagtgatctaaagtgacaacagagagatggatttgaggaccaggcctcttgccttttctctacccattctcccttgaagggtcaagccaggtgtttcgagcgggactttggcataaactagacagaagtcagtttgaggctgaagtttctggtgaaacttggaaggcaaataagttgtgctgctgattagaaaaaggctcacttgttttgaaaaacacaagtgaagaatttccatacactgacactgactgcatatattagactttagccaatattccctttgattttcttaacacggcaggtaaggcaaaggataacctattaaagattgggtgtgtggaaggcatgtttcttgtgatgatggggacgatggctttgagaatcccagagcaaagtggaatgcaaacagaggaactgagaaattattcttcctgcttaattgctatggatttaactgccactccaaaatgctgaattttttttagtaagggcaatgcttggtcctatagggttaaaatgtcatgtcaaggcacacaatcatagcaaacagattgccaatcataacaatgacaccatattcatcataatctcttatatttccacagcatttttttttgaggcagggtcttcccctgttgcccagtcgggagtgcagtggtgtgatcaaggctcactgcagcctcgaactcctaggctcaagtgaccctcctgcctcagcctctcgagtagctgggcgtacagtcgtgcacatcatgctcagctaatgctttttgtatttttagtaaatatggggtctcactagatactgggttgcccaggctggcttcaaaattctgagctcaagcaatcctcccacctcagcctcccaaagtgctgggattataggcacgagccactgcactgggacctataacattttaatcaaattgcttttttatatcttgtttcattttggtctcacttcagtgttggtagcgatgttgaactgattttgaaacatcactgtttttagacaaataaaacaccaaaagctttaagttatttgatttgtggagcaacagaacttgttatgagcaaaatgaaccaggactggaaccctggtcttttgagaatcccagaccaccagaatttgaagaactcagggaaactgaattagagtttttgatatggactgaatcactgtggaattattataagaaactctttggcagtggaacaacacttgttgtcacaggtaagtatcggaagaatacaacatttccaaggtaatagagggaaggcaggaaatgattaaactggaataatgtaataatgtttagaaaaaagaggaattggatggggatttgatgtagaaatcctaggagagactttaaaacaaatgctcatactaaaagagaacatagataacatggcacagatatcataataggatttggctttgtgcatatacggacttccataaagggctcatatgtaatgtatgaaatgatctcattaaaatgtctggccctgagaccaaatgtattatgacaggttagtttgtgatagactctataaagcggacacatgttcatctctgatggtcaaagagatgttgactcttgttgtgaaggagcccgggtgttggagtcaggtccacctggaactctggctccactactcactgcttagtgaaattgagtgattattctctggcctcagttttctaatccataaaatgggataacagtatgaattcagcagggttgtataagaattgcacaacatagtgtgaattaagtacttggcacattgtccaacccaaaataggtgcccaacaaatgttttctggattcacatgtaaagagacaatgggatctactatggagagttgctctcagtccatctaatttacagagcagcaattctccagaggattcagctgtacttctaactgctcaaatggaaggttatcttaacatcagctcacagacaaaaattgaacttatggattcgtttcttgttagcagactttttaatcacgtggcaaaaacattgtattaagatgtctgttttttatttttgttgttctatgtgctttacttaatcctttatcttaattgatatcatttctaacaccaacatattggtcctaagatttatagccaattagtttagggttctgttcatatgtctcaggaaaaaaaggttaaaatcttaccaaaaatagtcaagatatcaaatcaattaaatccagttggaaacatcataaatctgaaatacatatttaaacataaaatggctataactatttagctagtgaaaaaataagaaatagagaactcttaaataaatatccacatgtagatttaatatatcataccgtctataaaactgtagttgatacttggtaaatttacaacgctgcattttaataaactacaaacaacttaggcaatttaactcaaatatactatttgattatgcaaataaatgtatataaatgaatccaacaggtttatttaaataaataaaatatatatattctatttgttactgaagtaagtaaaaatgtaccatacttgaccataaaaaacactcttaatatgtacattttaaaagtagtattttaaaaatcatgtgagaggatgatccagaatatcggcccttaccatgtataatcgagtatgctatttaatgattcgttaactattaccttgagaaagttatggaagttccagattcattttgtcctgaaaagaatgaaacttaaagaatctagctaaagaaaggggcaagagacaatgaatgctgtggtaccgtacagaaaatgtccaagtttatcatttgatttttaatttctttagtacaatgaattagaagtatttcaatgaagagacactagttcttaggatgaaaattagattggaaaatacattgactagagactaaaattatataaatataatgtacaattgaaaaattactcatattttataacatgcttttaaaattagaagcaaactatatggtggagaaatatacactgtctcacaagtataacaagtaaaatactatttgcactaaaagcaaagagtatgaaattaagatgagcacattatgcctaattaaatttatagcatgctcacaaattaatatttctgtatatgtttactaattttgtatgaaaatcagaagctttgctacacagacagaaattatcaagattgttttcttttcttctgaaatgagaaatttaattcttattttcttaagaaattgttcaattattaaactcacttcaaaccagccaaagcattggagtttcaatgggaaatcaaaatagaaagaattgtaacatttataatttcagttattagattaaaaatacgtgtataacccattaacatcccagattcaagtgatatgcctttgtaaacatatgatgctttgttatgtatcttgaccctatccctataagaagctctgaaatcatgacttttaatagagcaattacatactcattttattcagcaggctaagacaaagagaataatggagatttaaaacagttaaatagcatattaggacagatacaaattctgggagagacataaagagtcaaaatatagatacactgatttacatagaccttctcattaatggggtaaatttatataaaaaccagtataaaaattacacccctggtgcattcttagtcattcttaaacttcaaatgaaattccaaaataaaatgtgcttttggtgaatattttctaaagcaaaatgaaattttgataagtgcattactggagaagattaacacaagagtatttctgaaaataatcaagaaaaaatttaaataagaattttggaaatgttgccattttgtttctaaagtcaagagatggtgaataatctggaggtacagctgtaagtactgctgcatcccaaaacttggagggtgcagatgtgaaattgagatgttatataaagttagatattaactagggggactgctcatggtatacacattgaagctacatggtcaacttgatagacagtatgtacatgcggaagtagattctctttaaaacaagtgactgtgtatgttaaaaataaaagtgaacaaaatggctaggcatggtggctcacacctataatcccaggatttgggaggctgaggcaggcagatcacttgagcgcaggagttttaaaccagcctggtcaatatggtgaaatatgtctctagaaaaaacaaatattagccaggcatggtgatgcatacctgtagtcccagctacttgggaggctgaggtgggaggatcacttgagcctgggaagtcgagactgcagtgagctatgatcttgccgctgcattccaacctggacgacagagcaagccccagtctcaacaacaacaacaaaaattttgacattgattcatatgggaaataagataaataacaagataaatatggtgcatcgcagaatcagttaaatgaagagtggaagtacacgaaattgcagaacatgagaatgtgtcatatttggccaaagaacataagttacaaaggatggaaaagggaagtgagaaaaggaccaaagagtctcatctgtagagagatcattaaggttttctgaccttccactttcccctgccatccaccttgaaaacctgcttcactgtgatgaaacaaaagagatttaaaaataaaataaatatgctcatgaactttggaagccctggtaggaggcagttaaaaatcacactcatcacagcatgtgcagaataaacaaaggccaggttttcgtccagcatctgacacttgagagctgtgacttttggcaagttatttaatgtcttgattctcttttcaacatctgtaaaataagcacaataataagtactgtgcagcctatcctggatgaaaggccgcggtggacaccagctcaatggcatcttctctttttatggttatgtactaggccactccaaaccgtgcaatgtgtgtgtttctctaatgattcttttaaactcatatttcatttctccccatagataaacaacttgatgcagatgtttcccccaagcccactatttttcttccttcgattgctgaaacaaaactccagaaggctggaacatacctttgtcttcttgagaaatttttcccagatattattaagatacattggcaagaaaagaagagcaacacgattctgggatcccaggaggggaacaccatgaagactaacgacacatacatgaaatttagctggttaacggtgccagaagagtcactggacaaagaacacagatgtatcgtcagacatgagaataataaaaacggaattgatcaagaaattatctttcctccaataaagacaggtatgtgtttacacatatcatctgtcagaacacttctttgaaagtgaatgctgcattttttcctttcagtattaatgaaaaacataaatctttcttaaaaattgttacatttaatggtagcgtaaatgccctgctacttttctatagaattaaaatggtataggttttggagaaaacaaaattgaaaaagttgctgaaggtttgtcagcctcagctccattatccaaaataagaaagtcacgtgctggtttttagggttgttagatggattaaagaaacaacatacacagaagcatctagcaacgtgacacgtggtaaacgctcaaaaagtgttctcccttcttttgatgactttacttgatcaggaaataacatatatatgtctttcaggaatgttctgcccaagcaggagagtcactcacctcaatcttgctacccacaaagtttaacctaaaaacaacgggttcattgttgacaaaataatgtttatctgaagataactgtagatcatatttatctgtagataatgtttatctgtggagtgtggctctacaaaacatagaatagtcttggtcactgcagttttatagaggccttgggtttttcagagtttcattttatatatcaccataaagtaacatttcataattacaggttggtaaggcttacatgtacaaacattcttccattttccataataaatgcatttcctgccattggtgaatgcagctcaataaacatttattgtacaattatgacacgccaggcttagtggaaatgtggatgaacagacaaggatgagttactgtcctaaggatgatgcatgacagtgcagagaatatactctcttcctgatcactcagggtcactcatgattcatgcgcgaggtcccaaaacagtgcctttgatgcagattctgtacatctctagacgattggtccaagggctgaatgtgctctggcccagtggtccagtctgtcactatatgtcaacatcctgaatatgaacataacagtccaacatctcaagagtgggcatgaaaaggactcattttgtgctttttcctgtggttaacaagtcctttttagcctgggggaacaagcattaacaaaatgtttgaagatctttgccacgtaccattccaaatttctagggtaagtctttagcttttcagatcctgagtttctgcaatgatcaaatgtgatttggacagttgcgttgactttctcctggggctataatggagtgcaaaggaaacaatggcagggaaaatgcttgctttcaaaatggtagcatggatgtgttcattcgtgtagttactgtattaggtatagcctttcctgaaactaactgaagtggggttataaaaacagtcccaattttctatttcctttgctgagacacaaagaggagacaaaagagcaaagcttgagggtagttttaccactgtgcttaagtgttctgatttttccagtgatcagggtgaaataaaaagcatagtaagttccagggcagtgaataccatacaggagacaagttacagttttataatgtgttttactttacactaaattctaaaagtaaaatgtctttttttttttccgagacagagtttcactcttgtagcccaggcaggagtgctatggtgtgatctcggctcacagcaacctccacctcccagtttcaagcgattcttctgcctcagcctcccgagaagttgaaattacaggtgcctggcaccatatctcgctaattattctatttttagtagagatcgggttttaccatgttggccaggctggtctcgaactcctgacttcaagtgatccacccgcctcagcctcccaaagtgctgggattacaggtgtgagtcactgtgccggacctaacagtaaaatgtctttcatgtgcttctcaaggcaactacattaaggaggacacatctcttaatgtcattctacagtagatttctaatgctctttcttggaagtttgtttttctgagaagagctaaaaatataataacatggaagtgatcatattatataatcaatgaagtgctttcaaaggagataaaactaacctggtctgcatttgcaaccagccttgattgagagagagagaactcaggatacacttagagattttattatggggaatagttactttattcattttacctcaatcaatgcatggaaataagtgacagtcattttcatttatcttttaataaataaagtcaccatgaggaaaatgaaaacccattaaagtcagtccttaaagatatttggacatgcagacatgataactaacatttccattcgtgagacttacccaaaacctatacctcaagtccatttcttagaatacatgaaataaagatctcagtgagtgtataaaactgcacaccagaatcatatccgtatagacaagaatacatctactagaaaaatataaaccaaaacaccaaggtgactctgtttttttctgttttaaaatatgttgtctttgtatgcatgtttgcttcttcctttttttttttaaacatcgcagataaattcaactctcacctcagttgagagagaactgtcaatgtgacttggcctctctctttctagtcccagaaagaattgcactgaaatgctgagctcctgtaataaaaatgaccatttgctgagagtaattaacatactgaaagagattttcttagaatagtgcacaatggcccaatggtgacattatattgtctctttataaattattttctatctatttctgtggattatttctacaaagcacttttcatatgtccaattccttttattcccctacaagtactgactgactactggctctgctgttcactgatatgactttcggcaagttgcctgcactttttaaacgttatttcctcattcagaacatggggccatacaaaatacaactcacttcagtgttattggggaattaaacaaataaatgcatgggaagcatttaacatagtgcctgacacaataatgagcactcagtagatgttagcttttattaatattgttgttgctatgtccagaaacactatacctccagaaaatcatgggtacttgctggggacgttggggatatgcatgattttgaaaggagtgactgctctttactgctcagatgagaaatttttctaagccagactccttcaaacatgtaagattctgttgtggattctaggactgaaagaattcttggccgagtgtggtggcttatcctggtaatctcatcatttgggaggacaaggcaggaagattgcttgagcccaggagttggaaacaagcctggacaacatggcgaaaccctgtctctacaaaaaatacaaacattagctggtcatgggagtgagtgcctgtactcccagctactcaggaggctaagataggaggatcacctgagcctgggcagtttgaggtttcagtgagccgtgatgacaccatactatactccactccagcctgggtgacagtgacatcctgcctcaaaaaaacccccaaaattattctttttgctgatttcatgtcagcagtgtgtgctgaaggctgtaaagtagccacttgttctgtttatttttccattgaacaagtatttatcaaaaacgtactttgtggaaggcactgtgctaggaactatgcatacagaaggaaaaccaaatgttcttggatactacactccagttgtgataaaaaagaaaaaagtattcttcacaaacttcaacattttgatgtgcaaaaacataatatatgaattagatctacctaactacacagaattagaccaattatttctgggattatgggctcatatttttaataactgtcctcctacctctctgttgacaggttttataaatattcatttaattacacacagtcacagacacactcagacacacacacatacacacacacacacaccttgacaaataatgggcatgaacaattgactggtacttgctctcattcttctagatgtcaccacagtggatcccaaatacaattattcaaaggatgcaaatggtaagtttttgtgttttttatttcctcctgatcattttaagttttgaacttctctggcttgaaaaatcagggaatggattttgctaggttggatgctgcagaatggacctaatcatattttaaattagtccctctttttctaggagttgtattaacaaacctaactactgcttcatgtaagagatgactgtaaattgaagggtacagtgatatgctttcagttatttcaaaaaacagactttactcatccatgtgtcttttttcttttcttttttttcttttttgagacggagtctcgctctgttgaacaggctggattgcagtgacgcgatctcacctcactacaacctccgcctctggagttcaagcgattctccagcctcagcttctcaagtagctgggactacaggcacatgccaccatgtccgggtcatctttgtatttttagcagagaccgggtttcactatgttggccaggctggtctagaattcctgacttcgtgatctgccccctcagccctccgaagtgctgggattacagacgtgagtcactgtgcccggcctaacagtaaaatgtctttcatgcgcttctcaaggcaactacgttaaggaggacacttctcttaatgtcattctacagtagatttctaatgctctttcttggaagtttgtttttctgagaaaagctaaaaatataacatggaagtgatcatattgtataatcaatgaagtgcttttcaaggagataaaactaatctggtccacgtttgcaaccaaccttgattgagagagagagagaactcaggatacacttggagattttattatggggaatagttactttattcttttttcctcaatcaattcatggaaataagtgatagtcatattcatttatcttttaataaatgaagtcaccatgaggaaaataaaaagacattgaaaacccattaaagttagcccttaaagatatttggacatgcagacttgataactaacgtttgcattcttgagacttacccaaaacccatacctcaagtccatgtttttagaattcatgaaataaagatctcagtgagtgcataaaattgcgcaccagaatcatatccgtatagacaagaacacatctactagaaaaataataaaccaacacaccaatgcaactgtgttttcttctgttttaaaatatgttgtctttgtatgcatgtttgcttcttccttttttttttttaacatcacagataaattcaactctcacctcaggttttattgagagaactgtcaatgtgacttggcctctgtctttctagtcccagaaagaatcgcactgaaatgctgagctcctgtaataaaaatgaccatttgctgagagtaattaacatactgaaagagattttcttagagtacacaatggtgacattatattgtctctttataaataactttctatctatttctgtggattattcctacaaagtacttttcatatgtccagtttcttttcttcccctacaactaccgtctgaatactggctctgctatttgctgatatgattctcggcaagttgcctgcactttttaaactttatttcctcattcagaacatggggccatgtaatactcatgtacgtgagtattacgtaataatgctcacttaagtgttactggggaattaaacaaaaaaatgcatggcaagcatttaacatagtgcctgacacaataatgagcactcagtagatgttagattttattaatattgttgttgttatgtccggaaacactatacctccagaaaatcatgggtacttgcttgggatgttggggatatgcatgatttggaaaggtatgactgcttttttctgcttagatgagaaatttttctaagccagactccttcaaatatgtaagattctgttgtggattctaggacggaaagaattcttggtcaggtgtggtttcttatccctgtaatcccagaattttgggaggacaaggcaggaagattgcttgagcccaggagtttgaaaccagcctgggcaacaagacgaaaccctgtctctacaaaagtacataaattagcttggcttggtggtgtgtgcctgtattaccagctattcgggagactgagatgggaggatctcctgaacctgtgaagtttgaggcttcagtgagccgtgatgacaccatactatactcgactccagcctgtgcgacagtgagactctgcgtcaaaaaaaaaaccccaaaattattgtttttgctgatttcaggtcagcagtgtgtgctgaagggtgtaaagtagccacttgatcagtttatttttccactgaacaagtatttatcaaaaacatactttgtggtctgtttttgataaataaaaaggcactgtgctaggagccatgaatacagaaggaaaaccaaatgttcttggatactacactccagttgtgataaaaaagaaaaatgtattcttcacgaacttcaacattttgatatgcaaaaacatagtatataaattagatctacctgattacgtagaatcagaccaattatttctggaattgagggctcatatttttaataactgtcctcctgcctctctgttgacaggttttataaatattcatttaattacacacacacacacacacaccttgacaaataatggacatgaacaattgactagtacttgctctcattcttctagatgtcatcacaatggatcccaaagacaattggtcaaaagatgcaaatggtaagcttttgtgtttttcctttcctcctgatcattttaagttttgaacttctctggcttgaaaaatcagggaatgggccgggtgcggtggctcacgcctgtaatcccagcactttgggaggccgaggcgggcggatcacgaggtcaggagatcgagaccatcccggctaaaacggtgaaaccccgtctctactaaaaatacaaaaaattagccgggcttagtggcgggcgcctgtagtcccagctacttgggaggctgaggcaggagaatggcgtgaacccgggaggcggagcttgcagtgagccgagattgcgccactgcactccactccagcctgggcgacagagcgagactccgtctcaaaaaaaaaaaaaaaaaaaaaaaaagaaaaatcagggaatggattttgctaggttggatgctgcagaatggacctagtgatattttaaattagtccctctttttctaggagttgtattaacaaacctaactactgcttcgggtatgagatgactgtaaattagagggtacagtgatatgctttcagttatttcaaaaaacagactttattcatccgtctgtcttttttttttttttttttttttttttttgagacggaggagtctcactctatcacccaggctggagtgcagtggcgcgatctcggctcaccataacctccgccttactggttcaagcgattctccagcctcagcttctcaagtagctgggactacaggtgcacaccaccatacctggctaatttttgtatttttaatagagatggggtttcaccacgctggccaggatggtcttgaattcttgacctcgtgatctgccccctcgggctcccaaacttctgggattataggcgtgagccactgtgcccggccttctgtcttttgttataatgactggggaaaacatgataccatgttgcttcttgagttgttttgttttagtctttggtctttgctagtagctaataacacgaactagtgtttatcaagtgctttttacacagaagggcttgttctgcattttctagtttaatcatcttaatactcctataaagtagtacaatatattttctcccattttacagtccctttaaagtaaataactataaaaatcccttatacatgtcacacagctaggtctggcatttcaaatcaggacatcaaacaaagaattcgtgcagttactaagtcctctattttttctacaatagaaaaaatagcaagaattacagatagcaagacattacaaggcaggaatctgaaacgaaagggacataatgtggggctgggtgggtgcatgagctttgcagactagactttcattccagctcttttaatgattaggtgtaagtgacctacattttgtgagtaacagttttctcatcagccaactaagaataattacaccagattcacagttattgaagagataagggcatgaatgtgagatgtctggcgtagggtatctcatttagcagacacagaatgaatacttgtttctggctttttctctctacatatgcacaaagaatgtgactagaagcattggctctagccctgctcaactttcctctatttccaataccaaggggctctgacttaggctgccacaccaggcaaggaggggcagtaccacctcacttgaccaagggcagggagtcacggacacatcacttcctgagatccttttccacaccaaggactgatgtttctggaattctcactttatgaagacaaaacatataaatggaaatttctgcaggaagagactcactcttgtagctcattgagtaggcactagtggtccacccccactgtctttacttattccttgacatcacatatctcttgtaaaacctcaaataatgttaaatgcaatcacccaataatagcatagccataattagaggcatttaggaaagacaggtgagtgtgccacaactacctaacacatcagcaaatctggattaaccactttctttgattttccacaatgcaaccttactttttaatagttgggaatgttctaagtgaatttagcagaggttgttaatcaacttgaaagctgaattctgacttgtctgactcttggtggtgctggtagcagtagatgtttacttttaggttttggtggtggtggaatatcacttcaacgtaaatcatcagaaataagtatttgtgaacccctctcgcattaatatatcttattctgtaaaaagaacatgtgcaatttctcttagatacactactgctgcagctcacaaacacctctgcatattacacgtacctcctcctgctcctcaagagtgtggtctattttgccatcatcacctgctgtctgcttagaagaacggctttctgctgcaatggagagaaatcataa

SEQ ID NO: 2 - DNA, 4249 bp, Homo sapiens
agtgcagcgcagaagacagagggtgactaggaagacgcgcgagcggggctggccggccggcgggtgggggaggggaggcgggggaaggcggctgagtgggcctctggagtgtgtgtgtctgtgtcagtgtgtgtgtgtgtgtgtgtatgtgtgtgtctggcgcctggccagggtgatttcccataaaccacatgccccccagtcctctcttaaaaggctgtgccgagggctggccagtgaggctcggcccggggaaagtgaaagtttgcctgggtcctctcggcgccagagccgctctccgcatcccaggacagcggtgcggccctcggccggggcgcccactccgcagcagccagcgagcgagcgagcgagcgagggcggccgacgcgcccggccgggacccagctgcccgtatgaccgcgccgggcgccgccgggcgctgccctcccacgacatggctgggctccctgctgttgttggtctgtctcctggcgagcaggagtatcaccgaggaggtgtcggagtactgtagccacatgattgggagtggacacctgcagtctctgcagcggctgattgacagtcagatggagacctcgtgccaaattacatttgagtttgtagaccaggaacagttgaaagatccagtgtgctaccttaagaaggcatttctcctggtacaagacataatggaggacaccatgcgcttcagagataacacccccaatgccatcgccattgtgcagctgcaggaactctctttgaggctgaagagctgcttcaccaaggattatgaagagcatgacaaggcctgcgtccgaactttctatgagacacctctccagttgctggagaaggtcaagaatgtctttaatgaaacaaagaatctccttgacaaggactggaatattttcagcaagaactgcaacaacagctttgctgaatgctccagccaagatgtggtgaccaagcctgattgcaactgcctgtaccccaaagccatccctagcagtgacccggcctctgtctcccctcatcagcccctcgccccctccatggcccctgtggctggcttgacctgggaggactctgagggaactgagggcagctccctcttgcctggtgagcagcccctgcacacagtggatccaggcagtgccaagcagcggccacccaggagcacctgccagagctttgagccgccagagaccccagttgtcaaggacagcaccatcggtggctcaccacagcctcgcccctctgtcggggccttcaaccccgggatggaggatattcttgactctgcaatgggcactaattgggtcccagaagaagcctctggagaggccagtgagattcccgtaccccaagggacagagctttccccctccaggccaggagggggcagcatgcagacagagcccgccagacccagcaacttcctctcagcatcttctccactccctgcatcagcaaagggccaacagccggcagatgtaactggtaccgccttgcccagggtgggccccgtgaggcccactggccaggactggaatcacaccccccagaagacagaccatccatctgccctgctcagagaccccccggagccaggctctcccaggatctcatcactgcgcccccagggcctcagcaacccctccaccctctctgctcagccacagctttccagaagccactcctcgggcagcgtgctgccccttggggagctggagggcaggaggagcaccagggatcggaggagccccgcagagccagaaggaggaccagcaagtgaaggggcagccaggcccctgccccgttttaactccgttcctttgactgacacaggccatgagaggcagtccgagggatcctccagcccgcagctccaggagtctgtcttccacctgctggtgcccagtgtcatcctggtcttgctggccgtcggaggcctcttgttctacaggtggaggcggcggagccatcaagagcctcagagagcggattctcccttggagcaaccagagggcagccccctgactcaggatgacagacaggtggaactgccagtgtagagggaattctaagctggacgcacagaacagtctctccgtgggaggagacattatggggcgtccaccaccacccctccctggccatcctcctggaatgtggtctgccctccaccagagctcctgcctgccaggactggaccagagcagccaggctggggcccctctgtctcaacccgcagacccttgactgaatgagagaggccagaggatgctccccatgctgccactatttattgtgagccctggaggctcccatgtgcttgaggaaggctggtgagcccggctcaggaccctcttccctcaggggctgcaccctcctctcactcccttccatgccggaacccaggccagggacccaccggcctgtggtttgtgggaaagcagggtggacgctgaggagtgaaagaaccctgcacccagagggcctgcctggtgccaaggtatcccagcctggacaggcatggacctgtctccagagagaggagcctgaagttcgtggggcgggacagcgtcggcctgatttcccgtaaaggtgtgcagcctgagagacgggaagaggaggcctctggacctgctggtctgcactgacagcctgaagggtctacaccctcggctcacctaagtgccctgtgctggttgccaggcgcagaggggaggccagccctgccctcaggacctgcctgacctgccagtgatgccaagagggggatcaagcactggcctctgcccctcctccttccagcacctgccagagcttctccaggaggccaagcagaggctcccctcatgaaggaagccattgcactgtgaacactgtacctgcctgctgaacagcctgcccccgtccatccatgagccagcatccgtccgtcctccactctccagcctctccccagcctcctgcactgagctggcctcaccagtcgactgagggagcccctcagccctgaccttctcctgacctggcctttgactccccggagtggagtggggtgggagaacctcctgggccgccagccagagccggtctttaggctgtgttgttcgcccaggtttctgcatcttgcactttgacattcccaagagggaagggactagtgggagagagcaagggaggggagggcacagacagagaggctacagggcgagctctgactgaagatgggcctttgaaatataggtatgcacctgaggttgggggagggtctgcactcccaaaccccagcgcagtgtcctttccctgctgccgacaggaacctggggctgaacaggttatccctgtcaggagccctggactgggctgcatctcagccccacctgcatggtatccagctcccatccacttctcacccttctttcctcctgaccttggtcagcagtgatgacctccaactctcacccaccccctctaccatcacctctaaccaggcaagccagggtgggagagcaatcaggagagccaggcctcagcttccaatgcctggagggcctccactttgtggccagcctgtggtggtggctctgaggcctaggcaacgagcgacagggctgccagttgcccctgggttcctttgtgctgctgtgtgcctcctctcctgccgccctttgtcctccgctaagagaccctgccctacctggccgctgggccccgtgactttcccttcctgcccaggaaagtgagggtcggctggccccaccttccctgtcctgatgccgacagcttagggaagggcagtgaacttgcatatggggcttagccttctagtcacagcctctatatttgatgctagaaaacacatatttttaaatggaagaaaaataaaaaggcattcccccttcatccccctaccttaaacatataatattttaaaggtcaaaaaagcaatccaacccactgcagaagctctttttgagcacttggtggcatcagagcaggaggagccccagagccacctctggtgtccccccaggctacctgctcaggaaccccttctgttctctgagaagtcaagagaggacattggctcacgcactgtgagattttgtttttatacttggaagtggtgaattattttatataaagtcatttaaatatctatttaaaagataggaagctgcttatatatttaataataaaagaagtgcacaagctgccaaaaaaaaaaaaaaaa

SEQ ID NO: 3 - protein, 554 aa, Homo sapiens
MTAPGAAGRCPPTTWLGSLLLLVCLLASRSITEEVSEYCSHMIGSGHLQSLQRLIDSQMETSCQITFEFVDQEQLKDPVCYLKKAFLLVQDIMEDTMRFRDNTPNAIAIVQLQELSLRLKSCFTKDYEEHDKACVRTFYETPLQLLEKVKNVFNETKNLLDKDWNIFSKNCNNSFAECSSQDVVTKPDCNCLYPKAIPSSDPASVSPHQPLAPSMAPVAGLTWEDSEGTEGSSLLPGEQPLHTVDPGSAKQRPPRSTCQSFEPPETPVVKDSTIGGSPQPRPSVGAFNPGMEDILDSAMGTNWVPEEASGEASEIPVPQGTELSPSRPGGGSMQTEPARPSNFLSASSPLPASAKGQQPADVTGTALPRVGPVRPTGQDWNHTPQKTDHPSALLRDPPEPGSPRISSLRPQGLSNPSTLSAQPQLSRSHSSGSVLPLGELEGRRSTRDRRSPAEPEGGPASEGAARPLPRFNSVPLTDTGHERQSEGSSSPQLQESVFHLLVPSVILVLLAVGGLLFYRWRRRSHQEPQRADSPLEQPEGSPLTQDDRQVELPV

SEQ ID NO: 4 - DNA, 3366 bp, Homo sapiens
cgtgggatttccagaccgcggctttctaatcggctcgggaggaagctctgcagctctcttgggaattaagctcaatctctggactctctctctttctctttctccccctccctctcctgcgaagaagctcaagacaaaaccaggaagccggcgaccctcacctcctcgggggctgggaggaaggaggaaaacgaaagtcgccgccgccgcgctgtcccccgagagctgcctttcctcgggcatccctggggctgccgcgggacctcgcagggcggatataaagaaccgcggccttgggaagaggcggagaccggcttttaaagaaagaagtcctgggtcctgcggtctggggcgaggcaagggcgcttttctgcccacgctccccgtggcccatcgatcccccgcgcgtccgccgctgttctaaggagagaagtgggggccccccaggctcgcgcgtggagcgaagcagcatgggcagtcggtgcgcgctggccctggcggtgctctcggccttgctgtgtcaggtctggagctctggggtgttcgaactgaagctgcaggagttcgtcaacaagaaggggctgctggggaaccgcaactgctgccgcgggggcgcggggccaccgccgtgcgcctgccggaccttcttccgcgtgtgcctcaagcactaccaggccagcgtgtcccccgagccgccctgcacctacggcagcgccgtcacccccgtgctgggcgtcgactccttcagtctgcccgacggcgggggcgccgactccgcgttcagcaaccccatccgcttccccttcggcttcacctggccgggcaccttctctctgattattgaagctctccacacagattctcctgatgacctcgcaacagaaaacccagaaagactcatcagccgcctggccacccagaggcacctgacggtgggcgaggagtggtcccaggacctgcacagcagcggccgcacggacctcaagtactcctaccgcttcgtgtgtgacgaacactactacggagagggctgctccgttttctgccgtccccgggacgatgccttcggccacttcacctgtggggagcgtggggagaaagtgtgcaaccctggctggaaagggccctactgcacagagccgatctgcctgcctggatgtgatgagcagcatggattttgtgacaaaccaggggaatgcaagtgcagagtgggctggcagggccggtactgtgacgagtgtatccgctatccaggctgtctccatggcacctgccagcagccctggcagtgcaactgccaggaaggctgggggggccttttctgcaaccaggacctgaactactgcacacaccataagccctgcaagaatggagccacctgcaccaacacgggccaggggagctacacttgctcttgccggcctgggtacacaggtgccacctgcgagctggggattgacgagtgtgaccccagcccttgtaagaacggagggagctgcacggatctcgagaacagctactcctgtacctgcccacccggcttctacggcaaaatctgtgaattgagtgccatgacctgtgcggacggcccttgctttaacgggggtcggtgctcagacagccccgatggagggtacagctgccgctgccccgtgggctactccggcttcaactgtgagaagaaaattgactactgcagctcttcaccctgttctaatggtgccaagtgtgtggacctcggtgatgcctacctgtgccgctgccaggccggcttctcggggaggcactgtgacgacaacgtggacgactgcgcctcctccccgtgcgccaacgggggcacctgccgggatggcgtgaacgacttctcctgcacctgcccgcctggctacacgggcaggaactgcagtgcccccgtcagcaggtgcgagcacgcaccctgccacaatggggccacctgccacgagaggggccaccgctatgtgtgcgagtgtgcccgaggctacgggggtcccaactgccagttcctgctccccgagctgcccccgggcccagcggtggtggacctcactgagaagctagagggccagggcgggccattcccctgggtggccgtgtgcgccggggtcatccttgtcctcatgctgctgctgggctgtgccgctgtggtggtctgcgtccggctgaggctgcagaagcaccggcccccagccgacccctgccggggggagacggagaccatgaacaacctggccaactgccagcgtgagaaggacatctcagtcagcatcatcggggccacgcagatcaagaacaccaacaagaaggcggacttccacggggaccacagcgccgacaagaatggcttcaaggcccgctacccagcggtggactataacctcgtgcaggacctcaagggtgacgacaccgccgtcagggacgcgcacagcaagcgtgacaccaagtgccagccccagggctcctcaggggaggagaaggggaccccgaccacactcaggggtggagaagcatctgaaagaaaaaggccggactcgggctgttcaacttcaaaagacaccaagtaccagtcggtgtacgtcatatccgaggagaaggatgagtgcgtcatagcaactgaggtgtaaaatggaagtgagatggcaagactcccgtttctcttaaaataagtaaaattccaaggatatatgccccaacgaatgctgctgaagaggagggaggcctcgtggactgctgctgagaaaccgagttcagaccgagcaggttctcctcctgaggtcctcgacgcctgccgacagcctgtcgcggcccggccgcctgcggcactgccttccgtgacgtcgccgttgcactatggacagttgctcttaagagaatatatatttaaatgggtgaactgaattacgcataagaagcatgcactgcctgagtgtatattttggattcttatgagccagtcttttcttgaattagaaacacaaacactgcctttattgtcctttttgatacgaagatgtgctttttctagatggaaaagatgtgtgttattttttggatttgtaaaaatatttttcatgatatctgtaaagcttgagtattttgtgatgttcgttttttataatttaaattttggtaaatatgtacaaaggcacttcgggtctatgtgactatatttttttgtatataaatgtatttatggaatattgtgcaaatgttatttgagttttttactgttttgttaatgaagaaattcctttttaaaatatttttccaaaataaattttatgaatgacaaaaaaaaaaaaaaaaaaaaaaaaaaaaaaaaaaaaaaaaaaaaaaaaaaaaaaaaaa

SEQ ID NO: 5 - protein, 723 aa, Homo sapiens
MGSRCALALAVLSALLCQVWSSGVFELKLQEFVNKKGLLGNRNCCRGGAGPPPCACRTFFRVCLKHYQASVSPEPPCTYGSAVTPVLGVDSFSLPDGGGADSAFSNPIRFPFGFTWPGTFSLIIEALHTDSPDDLATENPERLISRLATQRHLTVGEEWSQDLHSSGRTDLKYSYRFVCDEHYYGEGCSVFCRPRDDAFGHFTCGERGEKVCNPGWKGPYCTEPICLPGCDEQHGFCDKPGECKCRVGWQGRYCDECIRYPGCLHGTCQQPWQCNCQEGWGGLFCNQDLNYCTHHKPCKNGATCTNTGQGSYTCSCRPGYTGATCELGIDECDPSPCKNGGSCTDLENSYSCTCPPGFYGKICELSAMTCADGPCFNGGRCSDSPDGGYSCRCPVGYSGFNCEKKIDYCSSSPCSNGAKCVDLGDAYLCRCQAGFSGRHCDDNVDDCASSPCANGGTCRDGVNDFSCTCPPGYTGRNCSAPVSRCEHAPCHNGATCHERGHRYVCECARGYGGPNCQFLLPELPPGPAVVDLTEKLEGQGGPFPWVAVCAGVILVLMLLLGCAAVVVCVRLRLQKHRPPADPCRGETETMNNLANCQREKDISVSIIGATQIKNTNKKADFHGDHSADKNGFKARYPAVDYNLVQDLKGDDTAVRDAHSKRDTKCQPQGSSGEEKGTPTTLRGGEASERKRPDSGCSTSKDTKYQSVYVISEEKDECVIATEV

SEQ ID NO: 6 - protein, 848 aa, Homo sapiens
MLQTKDLIWTLFFLGTAVSLQVDIVPSQGEISVGESKFFLCQVAGDAKDKDISWFSPNGEKLTPNQQRISVVWNDDSSSTLTIYNANIDDAGIYKCVVTGEDGSESEATVNVKIFQKLMFKNAPTPQEFREGEDAVIVCDVVSSLPPTIIWKHKGRDVILKKDVRFIVLSNNYLQIRGIKKTDEGTYRCEGRILARGEINFKDIQVIVNVPPTIQARQNIVNATANLGQSVTLVCDAEGFPEPTMSWTKDGEQIEQEEDDEKYIFSDDSSQLTIKKVDKNDEAEYICIAENKAGEQDATIHLKVFAKPKITYVENQTAMELEEQVTLTCEASGDPIPSITWRTSTRNISSEEKTLDGHMVVRSHARVSSLTLKSIQYTDAGEYICTASNTIGQDSQSMYLEVQYAPKLQGPVAVYTWEGNQVNITCEVFAYPSATISWFRDGQLLPSSNYSNIKIYNTPSASYLEVTPDSENDFGNYNCTAVNRIGQESLEFILVQADTPSSPSIDQVEPYSSTAQVQFDEPEATGGVPILKYKAEWRAVGEEVWHSKWYDAKEASMEGIVTIVGLKPETTYAVRLAALNGKGLGEISAASEFKTQPVQGEPSAPKLEGQMGEDGNSIKVNLIKQDDGGSPIRHYLVRYRALSSEWKPEIRLPSGSDHVMLKSLDWNAEYEVYVVAENQQGKSKAAHFVFRTSAQPTAIPANGSPTSGLSTGAIVGILIVIFVLLLVVVDITCYFLNKCGLFMCIAVNLCGKAGPGAKGKDMEEGKAAFSKDESKEPIVEVRTEEERTPNHDGGKHTEPNETTPLTEPEKGPVEAKPECQETETKPAPAEVKTVPNDATQTKENESKA

SEQ ID NO: 7 - protein, 233 aa, Homo sapiens
MWQLLLPTALLLLVSAGMRTEDLPKAVVFLEPQWYSVLEKDSVTLKCQGAYSPEDNSTQWFHNESLISSQASSYFIDAATVNDSGEYRCQTNLSTLSDPVQLEVHIGWLLLQAPRWVFKEEDPIHLRCHSWKNTALHKVTYLQNGKDRKYFHHNSDFHIPKATLKDSGSYFCRGLVGSKNVSSETVNITITQGLAVSTISSFSPPGYQVSFCLVMVLLFAVDTGLYFSVKTNI

SEQ ID NO: 8 - protein, 177 aa, Homo sapiens
MAWMLLLILIMVHPGSCALWVSQPPEIRTLEGSSAFLPCSFNASQGRLAIGSVTWFRDEVVPGKEVRNGTPEFRGRLAPLASSRFLHDHQAELHIRDVRGHDASIYVCRVEVLGLGVGTGNGTRLVVEKEHPQLGAGTVLLLRAGFYAVSFLSVAVGSTVYYQGKYAKSTLSGFPQL

SEQ ID NO: 9 - protein, 270 aa, Homo sapiens
MAWRALHPLLLLLLLFPGSQAQSKAQVLQSVAGQTLTVRCQYPPTGSLYEKKGWCKEASALVCIRLVTSSKPRTMAWTSRFTIWDDPDAGFFTVTMTDLREEDSGHYWCRIYRPSDNSVSKSVRFYLVVSPASASTQTSWTPRDLVSSQTQTQSCVPPTAGARQAPESPSTIPVPSHPSSPLPVPLPSRPQNSTLRPGPAAPIALVPVFCGLLVAKSLVLSALLVWWVLRNRHMQHQGRSLLHPAQPRPQAHRHFPLSHRAPGGTYGGKP

SEQ ID NO: 10 - protein, 303 aa, Homo sapiens
MSSTLPALLCVGLCLSQRISAQQQTLPKPFIWAEPHFMVPKEKQVTICCQGNYGAVEYQLHFEGSLFAVDRPKPPERINKVQFYIPDMNSRMAGQYSCIYRVGELWSEPSNLLDLVVTEMYDTPTLSVHPGPEVISGEKVTFYCRLDTATSMFLLLKEGRSSHVQRGYGKVQAEFPLGPVTTAHRGTYRCFGSYNNHAWSFPSEPVKLLVTGDIENTSLAPEDPTFPDTWGTYLLTTETGLQKDHALWDHTAQNLLRMGLAFLVLVALVWFLVEDWLSRKRTRERASRASTWEGRRRLNTQTL

SEQ ID NO: 11 - protein, 216 aa, Homo sapiens
MGWIRGRRSRHSWEMSEFHNYNLDLKKSDFSTRWQKQRCPVVKSKCRENASPFFFCCFIAVAMGIRFIIMVTIWSAVFLNSLFNQEVQIPLTESYCGPCPKNWICYKNNCYQFFDESKNWYESQASCMSQNASLLKVYSKEDQDLLKLVKSYHWMGLVHIPTNGSWQWEDGSILSPNLLTIIEMQKGDCALYASSFKGYIENCSTPNTYICMQRTV

SEQ ID NO: 12 - protein, 336 aa, Homo sapiens
MDYPTLLLALLHVYRALCEEVLWHTSVPFAENMSLECVYPSMGILTQVEWFKIGTQQDSIAIFSPTHGMVIRKPYAERVYFLNSTMASNNMTLFFRNASEDDVGYYSCSLYTYPQGTWQKVIQVVQSDSFEAAVPSNSHIVSEPGKNVTLTCQPQMTWPVQAVRWEKIQPRQIDLLTYCNLVHGRNFTSKFPRQIVSNCSHGRWSVIVIPDVTVSDSGLYRCYLQASAGENETFVMRLTVAEGKTDNQYTLFVAGGTVLLLLFVISITTIIVIFLNRRRRRERRDLFTESWDTQKAPNNYRSPISTSQPTNQSMDDTREDIYVNYPTFSRRPKTRV

SEQ ID NO: 13 - protein, 281 aa, Homo sapiens
MQQPFNYPYPQIYWVDSSASSPWAPPGTVLPCPTSVPRRPGQRRPPPPPPPPPLPPPPPPPPLPPLPLPPLKKRGNHSTGLCLLVMFFMVLVALVGLGLGMFQLFHLQKELAELRESTSQMHTASSLEKQIGHPSPPPEKKELRKVAHLTGKSNSRSMPLEWEDTYGIVLLSGVKYKKGGLVINETGLYFVYSKVYFRGQSCNNLPLSHKVYMRNSKYPQDLVMMEGKMMSYCTTGQMWARSSYLGAVFNLTSADHLYVNVSELSLVNFEESQTFFGLYKL

SEQ ID NO: 14 - protein, 101 aa, Homo sapiens
MAMMEVQGGPSLGQTCVLIVIFTVLLQSLCVAVTYVYFTNELKQMQDKYSKSGIACFLKEDDSYWDPNDEESMNSPCWQVKWQLRQLVRKTPRMKRLWAAK

SEQ ID NO: 15 - protein, 233 aa, Homo sapiens
MDNQGVIYSDLNLPPNPKRQQRKPKGNKNSILATEQEITYAELNLQKASQDFQGNDKTYHCKDLPSAPEKLIVGILGIICLILMASVVTIVVIPSTLIQRHNNSSLNTRTQKARHCGHCPEEWITYSNSCYYIGKERRTWEESLLACTSKNSSLLSIDNEEEMKFLSIISPSSWIGVFRNSSHHPWVTMNGLAFKHEIKDSDNAELNCAVLQVNRLKSAQCGSSIIYHCKHKL